European Patent Application EP 4 768 039 A1, published July 1, 2026. Title: 药物组合物及其用途. Applicant: 上海瑞宏迪医药有限公司. The sequence listing filed with the application follows.

SEQUENCE LISTING (141 sequences)

SEQ ID NO: 1 - protein, 480 aa, Homo sapiens
MNASEFRRRGKEMVDYVANYMEGIEGRQVYPDVEPGYLRPLIPAAAPQEPDTFEDIINDVEKIIMPGVTHWHSPYFFAYFPTASSYPAMLADMLCGAIGCIGFSWAASPACTELETVMMDWLGKMLELPKAFLNEKAGEGGGVIQGSASEATLVALLAARTKVIHRLQAASPELTQAAIMEKLVAYSSDQAHSSVERAGLIGGVKLKAIPSDGNFAMRASALQEALERDKAAGLIPFFMVATLGTTTCCSFDNLLEVGPICNKEDIWLHVDAAYAGSAFICPEFRHLLNGVEFADSFNFNPHKWLLVNFDCSAMWVKKRTDLTGAFRLDPTYLKHSHQDSGLITDYRHWQIPLGRRFRSLKMWFVFRMYGVKGLQAYIRKHVQLSHEFESLVRQDPRFEICVEVILGLVCFRLKGSNKVNEALLQRINSAKKIHLVPCHLRDKFVLRFAICSRTVESAHVQRAWEHIKELAADVLRAERE

SEQ ID NO: 2 - protein, 211 aa, Homo sapiens
MKLWDVVAVCLVLLHTASAFPLPAGKRPPEAPAEDRSLGRRRAPFALSSDSNMPEDYPDQFDDVMDFIQATIKRLKRSPDKQMAVLPRRERNRQAAAANPENSRGKGRRGQRGKNRGCVLTAIHLNVTDLGLGYETKEELIFRYCSGSCDAAETTYDKILKNLSRNRRLVSDKVGQACCRPIAFDDDLSFLDDNLVYHILRKHSAKRCGCI

SEQ ID NO: 3 - DNA, 1443 bp, Homo sapiens
  source 1..1443: mol_type = other DNA
atgaacgcaagtgaattccgaaggagagggaaggagatggtggattacatggccaactacatggaaggcattgagggacgccaggtctaccctgacgtggagcccgggtacctgcggccgctgatccctgccgctgcccctcaggagccagacacgtttgaggacatcatcaacgacgttgagaagataatcatgcctggggtgacgcactggcacagcccctacttcttcgcctacttccccactgccagctcgtacccggccatgcttgcggacatgctgtgcggggccattggctgcatcggcttctcctgggcggcaagcccagcatgcacagagctggagactgtgatgatggactggctcgggaagatgctggaactaccaaaggcatttttgaatgagaaagctggagaagggggaggagtgatccagggaagtgccagtgaagccaccctggtggccctgctggccgctcggaccaaagtgatccatcggctgcaggcagcgtccccagagctcacacaggccgctatcatggagaagctggtggcttactcatccgatcaggcacactcctcagtggaaagagctgggttaattggtggagtgaaattaaaagccatcccctcagatggcaacttcgccatgcgtgcgtctgccctgcaggaagccctggagagagacaaagcggctggcctgattcctttctttatggttgccaccctggggaccacaacatgctgctcctttgacaatctcttagaagtcggtcctatctgcaacaaggaagacatatggctgcacgttgatgcagcctacgcaggcagtgcattcatctgccctgagttccggcaccttctgaatggagtggagtttgcagattcattcaactttaatccccacaaatggctattggtgaattttgactgttctgccatgtgggtgaaaaagagaacagacttaacgggagcctttagactggaccccacttacctgaagcacagccatcaggattcagggcttatcactgactaccggcattggcagataccactgggcagaagatttcgctctttgaaaatgtggtttgtatttaggatgtatggagtcaaaggactgcaggcttatatccgcaagcatgtccagctgtcccatgagtttgagtcactggtgcgccaggatccccgctttgaaatctgtgtggaagtcattctggggcttgtctgctttcggctaaagggttccaacaaagtgaatgaagctcttctgcaaagaataaacagtgccaaaaaaatccacttggttccatgtcacctcagggacaagtttgtcctgcgctttgccatctgttctcgcacggtggaatctgcccatgtgcagcgggcctgggaacacatcaaagagctggcggccgacgtgctgcgagcagagagggagtag

SEQ ID NO: 4 - DNA, 1443 bp, synthetic construct
  source 1..1443: mol_type = other DNA
atgaatgctagcgagtttcgcagaaggggcaaggagatggtggattacgtggctaattacatggagggcatcgagggccggcaggtgtacccagatgtggagccaggctacctgagaccactgatccctgctgccgccccacaggagccagacaccttcgaggatatcatcaatgacgtggagaagatcatcatgcctggcgtgacccactggcatagcccatacttctttgcctactttccaacagcctcttcctatcccgctatgctggctgatatgctgtgcggcgctatcggctgcatcggcttctcttgggccgctagccctgcttgcacagagctggagaccgtgatgatggattggctgggcaagatgctggagctgcctaaggcctttctgaacgagaaggctggcgagggcggcggcgtgatccagggctctgcctccgaggctacactggtggctctgctggctgcccggacaaaggtaatccacagactgcaggctgcctctccagagctgacccaggccgctatcatggagaagctggtggcttactctagcgaccaggctcattcttccgtggagcgggctggcctgatcggcggcgtgaagctgaaggccatcccttccgacggcaatttcgccatgagagcttctgccctgcaggaggctctggagagagataaggctgccggcctgatccctttctttatggtggccaccctgggcacaaccacctgttgctccttcgacaacctgctggaggtgggccctatctgtaacaaggaggacatctggctgcatgtggatgccgcttatgctggctctgcctttatctgccccgagtttagacatctgctgaacggcgtggagtttgccgacagctttaacttcaaccctcacaagtggctgctggtgaattttgactgctctgccatgtgggtgaagaagaggacagacctgaccggcgcttttaggctggatccaacctacctgaagcacagccatcaggacagcggcctgatcacagactacagacactggcagatcccactgggcagaaggtttcggtctctgaagatgtggttcgtgtttcgcatgtatggcgtgaagggcctgcaggcttatatccggaagcacgtgcagctgtctcatgagttcgagtccctggtgcggcaggacccaagatttgagatctgcgtggaggtaatcctgggcctggtgtgcttcaggctgaagggctctaataaggtgaacgaggctctgctgcagaggatcaacagcgccaagaagatccatctggtgccttgtcatctgagggacaagttcgtgctgagattcgccatctgctctagaacagtggagtctgctcatgtgcagagggcttgggagcatatcaaggagctggccgctgacgtgctgagggctgagagggagtga

SEQ ID NO: 5 - DNA, 1443 bp, synthetic construct
  source 1..1443: mol_type = other DNA
atgaacgctagcgagtttcggaggagaggcaaggagatggtggactacgtggccaactacatggagggcatcgagggcagacaggtgtacccagacgtggagcctggctatctgcggccactgatccctgctgccgccccacaggagccagatacctttgaggacatcatcaacgacgtggagaagatcatcatgcccggcgtgacccactggcattccccttacttctttgcctactttcctacagcttcttcctatcctgccatgctggccgatatgctgtgcggcgctatcggctgcatcggcttctcttgggccgcttcccccgcttgcaccgagctggagaccgtgatgatggattggctgggcaagatgctggagctgcccaaggctttcctgaatgagaaggctggcgagggcggcggcgtgatccagggctctgcttccgaggccacactggtggccctgctggctgccaggacaaaggtaatccacagactgcaggctgcctcccccgagctgacccaggccgctatcatggagaagctggtggcttactcctctgaccaggctcactcttccgtggagagagctggcctgatcggcggcgtgaagctgaaggctatcccttctgatggcaatttcgccatgagggcttctgctctgcaggaggctctggagagggataaggctgccggcctgatcccctttttcatggtggccaccctgggcacaaccacctgttgcagctttgacaatctgctggaggtgggccctatctgcaacaaggaggacatctggctgcacgtggatgctgcctacgctggcagcgccttcatctgtcccgagtttaggcacctgctgaatggcgtggagtttgctgactcctttaatttcaacccccataagtggctgctggtgaacttcgactgctctgctatgtgggtgaagaagaggacagatctgacaggcgcctttaggctggacccaacctacctgaagcactcccatcaggatagcggcctgatcaccgactaccggcactggcagatccctctgggcaggcgctttagatccctgaagatgtggttcgtgtttaggatgtacggcgtgaagggcctgcaggcttatatccggaagcatgtgcagctgtcccacgagttcgagtctctggtgcggcaggacccaaggtttgagatctgcgtggaggtaatcctgggcctggtgtgcttcagactgaagggctccaataaggtgaacgaggctctgctgcagagaatcaactccgccaagaagatccacctggtgccttgtcacctgagggataagttcgtgctgaggtttgccatctgctctagaaccgtggagagcgcccatgtgcagagggcttgggagcacatcaaggagctggctgccgacgtgctgagggctgagagagagtga

SEQ ID NO: 6 - DNA, 1443 bp, synthetic construct
  source 1..1443: mol_type = other DNA
atgaatgcctctgagttccgcagacgcggcaaggagatggtggactacgtggctaactacatggagggcatcgagggcagacaggtgtaccccgacgtggagcctggctatctgaggccactgatccctgctgctgcccctcaggagcccgacaccttcgaggatatcatcaatgacgtggagaagatcatcatgccaggcgtgacccattggcactctccatacttctttgcttacttccctaccgcctcttcctatccagctatgctggccgatatgctgtgcggcgccatcggctgcatcggctttagctgggctgcctctccagcttgtaccgagctggagacagtgatgatggactggctgggcaagatgctggagctgcctaaggcctttctgaacgagaaggccggcgagggcggcggcgtgatccagggctccgcttctgaggccaccctggtggctctgctggctgccagaaccaaggtaatccacaggctgcaggccgctagccctgagctgacccaggccgctatcatggagaagctggtggcttactcttccgaccaggcccattctagcgtggagagggctggcctgatcggcggcgtgaagctgaaggctatcccttctgacggcaacttcgccatgagagctagcgccctgcaggaggccctggagcgggacaaggctgccggcctgatcccatttttcatggtggctaccctgggcacaacaacctgctgttctttcgacaacctgctggaggtgggccctatctgcaataaggaggacatctggctgcatgtggatgctgcctatgctggcagcgcctttatctgcccagagttcaggcatctgctgaacggcgtggagtttgccgactcttttaacttcaatccccataagtggctgctggtgaactttgactgtagcgccatgtgggtgaagaagaggacagatctgaccggcgcctttcggctggatcctacctacctgaagcactctcatcaggattctggcctgatcaccgattacagacattggcagatccctctgggccggagatttcggagcctgaagatgtggttcgtgtttcggatgtatggcgtgaagggcctgcaggcctatatcagaaagcacgtgcagctgtcccacgagtttgagagcctggtgcgccaggacccacggtttgagatctgcgtggaggtaatcctgggcctggtgtgcttcaggctgaagggctctaataaggtgaacgaggctctgctgcagcgcatcaactccgctaagaagatccacctggtgccttgtcacctgcgggacaagttcgtgctgaggtttgccatctgctccagaaccgtggagtctgcccatgtgcagagagcttgggagcatatcaaggagctggccgctgatgtgctgagggctgagagagagtga

SEQ ID NO: 7 - DNA, 1443 bp, synthetic construct
  source 1..1443: mol_type = other DNA
atgaacgcctctgagtttcggaggaggggcaaggagatggtggactacgtggctaactatatggagggcatcgagggcagacaggtgtaccctgacgtggagccaggctacctgagaccactgatcccagccgccgctcctcaggagcctgacacctttgaggacatcatcaatgatgtggagaagatcatcatgcctggcgtgacccattggcacagcccttactttttcgcctatttcccaaccgctagctcctatccagccatgctggctgatatgctgtgcggcgctatcggctgtatcggctttagctgggctgcctctcctgcttgtacagagctggagacagtgatgatggattggctgggcaagatgctggagctgcccaaggcctttctgaacgagaaggccggcgagggcggcggcgtgatccagggctctgcttctgaggccacactggtggctctgctggccgctaggaccaaggtaatccacaggctgcaggctgccagcccagagctgacccaggctgccatcatggagaagctggtggcctactctagcgaccaggctcattcctctgtggagagggctggcctgatcggcggcgtgaagctgaaggctatcccttccgatggcaatttcgctatgagagccagcgccctgcaggaggctctggagagggacaaggctgccggcctgatccctttcttcatggtggccacactgggcacaaccacatgctgttctttcgacaacctgctggaggtgggccccatctgcaataaggaggacatctggctgcatgtggatgctgcctacgccggctccgcttttatctgccctgagtttcggcatctgctgaacggcgtggagtttgccgacagctttaacttcaatccccacaagtggctgctggtgaacttcgactgctctgctatgtgggtgaagaagaggacagatctgaccggcgctttcagactggatccaacctacctgaagcactctcatcaggactctggcctgatcaccgattaccggcattggcagatccctctgggccgccggtttaggagcctgaagatgtggttcgtgtttcggatgtatggcgtgaagggcctgcaggcctatatccggaagcatgtgcagctgtctcatgagtttgagtccctggtgcgccaggaccctaggttcgagatctgcgtggaggtaatcctgggcctggtgtgcttcaggctgaagggcagcaataaggtgaacgaggctctgctgcagaggatcaattccgctaagaagatccacctggtgccttgtcatctgcgggataagtttgtgctgaggttcgccatctgtagccgcaccgtggagtctgcccacgtgcagagagcttgggagcacatcaaggagctggccgctgatgtgctgagagctgagagggagtga

SEQ ID NO: 8 - DNA, 636 bp, synthetic construct
  source 1..636: mol_type = other DNA
atgaagttatgggatgtcgtggctgtctgcctggtgctgctccacaccgcgtccgccttcccgctgcccgccggtaagaggcctcccgaggcgcccgccgaagaccgctccctcggccgccgccgcgcgcccttcgcgctgagcagtgactcaaatatgccagaggattatcctgatcagttcgatgatgtcatggattttattcaagccaccattaaaagactgaaaaggtcaccagataaacaaatggcagtgcttcctagaagagagcggaatcggcaggctgcagctgccaacccagagaattccagaggaaaaggtcggagaggccagaggggcaaaaaccggggttgtgtcttaactgcaatacatttaaatgtcactgacttgggtctgggctatgaaaccaaggaggaactgatttttaggtactgcagcggctcttgcgatgcagctgagacaacgtacgacaaaatattgaaaaacttatccagaaatagaaggctggtgagtgacaaagtagggcaggcatgttgcagacccatcgcctttgatgatgacctgtcgtttttagatgataacctggtttaccatattctaagaaagcattccgctaaaaggtgtggatgtatctga

SEQ ID NO: 9 - DNA, 636 bp, synthetic construct
  source 1..636: mol_type = other DNA
atgaagctgtgggatgtggtggccgtgtgcctggtgctgctgcatacagctagcgcctttcccctgccagctggcaagagaccacctgaggctcctgccgaggacagatctctgggcaggagacgggcccctttcgctctgtctagcgattccaacatgcccgaggactatccagaccagttcgatgacgtgatggacttcatccaggctaccatcaagaggctgaagagaagcccagacaagcagatggctgtgctgcctagacgcgagaggaatagacaggccgctgctgccaatcctgagaacagcaggggcaagggccggaggggccagcgcggcaagaatagaggctgcgtgctgaccgctatccacctgaacgtgacagacctgggcctgggctacgagaccaaggaggagctgatcttccgctattgttccggctcttgtgatgccgctgagaccacatatgacaagatcctgaagaacctgagcagaaacaggagactggtgtctgacaaggtgggccaggcctgttgcagaccaatcgccttcgatgatgacctgagctttctggacgataacctggtgtatcacatcctgagaaagcactctgccaagagatgtggctgcatctga

SEQ ID NO: 10 - DNA, 636 bp, synthetic construct
  source 1..636: mol_type = other DNA
atgaagctgtgggatgtggtggccgtgtgcctggtgctgctgcatacagcttctgcctttcctctgcccgctggcaagaggcctccagaggccccagctgaggacagatccctgggcagaaggagagccccttttgctctgtccagcgactctaacatgcccgaggattatcccgaccagttcgacgatgtgatggacttcatccaggctaccatcaagaggctgaagagaagcccagataagcagatggctgtgctgccacgcagagagaggaacagacaggccgctgctgctaaccctgagaactctcggggcaagggcagaaggggccagagaggcaagaatcgcggctgcgtgctgacagctatccacctgaacgtgacagatctgggcctgggctacgagacaaaggaggagctgatcttcagatactgttctggcagctgtgatgctgccgagacaacctacgacaagatcctgaagaacctgagcagaaatcggaggctggtgtccgataaggtgggccaggcctgttgcagacctatcgctttcgacgacgatctgagcttcctggacgataacctggtgtaccacatcctgcggaagcattctgccaagagatgcggctgtatctga

SEQ ID NO: 11 - DNA, 636 bp, synthetic construct
  source 1..636: mol_type = other DNA
atgaagctgtgggatgtggtggccgtgtgcctggtgctgctgcatacagcttctgccttccctctgccagctggcaagagaccacctgaggcccccgctgaggatagaagcctgggccgcagaagggctccttttgccctgagctccgactctaatatgcctgaggattacccagaccagttcgatgacgtgatggactttatccaggccacaatcaagcgcctgaagaggtctccagacaagcagatggctgtgctgcctaggagagagagaaaccggcaggctgccgctgctaatccagagaactctaggggcaagggcaggagaggccagaggggcaagaatcgcggctgcgtgctgaccgctatccatctgaatgtgaccgatctgggcctgggctacgagacaaaggaggagctgatcttcaggtactgcagcggctcttgtgacgccgctgagaccacatacgacaagatcctgaagaacctgagcagaaaccgcagactggtgtctgataaggtgggccaggcttgttgcaggcccatcgcttttgatgacgatctgtctttcctggacgataatctggtgtaccacatcctgcggaagcactctgctaagcggtgtggctgcatctga

SEQ ID NO: 12 - DNA, 636 bp, synthetic construct
  source 1..636: mol_type = other DNA
atgaagctgtgggatgtggtggccgtgtgcctggtgctgctgcacaccgcttctgccttcccactgcctgccggcaagagacctcccgaggcccctgccgaggacagaagcctgggcaggcggagagccccatttgctctgtctagcgattccaacatgcctgaggattaccccgatcagttcgatgacgtgatggatttcatccaggccaccatcaagagactgaagagatctcctgacaagcagatggctgtgctgcctagaagggagagaaacaggcaggccgctgctgccaatccagagaactccaggggcaagggcagaaggggccagcgcggcaagaatagaggctgcgtgctgacagccatccacctgaacgtgaccgacctgggcctgggctacgagaccaaggaggagctgatcttcaggtactgtagcggctcctgtgatgctgccgagaccacatacgacaagatcctgaagaacctgtccaggaacagaaggctggtgtctgacaaggtgggccaggcttgctgtaggccaatcgctttcgacgacgatctgtcctttctggatgacaacctggtgtaccacatcctgaggaagcattccgctaagagatgtggctgcatctga

SEQ ID NO: 13 - DNA, 3064 bp, synthetic construct
  source 1..3064: mol_type = other DNA
cctgcaggcagctgcgcgctcgctcgctcactgaggccgcccgggcaaagcccgggcgtcgggcgacctttggtcgcccggcctcagtgagcgagcgagcgcgcagagagggagtggccaactccatcactaggggttcctatcgatatcaagcttcgttacataacttacggtaaatggcccgcctggctgaccgcccaacgacccccgcccattgacgtcaatagtaacgccaatagggactttccattgacgtcaatgggtggagtatttacggtaaactgcccacttggcagtacatcaagtgtatcatatgccaagtacgccccctattgacgtcaatgacggtaaatggcccgcctggcattgtgcccagtacatgaccttatgggactttcctacttggcagtacatctacgtattagtcatcgctattaccatggtcgaggtgagccccacgttctgcttcactctccccatctcccccccctccccacccccaattttgtatttatttattttttaattattttgtgcagcgatgggggcggggggggggggggggcgcgcgccaggcggggcggggcggggcgaggggcggggcggggcgaggcggagaggtgcggcggcagccaatcagagcggcgcgctccgaaagtttccttttatggcgaggcggcggcggcggcggccctataaaaagcgaagcgcgcggcgggcgggagtcgctgcgcgctgccttcgccccgtgccccgctccgccgccgcctcgcgccgcccgccccggctctgactgaccgcgttactcccacaggtgagcgggcgggacggcccttctcctccgggctgtaattagctgagcaagaggtaagggtttaagggatggttggttggtggggtattaatgtttaattacctggagcacctgcctgaaatcactttttttcaggttgggggattcgaacatcggccgccaccatgaacgccagcgagttcaggaggaggggcaaggagatggtggactacgtggccaactacatggagggcatcgagggcaggcaggtgtaccccgacgtggagcccggctacctgaggcccctgatccccgccgccgccccccaggagcccgacaccttcgaggacatcatcaacgacgtggagaagatcatcatgcccggcgtgacccactggcacagcccctacttcttcgcctacttccccaccgccagcagctaccccgccatgctggccgacatgctgtgcggcgccatcggctgcatcggcttcagctgggccgccagccccgcctgcaccgagctggagaccgtgatgatggactggctgggcaagatgctggagctgcccaaggccttcctgaacgagaaggccggcgagggcggcggcgtgatccagggcagcgccagcgaggccaccctggtggccctgctggccgccaggaccaaggtgatccacaggctgcaggccgccagccccgagctgacccaggccgccatcatggagaagctggtggcctacagcagcgaccaggcccacagcagcgtggagagggccggcctgatcggcggcgtgaagctgaaggccatccccagcgacggcaacttcgccatgagggccagcgccctgcaggaggccctggagagggacaaggccgccggcctgatccccttcttcatggtggccaccctgggcaccaccacctgctgcagcttcgacaacctgctggaggtgggccccatctgcaacaaggaggacatctggctgcacgtggacgccgcctacgccggcagcgccttcatctgccccgagttcaggcacctgctgaacggcgtggagttcgccgacagcttcaacttcaacccccacaagtggctgctggtgaacttcgactgcagcgccatgtgggtgaagaagaggaccgacctgaccggcgccttcaggctggaccccacctacctgaagcacagccaccaggacagcggcctgatcaccgactacaggcactggcagatccccctgggcaggaggttcaggagcctgaagatgtggttcgtgttcaggatgtacggcgtgaagggcctgcaggcctacatcaggaagcacgtgcagctgagccacgagttcgagagcctggtgaggcaggaccccaggttcgagatctgcgtggaggtgatcctgggcctggtgtgcttcaggctgaagggcagcaacaaggtgaacgaggccctgctgcagaggatcaacagcgccaagaagatccacctggtgccctgccacctgagggacaagttcgtgctgaggttcgccatctgcagcaggaccgtggagagcgcccacgtgcagagggcctgggagcacatcaaggagctggccgccgacgtgctgagggccgagagggagtgactcgaggggtggcatccctgtgacccctccccagtgcctctcctggccctggaagttgccactccagtgcccaccagccttgtcctaataaaattaagttgcatcattttgtctgactaggtgtccttctataatattatggggtggaggggggtggtatggagcaaggggcaagttgggaagacaacctgtagggcctgcggggtctattgggaaccaagctggagtgcagtggcacaatcttggctcactgcaatctccgcctcctgggttcaagcgattctcctgcctcagcctcccgagttgttgggattccaggcatgcatgaccaggctcagctaatttttgtttttttggtagagacggggtttcaccatattggccaggctggtctccaactcctaatctcaggtgatctacccaccttggcctcccaaattgctgggattacaggcgtgaaccactgctcccttccctgtccttcggaccgagcggcagatctaggaacccctagtgatggagttggccactccctctctgcgcgctcgctcgctcactgaggccgggcgaccaaaggtcgcccgacgcccgggctttgcccgggcggcctcagtgagcgagcgagcgcgcagctgcctgcagg

SEQ ID NO: 14 - DNA, 2709 bp, synthetic construct
  source 1..2709: mol_type = other DNA
cctgcaggcagctgcgcgctcgctcgctcactgaggccgcccgggcaaagcccgggcgtcgggcgacctttggtcgcccggcctcagtgagcgagcgagcgcgcagagagggagtggccaactccatcactaggggttcctatcgatatcaagcttcgttacataacttacggtaaatggcccgcctggctgaccgcccaacgacccccgcccattgacgtcaatagtaacgccaatagggactttccattgacgtcaatgggtggagtatttacggtaaactgcccacttggcagtacatcaagtgtatcatatgccaagtacgccccctattgacgtcaatgacggtaaatggcccgcctggcattgtgcccagtacatgaccttatgggactttcctacttggcagtacatctacgtattagtcatcgctattaccatggtcgaggtgagccccacgttctgcttcactctccccatctcccccccctccccacccccaattttgtatttatttattttttaattattttgtgcagcgatgggggcggggggggggggggggcgcgcgccaggcggggcggggcggggcgaggggcggggcggggcgaggcggagaggtgcggcggcagccaatcagagcggcgcgctccgaaagtttccttttatggcgaggcggcggcggcggcggccctataaaaagcgaagcgcgcggcgggcgggagtcgctgcgcgctgccttcgccccgtgccccgctccgccgccgcctcgcgccgcccgccccggctctgactgaccgcgttactcccacaggtgagcgggcgggacggcccttctcctccgggctgtaattagctgagcaagaggtaagggtttaagggatggttggttggtggggtattaatgtttaattacctggagcacctgcctgaaatcactttttttcaggttgggggattcgaacatcggccgccaccatgaacgccagcgagttcaggaggaggggcaaggagatggtggactacgtggccaactacatggagggcatcgagggcaggcaggtgtaccccgacgtggagcccggctacctgaggcccctgatccccgccgccgccccccaggagcccgacaccttcgaggacatcatcaacgacgtggagaagatcatcatgcccggcgtgacccactggcacagcccctacttcttcgcctacttccccaccgccagcagctaccccgccatgctggccgacatgctgtgcggcgccatcggctgcatcggcttcagctgggccgccagccccgcctgcaccgagctggagaccgtgatgatggactggctgggcaagatgctggagctgcccaaggccttcctgaacgagaaggccggcgagggcggcggcgtgatccagggcagcgccagcgaggccaccctggtggccctgctggccgccaggaccaaggtgatccacaggctgcaggccgccagccccgagctgacccaggccgccatcatggagaagctggtggcctacagcagcgaccaggcccacagcagcgtggagagggccggcctgatcggcggcgtgaagctgaaggccatccccagcgacggcaacttcgccatgagggccagcgccctgcaggaggccctggagagggacaaggccgccggcctgatccccttcttcatggtggccaccctgggcaccaccacctgctgcagcttcgacaacctgctggaggtgggccccatctgcaacaaggaggacatctggctgcacgtggacgccgcctacgccggcagcgccttcatctgccccgagttcaggcacctgctgaacggcgtggagttcgccgacagcttcaacttcaacccccacaagtggctgctggtgaacttcgactgcagcgccatgtgggtgaagaagaggaccgacctgaccggcgccttcaggctggaccccacctacctgaagcacagccaccaggacagcggcctgatcaccgactacaggcactggcagatccccctgggcaggaggttcaggagcctgaagatgtggttcgtgttcaggatgtacggcgtgaagggcctgcaggcctacatcaggaagcacgtgcagctgagccacgagttcgagagcctggtgaggcaggaccccaggttcgagatctgcgtggaggtgatcctgggcctggtgtgcttcaggctgaagggcagcaacaaggtgaacgaggccctgctgcagaggatcaacagcgccaagaagatccacctggtgccctgccacctgagggacaagttcgtgctgaggttcgccatctgcagcaggaccgtggagagcgcccacgtgcagagggcctgggagcacatcaaggagctggccgccgacgtgctgagggccgagagggagtgactcgagtaagatacattgatgagtttggacaaaccacaactagaatgcagtgaaaaaaatgctttatttgtgaaatttgtgatgctattgctttatttgtaaccattataagctgcaataaacaagttcggaccgagcggcagatctaggaacccctagtgatggagttggccactccctctctgcgcgctcgctcgctcactgaggccgggcgaccaaaggtcgcccgacgcccgggctttgcccgggcggcctcagtgagcgagcgagcgcgcagctgcctgcagg

SEQ ID NO: 15 - DNA, 3298 bp, synthetic construct
  source 1..3298: mol_type = other DNA
cctgcaggcagctgcgcgctcgctcgctcactgaggccgcccgggcaaagcccgggcgtcgggcgacctttggtcgcccggcctcagtgagcgagcgagcgcgcagagagggagtggccaactccatcactaggggttcctatcgatatcaagcttcgttacataacttacggtaaatggcccgcctggctgaccgcccaacgacccccgcccattgacgtcaatagtaacgccaatagggactttccattgacgtcaatgggtggagtatttacggtaaactgcccacttggcagtacatcaagtgtatcatatgccaagtacgccccctattgacgtcaatgacggtaaatggcccgcctggcattgtgcccagtacatgaccttatgggactttcctacttggcagtacatctacgtattagtcatcgctattaccatggtcgaggtgagccccacgttctgcttcactctccccatctcccccccctccccacccccaattttgtatttatttattttttaattattttgtgcagcgatgggggcggggggggggggggggcgcgcgccaggcggggcggggcggggcgaggggcggggcggggcgaggcggagaggtgcggcggcagccaatcagagcggcgcgctccgaaagtttccttttatggcgaggcggcggcggcggcggccctataaaaagcgaagcgcgcggcgggcgggagtcgctgcgcgctgccttcgccccgtgccccgctccgccgccgcctcgcgccgcccgccccggctctgactgaccgcgttactcccacaggtgagcgggcgggacggcccttctcctccgggctgtaattagctgagcaagaggtaagggtttaagggatggttggttggtggggtattaatgtttaattacctggagcacctgcctgaaatcactttttttcaggttgggggattcgaacatcggccgccaccatgaacgccagcgagttcaggaggaggggcaaggagatggtggactacgtggccaactacatggagggcatcgagggcaggcaggtgtaccccgacgtggagcccggctacctgaggcccctgatccccgccgccgccccccaggagcccgacaccttcgaggacatcatcaacgacgtggagaagatcatcatgcccggcgtgacccactggcacagcccctacttcttcgcctacttccccaccgccagcagctaccccgccatgctggccgacatgctgtgcggcgccatcggctgcatcggcttcagctgggccgccagccccgcctgcaccgagctggagaccgtgatgatggactggctgggcaagatgctggagctgcccaaggccttcctgaacgagaaggccggcgagggcggcggcgtgatccagggcagcgccagcgaggccaccctggtggccctgctggccgccaggaccaaggtgatccacaggctgcaggccgccagccccgagctgacccaggccgccatcatggagaagctggtggcctacagcagcgaccaggcccacagcagcgtggagagggccggcctgatcggcggcgtgaagctgaaggccatccccagcgacggcaacttcgccatgagggccagcgccctgcaggaggccctggagagggacaaggccgccggcctgatccccttcttcatggtggccaccctgggcaccaccacctgctgcagcttcgacaacctgctggaggtgggccccatctgcaacaaggaggacatctggctgcacgtggacgccgcctacgccggcagcgccttcatctgccccgagttcaggcacctgctgaacggcgtggagttcgccgacagcttcaacttcaacccccacaagtggctgctggtgaacttcgactgcagcgccatgtgggtgaagaagaggaccgacctgaccggcgccttcaggctggaccccacctacctgaagcacagccaccaggacagcggcctgatcaccgactacaggcactggcagatccccctgggcaggaggttcaggagcctgaagatgtggttcgtgttcaggatgtacggcgtgaagggcctgcaggcctacatcaggaagcacgtgcagctgagccacgagttcgagagcctggtgaggcaggaccccaggttcgagatctgcgtggaggtgatcctgggcctggtgtgcttcaggctgaagggcagcaacaaggtgaacgaggccctgctgcagaggatcaacagcgccaagaagatccacctggtgccctgccacctgagggacaagttcgtgctgaggttcgccatctgcagcaggaccgtggagagcgcccacgtgcagagggcctgggagcacatcaaggagctggccgccgacgtgctgagggccgagagggagtgactcgagaatcaacctctggattacaaaatttgtgaaagattgactggtattcttaactatgttgctccttttacgctatgtggatacgctgctttaatgcctttgtatcatgctattgcttcccgtatggctttcattttctcctccttgtataaatcctggttgctgtctctttatgaggagttgtggcccgttgtcaggcaacgtggcgtggtgtgcactgtgtttgctgacgcaacccccactggttggggcattgccaccacctgtcagctcctttccgggactttcgctttccccctccctattgccacggcggaactcatcgccgcctgccttgcccgctgctggacaggggctcggctgttgggcactgacaattccgtggtgttgtcggggaaatcatcgtcctttccttggctgctcgcctgtgttgccacctggattctgcgcgggacgtccttctgctacgtcccttcggccctcaatccagcggaccttccttcccgcggcctgctgccggctctgcggcctcttccgcgtcttcgccttcgccctcagacgagtcggatctccctttgggccgcctccccgctaagatacattgatgagtttggacaaaccacaactagaatgcagtgaaaaaaatgctttatttgtgaaatttgtgatgctattgctttatttgtaaccattataagctgcaataaacaagttcggaccgagcggcagatctaggaacccctagtgatggagttggccactccctctctgcgcgctcgctcgctcactgaggccgggcgaccaaaggtcgcccgacgcccgggctttgcccgggcggcctcagtgagcgagcgagcgcgcagctgcctgcagg

SEQ ID NO: 16 - DNA, 3988 bp, synthetic construct
  source 1..3988: mol_type = other DNA
cctgcaggcagctgcgcgctcgctcgctcactgaggccgcccgggcaaagcccgggcgtcgggcgacctttggtcgcccggcctcagtgagcgagcgagcgcgcagagagggagtggccaactccatcactaggggttcctatcgatatcaagcttcgttacataacttacggtaaatggcccgcctggctgaccgcccaacgacccccgcccattgacgtcaatagtaacgccaatagggactttccattgacgtcaatgggtggagtatttacggtaaactgcccacttggcagtacatcaagtgtatcatatgccaagtacgccccctattgacgtcaatgacggtaaatggcccgcctggcattgtgcccagtacatgaccttatgggactttcctacttggcagtacatctacgtattagtcatcgctattaccatggtcgaggtgagccccacgttctgcttcactctccccatctcccccccctccccacccccaattttgtatttatttattttttaattattttgtgcagcgatgggggcggggggggggggggggcgcgcgccaggcggggcggggcggggcgaggggcggggcggggcgaggcggagaggtgcggcggcagccaatcagagcggcgcgctccgaaagtttccttttatggcgaggcggcggcggcggcggccctataaaaagcgaagcgcgcggcgggcgggagtcgctgcgcgctgccttcgccccgtgccccgctccgccgccgcctcgcgccgcccgccccggctctgactgaccgcgttactcccacaggtgagcgggcgggacggcccttctcctccgggctgtaattagctgagcaagaggtaagggtttaagggatggttggttggtggggtattaatgtttaattacctggagcacctgcctgaaatcactttttttcaggttgggggattcgaacatcggccgccaccatgaacgccagcgagttcaggaggaggggcaaggagatggtggactacgtggccaactacatggagggcatcgagggcaggcaggtgtaccccgacgtggagcccggctacctgaggcccctgatccccgccgccgccccccaggagcccgacaccttcgaggacatcatcaacgacgtggagaagatcatcatgcccggcgtgacccactggcacagcccctacttcttcgcctacttccccaccgccagcagctaccccgccatgctggccgacatgctgtgcggcgccatcggctgcatcggcttcagctgggccgccagccccgcctgcaccgagctggagaccgtgatgatggactggctgggcaagatgctggagctgcccaaggccttcctgaacgagaaggccggcgagggcggcggcgtgatccagggcagcgccagcgaggccaccctggtggccctgctggccgccaggaccaaggtgatccacaggctgcaggccgccagccccgagctgacccaggccgccatcatggagaagctggtggcctacagcagcgaccaggcccacagcagcgtggagagggccggcctgatcggcggcgtgaagctgaaggccatccccagcgacggcaacttcgccatgagggccagcgccctgcaggaggccctggagagggacaaggccgccggcctgatccccttcttcatggtggccaccctgggcaccaccacctgctgcagcttcgacaacctgctggaggtgggccccatctgcaacaaggaggacatctggctgcacgtggacgccgcctacgccggcagcgccttcatctgccccgagttcaggcacctgctgaacggcgtggagttcgccgacagcttcaacttcaacccccacaagtggctgctggtgaacttcgactgcagcgccatgtgggtgaagaagaggaccgacctgaccggcgccttcaggctggaccccacctacctgaagcacagccaccaggacagcggcctgatcaccgactacaggcactggcagatccccctgggcaggaggttcaggagcctgaagatgtggttcgtgttcaggatgtacggcgtgaagggcctgcaggcctacatcaggaagcacgtgcagctgagccacgagttcgagagcctggtgaggcaggaccccaggttcgagatctgcgtggaggtgatcctgggcctggtgtgcttcaggctgaagggcagcaacaaggtgaacgaggccctgctgcagaggatcaacagcgccaagaagatccacctggtgccctgccacctgagggacaagttcgtgctgaggttcgccatctgcagcaggaccgtggagagcgcccacgtgcagagggcctgggagcacatcaaggagctggccgccgacgtgctgagggccgagagggaggccaccaacttctccctgctgaagcaggccggcgacgtggaggagaaccccggccccatgaagttatgggatgtcgtggctgtctgcctggtgctgctccacaccgcgtccgccttcccgctgcccgccggtaagaggcctcccgaggcgcccgccgaagaccgctccctcggccgccgccgcgcgcccttcgcgctgagcagtgactcaaatatgccagaggattatcctgatcagttcgatgatgtcatggattttattcaagccaccattaaaagactgaaaaggtcaccagataaacaaatggcagtgcttcctagaagagagcggaatcggcaggctgcagctgccaacccagagaattccagaggaaaaggtcggagaggccagaggggcaaaaaccggggttgtgtcttaactgcaatacatttaaatgtcactgacttgggtctgggctatgaaaccaaggaggaactgatttttaggtactgcagcggctcttgcgatgcagctgagacaacgtacgacaaaatattgaaaaacttatccagaaatagaaggctggtgagtgacaaagtagggcaggcatgttgcagacccatcgcctttgatgatgacctgtcgtttttagatgataacctggtttaccatattctaagaaagcattccgctaaaaggtgtggatgtatctgactcgagaatcaacctctggattacaaaatttgtgaaagattgactggtattcttaactatgttgctccttttacgctatgtggatacgctgctttaatgcctttgtatcatgctattgcttcccgtatggctttcattttctcctccttgtataaatcctggttgctgtctctttatgaggagttgtggcccgttgtcaggcaacgtggcgtggtgtgcactgtgtttgctgacgcaacccccactggttggggcattgccaccacctgtcagctcctttccgggactttcgctttccccctccctattgccacggcggaactcatcgccgcctgccttgcccgctgctggacaggggctcggctgttgggcactgacaattccgtggtgttgtcggggaaatcatcgtcctttccttggctgctcgcctgtgttgccacctggattctgcgcgggacgtccttctgctacgtcccttcggccctcaatccagcggaccttccttcccgcggcctgctgccggctctgcggcctcttccgcgtcttcgccttcgccctcagacgagtcggatctccctttgggccgcctccccgctaagatacattgatgagtttggacaaaccacaactagaatgcagtgaaaaaaatgctttatttgtgaaatttgtgatgctattgctttatttgtaaccattataagctgcaataaacaagttcggaccgagcggcagatctaggaacccctagtgatggagttggccactccctctctgcgcgctcgctcgctcactgaggccgggcgaccaaaggtcgcccgacgcccgggctttgcccgggcggcctcagtgagcgagcgagcgcgcagctgcctgcagg

SEQ ID NO: 17 - DNA, 3991 bp, synthetic construct
  source 1..3991: mol_type = other DNA
cctgcaggcagctgcgcgctcgctcgctcactgaggccgcccgggcaaagcccgggcgtcgggcgacctttggtcgcccggcctcagtgagcgagcgagcgcgcagagagggagtggccaactccatcactaggggttcctatcgatatcaagcttcgttacataacttacggtaaatggcccgcctggctgaccgcccaacgacccccgcccattgacgtcaatagtaacgccaatagggactttccattgacgtcaatgggtggagtatttacggtaaactgcccacttggcagtacatcaagtgtatcatatgccaagtacgccccctattgacgtcaatgacggtaaatggcccgcctggcattgtgcccagtacatgaccttatgggactttcctacttggcagtacatctacgtattagtcatcgctattaccatggtcgaggtgagccccacgttctgcttcactctccccatctcccccccctccccacccccaattttgtatttatttattttttaattattttgtgcagcgatgggggcggggggggggggggggcgcgcgccaggcggggcggggcggggcgaggggcggggcggggcgaggcggagaggtgcggcggcagccaatcagagcggcgcgctccgaaagtttccttttatggcgaggcggcggcggcggcggccctataaaaagcgaagcgcgcggcgggcgggagtcgctgcgcgctgccttcgccccgtgccccgctccgccgccgcctcgcgccgcccgccccggctctgactgaccgcgttactcccacaggtgagcgggcgggacggcccttctcctccgggctgtaattagctgagcaagaggtaagggtttaagggatggttggttggtggggtattaatgtttaattacctggagcacctgcctgaaatcactttttttcaggttgggggattcgaacatcggccgccaccatgaagttatgggatgtcgtggctgtctgcctggtgctgctccacaccgcgtccgccttcccgctgcccgccggtaagaggcctcccgaggcgcccgccgaagaccgctccctcggccgccgccgcgcgcccttcgcgctgagcagtgactcaaatatgccagaggattatcctgatcagttcgatgatgtcatggattttattcaagccaccattaaaagactgaaaaggtcaccagataaacaaatggcagtgcttcctagaagagagcggaatcggcaggctgcagctgccaacccagagaattccagaggaaaaggtcggagaggccagaggggcaaaaaccggggttgtgtcttaactgcaatacatttaaatgtcactgacttgggtctgggctatgaaaccaaggaggaactgatttttaggtactgcagcggctcttgcgatgcagctgagacaacgtacgacaaaatattgaaaaacttatccagaaatagaaggctggtgagtgacaaagtagggcaggcatgttgcagacccatcgcctttgatgatgacctgtcgtttttagatgataacctggtttaccatattctaagaaagcattccgctaaaaggtgtggatgtatctgagccaccaacttctccctgctgaagcaggccggcgacgtggaggagaaccccggccccatgaacgccagcgagttcaggaggaggggcaaggagatggtggactacgtggccaactacatggagggcatcgagggcaggcaggtgtaccccgacgtggagcccggctacctgaggcccctgatccccgccgccgccccccaggagcccgacaccttcgaggacatcatcaacgacgtggagaagatcatcatgcccggcgtgacccactggcacagcccctacttcttcgcctacttccccaccgccagcagctaccccgccatgctggccgacatgctgtgcggcgccatcggctgcatcggcttcagctgggccgccagccccgcctgcaccgagctggagaccgtgatgatggactggctgggcaagatgctggagctgcccaaggccttcctgaacgagaaggccggcgagggcggcggcgtgatccagggcagcgccagcgaggccaccctggtggccctgctggccgccaggaccaaggtgatccacaggctgcaggccgccagccccgagctgacccaggccgccatcatggagaagctggtggcctacagcagcgaccaggcccacagcagcgtggagagggccggcctgatcggcggcgtgaagctgaaggccatccccagcgacggcaacttcgccatgagggccagcgccctgcaggaggccctggagagggacaaggccgccggcctgatccccttcttcatggtggccaccctgggcaccaccacctgctgcagcttcgacaacctgctggaggtgggccccatctgcaacaaggaggacatctggctgcacgtggacgccgcctacgccggcagcgccttcatctgccccgagttcaggcacctgctgaacggcgtggagttcgccgacagcttcaacttcaacccccacaagtggctgctggtgaacttcgactgcagcgccatgtgggtgaagaagaggaccgacctgaccggcgccttcaggctggaccccacctacctgaagcacagccaccaggacagcggcctgatcaccgactacaggcactggcagatccccctgggcaggaggttcaggagcctgaagatgtggttcgtgttcaggatgtacggcgtgaagggcctgcaggcctacatcaggaagcacgtgcagctgagccacgagttcgagagcctggtgaggcaggaccccaggttcgagatctgcgtggaggtgatcctgggcctggtgtgcttcaggctgaagggcagcaacaaggtgaacgaggccctgctgcagaggatcaacagcgccaagaagatccacctggtgccctgccacctgagggacaagttcgtgctgaggttcgccatctgcagcaggaccgtggagagcgcccacgtgcagagggcctgggagcacatcaaggagctggccgccgacgtgctgagggccgagagggagtgactcgagaatcaacctctggattacaaaatttgtgaaagattgactggtattcttaactatgttgctccttttacgctatgtggatacgctgctttaatgcctttgtatcatgctattgcttcccgtatggctttcattttctcctccttgtataaatcctggttgctgtctctttatgaggagttgtggcccgttgtcaggcaacgtggcgtggtgtgcactgtgtttgctgacgcaacccccactggttggggcattgccaccacctgtcagctcctttccgggactttcgctttccccctccctattgccacggcggaactcatcgccgcctgccttgcccgctgctggacaggggctcggctgttgggcactgacaattccgtggtgttgtcggggaaatcatcgtcctttccttggctgctcgcctgtgttgccacctggattctgcgcgggacgtccttctgctacgtcccttcggccctcaatccagcggaccttccttcccgcggcctgctgccggctctgcggcctcttccgcgtcttcgccttcgccctcagacgagtcggatctccctttgggccgcctccccgctaagatacattgatgagtttggacaaaccacaactagaatgcagtgaaaaaaatgctttatttgtgaaatttgtgatgctattgctttatttgtaaccattataagctgcaataaacaagttcggaccgagcggcagatctaggaacccctagtgatggagttggccactccctctctgcgcgctcgctcgctcactgaggccgggcgaccaaaggtcgcccgacgcccgggctttgcccgggcggcctcagtgagcgagcgagcgcgcagctgcctgcagg

SEQ ID NO: 18 - DNA, 3933 bp, synthetic construct
  source 1..3933: mol_type = other DNA
cctgcaggcagctgcgcgctcgctcgctcactgaggccgcccgggcaaagcccgggcgtcgggcgacctttggtcgcccggcctcagtgagcgagcgagcgcgcagagagggagtggccaactccatcactaggggttcctatcgatatcaagcttcgttacataacttacggtaaatggcccgcctggctgaccgcccaacgacccccgcccattgacgtcaatagtaacgccaatagggactttccattgacgtcaatgggtggagtatttacggtaaactgcccacttggcagtacatcaagtgtatcatatgccaagtacgccccctattgacgtcaatgacggtaaatggcccgcctggcattgtgcccagtacatgaccttatgggactttcctacttggcagtacatctacgtattagtcatcgctattaccatggtcgaggtgagccccacgttctgcttcactctccccatctcccccccctccccacccccaattttgtatttatttattttttaattattttgtgcagcgatgggggcggggggggggggggggcgcgcgccaggcggggcggggcggggcgaggggcggggcggggcgaggcggagaggtgcggcggcagccaatcagagcggcgcgctccgaaagtttccttttatggcgaggcggcggcggcggcggccctataaaaagcgaagcgcgcggcgggcgggagtcgctgcgcgctgccttcgccccgtgccccgctccgccgccgcctcgcgccgcccgccccggctctgactgaccgcgttactcccacaggtgagcgggcgggacggcccttctcctccgggctgtaattagctgagcaagaggtaagggtttaagggatggttggttggtggggtattaatgtttaattacctggagcacctgcctgaaatcactttttttcaggttgggggattcgaacatcggccgccaccatgaacgccagcgagttcaggaggaggggcaaggagatggtggactacgtggccaactacatggagggcatcgagggcaggcaggtgtaccccgacgtggagcccggctacctgaggcccctgatccccgccgccgccccccaggagcccgacaccttcgaggacatcatcaacgacgtggagaagatcatcatgcccggcgtgacccactggcacagcccctacttcttcgcctacttccccaccgccagcagctaccccgccatgctggccgacatgctgtgcggcgccatcggctgcatcggcttcagctgggccgccagccccgcctgcaccgagctggagaccgtgatgatggactggctgggcaagatgctggagctgcccaaggccttcctgaacgagaaggccggcgagggcggcggcgtgatccagggcagcgccagcgaggccaccctggtggccctgctggccgccaggaccaaggtgatccacaggctgcaggccgccagccccgagctgacccaggccgccatcatggagaagctggtggcctacagcagcgaccaggcccacagcagcgtggagagggccggcctgatcggcggcgtgaagctgaaggccatccccagcgacggcaacttcgccatgagggccagcgccctgcaggaggccctggagagggacaaggccgccggcctgatccccttcttcatggtggccaccctgggcaccaccacctgctgcagcttcgacaacctgctggaggtgggccccatctgcaacaaggaggacatctggctgcacgtggacgccgcctacgccggcagcgccttcatctgccccgagttcaggcacctgctgaacggcgtggagttcgccgacagcttcaacttcaacccccacaagtggctgctggtgaacttcgactgcagcgccatgtgggtgaagaagaggaccgacctgaccggcgccttcaggctggaccccacctacctgaagcacagccaccaggacagcggcctgatcaccgactacaggcactggcagatccccctgggcaggaggttcaggagcctgaagatgtggttcgtgttcaggatgtacggcgtgaagggcctgcaggcctacatcaggaagcacgtgcagctgagccacgagttcgagagcctggtgaggcaggaccccaggttcgagatctgcgtggaggtgatcctgggcctggtgtgcttcaggctgaagggcagcaacaaggtgaacgaggccctgctgcagaggatcaacagcgccaagaagatccacctggtgccctgccacctgagggacaagttcgtgctgaggttcgccatctgcagcaggaccgtggagagcgcccacgtgcagagggcctgggagcacatcaaggagctggccgccgacgtgctgagggccgagagggagtgactcgagtaagatacattgatgagtttggacaaaccacaactagaatgcagtgaaaaaaatgctttatttgtgaaatttgtgatgctattgctttatttgtaaccattataagctgcaataaacaagttcgttacataacttacggtaaatggcccgcctggctgaccgcccaacgacccccgcccattgacgtcaataatgacgtatgttcccatagtaacgtcaatagggactttccattgacgtcaatgggtggagtatttacggtaaactgcccacttggcagtacatcaagtgtatcatatgccaagtacgccccctattgacgtcaatgacggtaaatggcccgcctggcattatgcccagtacatgaccttatgggactttcctacttggcagtacatctacgtattagtcatcgctattaccatggtgatgcggttttggcagtacatcaatgggcgtggatagcggtttgactcacggggatttccaagtctccaccccattgacgtcaatgggagtttgttttgcaccaaaatcaacgggactttccaaaatgtcgtaacaactccgccccattgacgcaaatgggcggtaggcgtgtacggtgggaggtctatataagcagagctgccaccatgaagttatgggatgtcgtggctgtctgcctggtgctgctccacaccgcgtccgccttcccgctgcccgccggtaagaggcctcccgaggcgcccgccgaagaccgctccctcggccgccgccgcgcgcccttcgcgctgagcagtgactcaaatatgccagaggattatcctgatcagttcgatgatgtcatggattttattcaagccaccattaaaagactgaaaaggtcaccagataaacaaatggcagtgcttcctagaagagagcggaatcggcaggctgcagctgccaacccagagaattccagaggaaaaggtcggagaggccagaggggcaaaaaccggggttgtgtcttaactgcaatacatttaaatgtcactgacttgggtctgggctatgaaaccaaggaggaactgatttttaggtactgcagcggctcttgcgatgcagctgagacaacgtacgacaaaatattgaaaaacttatccagaaatagaaggctggtgagtgacaaagtagggcaggcatgttgcagacccatcgcctttgatgatgacctgtcgtttttagatgataacctggtttaccatattctaagaaagcattccgctaaaaggtgtggatgtatctgaaataaagtctgagtgggcggcagcctgtgtgtgcctgggttctctctgtcccggaatgtgcaaacaatggaggtgcggaccgagcggcagatctaggaacccctagtgatggagttggccactccctctctgcgcgctcgctcgctcactgaggccgggcgaccaaaggtcgcccgacgcccgggctttgcccgggcggcctcagtgagcgagcgagcgcgcagctgcctgcagg

SEQ ID NO: 19 - DNA, 4522 bp, synthetic construct
  source 1..4522: mol_type = other DNA
cctgcaggcagctgcgcgctcgctcgctcactgaggccgcccgggcaaagcccgggcgtcgggcgacctttggtcgcccggcctcagtgagcgagcgagcgcgcagagagggagtggccaactccatcactaggggttcctatcgatatcaagcttcgttacataacttacggtaaatggcccgcctggctgaccgcccaacgacccccgcccattgacgtcaatagtaacgccaatagggactttccattgacgtcaatgggtggagtatttacggtaaactgcccacttggcagtacatcaagtgtatcatatgccaagtacgccccctattgacgtcaatgacggtaaatggcccgcctggcattgtgcccagtacatgaccttatgggactttcctacttggcagtacatctacgtattagtcatcgctattaccatggtcgaggtgagccccacgttctgcttcactctccccatctcccccccctccccacccccaattttgtatttatttattttttaattattttgtgcagcgatgggggcggggggggggggggggcgcgcgccaggcggggcggggcggggcgaggggcggggcggggcgaggcggagaggtgcggcggcagccaatcagagcggcgcgctccgaaagtttccttttatggcgaggcggcggcggcggcggccctataaaaagcgaagcgcgcggcgggcgggagtcgctgcgcgctgccttcgccccgtgccccgctccgccgccgcctcgcgccgcccgccccggctctgactgaccgcgttactcccacaggtgagcgggcgggacggcccttctcctccgggctgtaattagctgagcaagaggtaagggtttaagggatggttggttggtggggtattaatgtttaattacctggagcacctgcctgaaatcactttttttcaggttgggggattcgaacatcggccgccaccatgaacgccagcgagttcaggaggaggggcaaggagatggtggactacgtggccaactacatggagggcatcgagggcaggcaggtgtaccccgacgtggagcccggctacctgaggcccctgatccccgccgccgccccccaggagcccgacaccttcgaggacatcatcaacgacgtggagaagatcatcatgcccggcgtgacccactggcacagcccctacttcttcgcctacttccccaccgccagcagctaccccgccatgctggccgacatgctgtgcggcgccatcggctgcatcggcttcagctgggccgccagccccgcctgcaccgagctggagaccgtgatgatggactggctgggcaagatgctggagctgcccaaggccttcctgaacgagaaggccggcgagggcggcggcgtgatccagggcagcgccagcgaggccaccctggtggccctgctggccgccaggaccaaggtgatccacaggctgcaggccgccagccccgagctgacccaggccgccatcatggagaagctggtggcctacagcagcgaccaggcccacagcagcgtggagagggccggcctgatcggcggcgtgaagctgaaggccatccccagcgacggcaacttcgccatgagggccagcgccctgcaggaggccctggagagggacaaggccgccggcctgatccccttcttcatggtggccaccctgggcaccaccacctgctgcagcttcgacaacctgctggaggtgggccccatctgcaacaaggaggacatctggctgcacgtggacgccgcctacgccggcagcgccttcatctgccccgagttcaggcacctgctgaacggcgtggagttcgccgacagcttcaacttcaacccccacaagtggctgctggtgaacttcgactgcagcgccatgtgggtgaagaagaggaccgacctgaccggcgccttcaggctggaccccacctacctgaagcacagccaccaggacagcggcctgatcaccgactacaggcactggcagatccccctgggcaggaggttcaggagcctgaagatgtggttcgtgttcaggatgtacggcgtgaagggcctgcaggcctacatcaggaagcacgtgcagctgagccacgagttcgagagcctggtgaggcaggaccccaggttcgagatctgcgtggaggtgatcctgggcctggtgtgcttcaggctgaagggcagcaacaaggtgaacgaggccctgctgcagaggatcaacagcgccaagaagatccacctggtgccctgccacctgagggacaagttcgtgctgaggttcgccatctgcagcaggaccgtggagagcgcccacgtgcagagggcctgggagcacatcaaggagctggccgccgacgtgctgagggccgagagggagtgactcgagtaagatacattgatgagtttggacaaaccacaactagaatgcagtgaaaaaaatgctttatttgtgaaatttgtgatgctattgctttatttgtaaccattataagctgcaataaacaagttcgttacataacttacggtaaatggcccgcctggctgaccgcccaacgacccccgcccattgacgtcaataatgacgtatgttcccatagtaacgtcaatagggactttccattgacgtcaatgggtggagtatttacggtaaactgcccacttggcagtacatcaagtgtatcatatgccaagtacgccccctattgacgtcaatgacggtaaatggcccgcctggcattatgcccagtacatgaccttatgggactttcctacttggcagtacatctacgtattagtcatcgctattaccatggtgatgcggttttggcagtacatcaatgggcgtggatagcggtttgactcacggggatttccaagtctccaccccattgacgtcaatgggagtttgttttgcaccaaaatcaacgggactttccaaaatgtcgtaacaactccgccccattgacgcaaatgggcggtaggcgtgtacggtgggaggtctatataagcagagctgccaccatgaagttatgggatgtcgtggctgtctgcctggtgctgctccacaccgcgtccgccttcccgctgcccgccggtaagaggcctcccgaggcgcccgccgaagaccgctccctcggccgccgccgcgcgcccttcgcgctgagcagtgactcaaatatgccagaggattatcctgatcagttcgatgatgtcatggattttattcaagccaccattaaaagactgaaaaggtcaccagataaacaaatggcagtgcttcctagaagagagcggaatcggcaggctgcagctgccaacccagagaattccagaggaaaaggtcggagaggccagaggggcaaaaaccggggttgtgtcttaactgcaatacatttaaatgtcactgacttgggtctgggctatgaaaccaaggaggaactgatttttaggtactgcagcggctcttgcgatgcagctgagacaacgtacgacaaaatattgaaaaacttatccagaaatagaaggctggtgagtgacaaagtagggcaggcatgttgcagacccatcgcctttgatgatgacctgtcgtttttagatgataacctggtttaccatattctaagaaagcattccgctaaaaggtgtggatgtatctgaaatcaacctctggattacaaaatttgtgaaagattgactggtattcttaactatgttgctccttttacgctatgtggatacgctgctttaatgcctttgtatcatgctattgcttcccgtatggctttcattttctcctccttgtataaatcctggttgctgtctctttatgaggagttgtggcccgttgtcaggcaacgtggcgtggtgtgcactgtgtttgctgacgcaacccccactggttggggcattgccaccacctgtcagctcctttccgggactttcgctttccccctccctattgccacggcggaactcatcgccgcctgccttgcccgctgctggacaggggctcggctgttgggcactgacaattccgtggtgttgtcggggaaatcatcgtcctttccttggctgctcgcctgtgttgccacctggattctgcgcgggacgtccttctgctacgtcccttcggccctcaatccagcggaccttccttcccgcggcctgctgccggctctgcggcctcttccgcgtcttcgccttcgccctcagacgagtcggatctccctttgggccgcctccccgcaataaagtctgagtgggcggcagcctgtgtgtgcctgggttctctctgtcccggaatgtgcaaacaatggaggtgcggaccgagcggcagatctaggaacccctagtgatggagttggccactccctctctgcgcgctcgctcgctcactgaggccgggcgaccaaaggtcgcccgacgcccgggctttgcccgggcggcctcagtgagcgagcgagcgcgcagctgcctgcagg

SEQ ID NO: 20 - DNA, 4506 bp, synthetic construct
  source 1..4506: mol_type = other DNA
cctgcaggcagctgcgcgctcgctcgctcactgaggccgcccgggcaaagcccgggcgtcgggcgacctttggtcgcccggcctcagtgagcgagcgagcgcgcagagagggagtggccaactccatcactaggggttcctatcgatatcaagcttcgttacataacttacggtaaatggcccgcctggctgaccgcccaacgacccccgcccattgacgtcaatagtaacgccaatagggactttccattgacgtcaatgggtggagtatttacggtaaactgcccacttggcagtacatcaagtgtatcatatgccaagtacgccccctattgacgtcaatgacggtaaatggcccgcctggcattgtgcccagtacatgaccttatgggactttcctacttggcagtacatctacgtattagtcatcgctattaccatggtcgaggtgagccccacgttctgcttcactctccccatctcccccccctccccacccccaattttgtatttatttattttttaattattttgtgcagcgatgggggcggggggggggggggggcgcgcgccaggcggggcggggcggggcgaggggcggggcggggcgaggcggagaggtgcggcggcagccaatcagagcggcgcgctccgaaagtttccttttatggcgaggcggcggcggcggcggccctataaaaagcgaagcgcgcggcgggcgggagtcgctgcgcgctgccttcgccccgtgccccgctccgccgccgcctcgcgccgcccgccccggctctgactgaccgcgttactcccacaggtgagcgggcgggacggcccttctcctccgggctgtaattagctgagcaagaggtaagggtttaagggatggttggttggtggggtattaatgtttaattacctggagcacctgcctgaaatcactttttttcaggttgggggattcgaacatcggccgccaccatgaacgccagcgagttcaggaggaggggcaaggagatggtggactacgtggccaactacatggagggcatcgagggcaggcaggtgtaccccgacgtggagcccggctacctgaggcccctgatccccgccgccgccccccaggagcccgacaccttcgaggacatcatcaacgacgtggagaagatcatcatgcccggcgtgacccactggcacagcccctacttcttcgcctacttccccaccgccagcagctaccccgccatgctggccgacatgctgtgcggcgccatcggctgcatcggcttcagctgggccgccagccccgcctgcaccgagctggagaccgtgatgatggactggctgggcaagatgctggagctgcccaaggccttcctgaacgagaaggccggcgagggcggcggcgtgatccagggcagcgccagcgaggccaccctggtggccctgctggccgccaggaccaaggtgatccacaggctgcaggccgccagccccgagctgacccaggccgccatcatggagaagctggtggcctacagcagcgaccaggcccacagcagcgtggagagggccggcctgatcggcggcgtgaagctgaaggccatccccagcgacggcaacttcgccatgagggccagcgccctgcaggaggccctggagagggacaaggccgccggcctgatccccttcttcatggtggccaccctgggcaccaccacctgctgcagcttcgacaacctgctggaggtgggccccatctgcaacaaggaggacatctggctgcacgtggacgccgcctacgccggcagcgccttcatctgccccgagttcaggcacctgctgaacggcgtggagttcgccgacagcttcaacttcaacccccacaagtggctgctggtgaacttcgactgcagcgccatgtgggtgaagaagaggaccgacctgaccggcgccttcaggctggaccccacctacctgaagcacagccaccaggacagcggcctgatcaccgactacaggcactggcagatccccctgggcaggaggttcaggagcctgaagatgtggttcgtgttcaggatgtacggcgtgaagggcctgcaggcctacatcaggaagcacgtgcagctgagccacgagttcgagagcctggtgaggcaggaccccaggttcgagatctgcgtggaggtgatcctgggcctggtgtgcttcaggctgaagggcagcaacaaggtgaacgaggccctgctgcagaggatcaacagcgccaagaagatccacctggtgccctgccacctgagggacaagttcgtgctgaggttcgccatctgcagcaggaccgtggagagcgcccacgtgcagagggcctgggagcacatcaaggagctggccgccgacgtgctgagggccgagagggagtgactcgagtaagatacattgatgagtttggacaaaccacaactagaatgcagtgaaaaaaatgctttatttgtgaaatttgtgatgctattgctttatttgtaaccattataagctgcaataaacaagttcgttacataacttacggtaaatggcccgcctggctgaccgcccaacgacccccgcccattgacgtcaataatgacgtatgttcccatagtaacgtcaatagggactttccattgacgtcaatgggtggagtatttacggtaaactgcccacttggcagtacatcaagtgtatcatatgccaagtacgccccctattgacgtcaatgacggtaaatggcccgcctggcattatgcccagtacatgaccttatgggactttcctacttggcagtacatctacgtattagtcatcgctattaccatggtgatgcggttttggcagtacatcaatgggcgtggatagcggtttgactcacggggatttccaagtctccaccccattgacgtcaatgggagtttgttttgcaccaaaatcaacgggactttccaaaatgtcgtaacaactccgccccattgacgcaaatgggcggtaggcgtgtacggtgggaggtctatataagcagagctgtgagtttggggacccttgattgttctttctttttcgctattgtaaaattcatgttatatggagggggcaaagttttcagggtgttgtttagaatgggaagatgtcccttgtatcaccatggaccctcatgataattttgtttctttcactttctactctgttgacaaccattgtctcctcttattttcttttcattttctgtaactttttcgttaaactttagcttgcatttgtaacgaatttttaaattcacttttgtttatttgtcagattgtaagtactttctctaatcacttttttttcaaggcaatcagggtatattatattgtacttcagcacagttttagagaacaattgttataattaaatgataaggtagaatatttctgcatataaattctggctggcgtggaaatattcttattggtagaaacaactacatcctggtcatcatcctgcctttctctttatggttacaatgatatacactgtttgagatgaggataaaatactctgagtccaaaccgggcccctctgctaaccatgttcatgccttcttctttttcctacaggccaccatgaagttatgggatgtcgtggctgtctgcctggtgctgctccacaccgcgtccgccttcccgctgcccgccggtaagaggcctcccgaggcgcccgccgaagaccgctccctcggccgccgccgcgcgcccttcgcgctgagcagtgactcaaatatgccagaggattatcctgatcagttcgatgatgtcatggattttattcaagccaccattaaaagactgaaaaggtcaccagataaacaaatggcagtgcttcctagaagagagcggaatcggcaggctgcagctgccaacccagagaattccagaggaaaaggtcggagaggccagaggggcaaaaaccggggttgtgtcttaactgcaatacatttaaatgtcactgacttgggtctgggctatgaaaccaaggaggaactgatttttaggtactgcagcggctcttgcgatgcagctgagacaacgtacgacaaaatattgaaaaacttatccagaaatagaaggctggtgagtgacaaagtagggcaggcatgttgcagacccatcgcctttgatgatgacctgtcgtttttagatgataacctggtttaccatattctaagaaagcattccgctaaaaggtgtggatgtatctgaaataaagtctgagtgggcggcagcctgtgtgtgcctgggttctctctgtcccggaatgtgcaaacaatggaggtgcggaccgagcggcagatctaggaacccctagtgatggagttggccactccctctctgcgcgctcgctcgctcactgaggccgggcgaccaaaggtcgcccgacgcccgggctttgcccgggcggcctcagtgagcgagcgagcgcgcagctgcctgcagg

SEQ ID NO: 21 - DNA, 4506 bp, synthetic construct
  source 1..4506: mol_type = other DNA
cctgcaggcagctgcgcgctcgctcgctcactgaggccgcccgggcaaagcccgggcgtcgggcgacctttggtcgcccggcctcagtgagcgagcgagcgcgcagagagggagtggccaactccatcactaggggttcctatcgatatccgttacataacttacggtaaatggcccgcctggctgaccgcccaacgacccccgcccattgacgtcaataatgacgtatgttcccatagtaacgtcaatagggactttccattgacgtcaatgggtggagtatttacggtaaactgcccacttggcagtacatcaagtgtatcatatgccaagtacgccccctattgacgtcaatgacggtaaatggcccgcctggcattatgcccagtacatgaccttatgggactttcctacttggcagtacatctacgtattagtcatcgctattaccatggtgatgcggttttggcagtacatcaatgggcgtggatagcggtttgactcacggggatttccaagtctccaccccattgacgtcaatgggagtttgttttgcaccaaaatcaacgggactttccaaaatgtcgtaacaactccgccccattgacgcaaatgggcggtaggcgtgtacggtgggaggtctatataagcagagctgtgagtttggggacccttgattgttctttctttttcgctattgtaaaattcatgttatatggagggggcaaagttttcagggtgttgtttagaatgggaagatgtcccttgtatcaccatggaccctcatgataattttgtttctttcactttctactctgttgacaaccattgtctcctcttattttcttttcattttctgtaactttttcgttaaactttagcttgcatttgtaacgaatttttaaattcacttttgtttatttgtcagattgtaagtactttctctaatcacttttttttcaaggcaatcagggtatattatattgtacttcagcacagttttagagaacaattgttataattaaatgataaggtagaatatttctgcatataaattctggctggcgtggaaatattcttattggtagaaacaactacatcctggtcatcatcctgcctttctctttatggttacaatgatatacactgtttgagatgaggataaaatactctgagtccaaaccgggcccctctgctaaccatgttcatgccttcttctttttcctacaggccaccatgaagttatgggatgtcgtggctgtctgcctggtgctgctccacaccgcgtccgccttcccgctgcccgccggtaagaggcctcccgaggcgcccgccgaagaccgctccctcggccgccgccgcgcgcccttcgcgctgagcagtgactcaaatatgccagaggattatcctgatcagttcgatgatgtcatggattttattcaagccaccattaaaagactgaaaaggtcaccagataaacaaatggcagtgcttcctagaagagagcggaatcggcaggctgcagctgccaacccagagaattccagaggaaaaggtcggagaggccagaggggcaaaaaccggggttgtgtcttaactgcaatacatttaaatgtcactgacttgggtctgggctatgaaaccaaggaggaactgatttttaggtactgcagcggctcttgcgatgcagctgagacaacgtacgacaaaatattgaaaaacttatccagaaatagaaggctggtgagtgacaaagtagggcaggcatgttgcagacccatcgcctttgatgatgacctgtcgtttttagatgataacctggtttaccatattctaagaaagcattccgctaaaaggtgtggatgtatctgaaataaagtctgagtgggcggcagcctgtgtgtgcctgggttctctctgtcccggaatgtgcaaacaatggaggtgaagcttcgttacataacttacggtaaatggcccgcctggctgaccgcccaacgacccccgcccattgacgtcaatagtaacgccaatagggactttccattgacgtcaatgggtggagtatttacggtaaactgcccacttggcagtacatcaagtgtatcatatgccaagtacgccccctattgacgtcaatgacggtaaatggcccgcctggcattgtgcccagtacatgaccttatgggactttcctacttggcagtacatctacgtattagtcatcgctattaccatggtcgaggtgagccccacgttctgcttcactctccccatctcccccccctccccacccccaattttgtatttatttattttttaattattttgtgcagcgatgggggcggggggggggggggggcgcgcgccaggcggggcggggcggggcgaggggcggggcggggcgaggcggagaggtgcggcggcagccaatcagagcggcgcgctccgaaagtttccttttatggcgaggcggcggcggcggcggccctataaaaagcgaagcgcgcggcgggcgggagtcgctgcgcgctgccttcgccccgtgccccgctccgccgccgcctcgcgccgcccgccccggctctgactgaccgcgttactcccacaggtgagcgggcgggacggcccttctcctccgggctgtaattagctgagcaagaggtaagggtttaagggatggttggttggtggggtattaatgtttaattacctggagcacctgcctgaaatcactttttttcaggttgggggattcgaacatcggccgccaccatgaacgccagcgagttcaggaggaggggcaaggagatggtggactacgtggccaactacatggagggcatcgagggcaggcaggtgtaccccgacgtggagcccggctacctgaggcccctgatccccgccgccgccccccaggagcccgacaccttcgaggacatcatcaacgacgtggagaagatcatcatgcccggcgtgacccactggcacagcccctacttcttcgcctacttccccaccgccagcagctaccccgccatgctggccgacatgctgtgcggcgccatcggctgcatcggcttcagctgggccgccagccccgcctgcaccgagctggagaccgtgatgatggactggctgggcaagatgctggagctgcccaaggccttcctgaacgagaaggccggcgagggcggcggcgtgatccagggcagcgccagcgaggccaccctggtggccctgctggccgccaggaccaaggtgatccacaggctgcaggccgccagccccgagctgacccaggccgccatcatggagaagctggtggcctacagcagcgaccaggcccacagcagcgtggagagggccggcctgatcggcggcgtgaagctgaaggccatccccagcgacggcaacttcgccatgagggccagcgccctgcaggaggccctggagagggacaaggccgccggcctgatccccttcttcatggtggccaccctgggcaccaccacctgctgcagcttcgacaacctgctggaggtgggccccatctgcaacaaggaggacatctggctgcacgtggacgccgcctacgccggcagcgccttcatctgccccgagttcaggcacctgctgaacggcgtggagttcgccgacagcttcaacttcaacccccacaagtggctgctggtgaacttcgactgcagcgccatgtgggtgaagaagaggaccgacctgaccggcgccttcaggctggaccccacctacctgaagcacagccaccaggacagcggcctgatcaccgactacaggcactggcagatccccctgggcaggaggttcaggagcctgaagatgtggttcgtgttcaggatgtacggcgtgaagggcctgcaggcctacatcaggaagcacgtgcagctgagccacgagttcgagagcctggtgaggcaggaccccaggttcgagatctgcgtggaggtgatcctgggcctggtgtgcttcaggctgaagggcagcaacaaggtgaacgaggccctgctgcagaggatcaacagcgccaagaagatccacctggtgccctgccacctgagggacaagttcgtgctgaggttcgccatctgcagcaggaccgtggagagcgcccacgtgcagagggcctgggagcacatcaaggagctggccgccgacgtgctgagggccgagagggagtgactcgagtaagatacattgatgagtttggacaaaccacaactagaatgcagtgaaaaaaatgctttatttgtgaaatttgtgatgctattgctttatttgtaaccattataagctgcaataaacaagttcggaccgagcggcagatctaggaacccctagtgatggagttggccactccctctctgcgcgctcgctcgctcactgaggccgggcgaccaaaggtcgcccgacgcccgggctttgcccgggcggcctcagtgagcgagcgagcgcgcagctgcctgcagg

SEQ ID NO: 22 - DNA, 4522 bp, synthetic construct
  source 1..4522: mol_type = other DNA
cctgcaggcagctgcgcgctcgctcgctcactgaggccgcccgggcaaagcccgggcgtcgggcgacctttggtcgcccggcctcagtgagcgagcgagcgcgcagagagggagtggccaactccatcactaggggttcctatcgatatccgttacataacttacggtaaatggcccgcctggctgaccgcccaacgacccccgcccattgacgtcaataatgacgtatgttcccatagtaacgtcaatagggactttccattgacgtcaatgggtggagtatttacggtaaactgcccacttggcagtacatcaagtgtatcatatgccaagtacgccccctattgacgtcaatgacggtaaatggcccgcctggcattatgcccagtacatgaccttatgggactttcctacttggcagtacatctacgtattagtcatcgctattaccatggtgatgcggttttggcagtacatcaatgggcgtggatagcggtttgactcacggggatttccaagtctccaccccattgacgtcaatgggagtttgttttgcaccaaaatcaacgggactttccaaaatgtcgtaacaactccgccccattgacgcaaatgggcggtaggcgtgtacggtgggaggtctatataagcagagctgccaccatgaagttatgggatgtcgtggctgtctgcctggtgctgctccacaccgcgtccgccttcccgctgcccgccggtaagaggcctcccgaggcgcccgccgaagaccgctccctcggccgccgccgcgcgcccttcgcgctgagcagtgactcaaatatgccagaggattatcctgatcagttcgatgatgtcatggattttattcaagccaccattaaaagactgaaaaggtcaccagataaacaaatggcagtgcttcctagaagagagcggaatcggcaggctgcagctgccaacccagagaattccagaggaaaaggtcggagaggccagaggggcaaaaaccggggttgtgtcttaactgcaatacatttaaatgtcactgacttgggtctgggctatgaaaccaaggaggaactgatttttaggtactgcagcggctcttgcgatgcagctgagacaacgtacgacaaaatattgaaaaacttatccagaaatagaaggctggtgagtgacaaagtagggcaggcatgttgcagacccatcgcctttgatgatgacctgtcgtttttagatgataacctggtttaccatattctaagaaagcattccgctaaaaggtgtggatgtatctgaaataaagtctgagtgggcggcagcctgtgtgtgcctgggttctctctgtcccggaatgtgcaaacaatggaggtgaagcttcgttacataacttacggtaaatggcccgcctggctgaccgcccaacgacccccgcccattgacgtcaatagtaacgccaatagggactttccattgacgtcaatgggtggagtatttacggtaaactgcccacttggcagtacatcaagtgtatcatatgccaagtacgccccctattgacgtcaatgacggtaaatggcccgcctggcattgtgcccagtacatgaccttatgggactttcctacttggcagtacatctacgtattagtcatcgctattaccatggtcgaggtgagccccacgttctgcttcactctccccatctcccccccctccccacccccaattttgtatttatttattttttaattattttgtgcagcgatgggggcggggggggggggggggcgcgcgccaggcggggcggggcggggcgaggggcggggcggggcgaggcggagaggtgcggcggcagccaatcagagcggcgcgctccgaaagtttccttttatggcgaggcggcggcggcggcggccctataaaaagcgaagcgcgcggcgggcgggagtcgctgcgcgctgccttcgccccgtgccccgctccgccgccgcctcgcgccgcccgccccggctctgactgaccgcgttactcccacaggtgagcgggcgggacggcccttctcctccgggctgtaattagctgagcaagaggtaagggtttaagggatggttggttggtggggtattaatgtttaattacctggagcacctgcctgaaatcactttttttcaggttgggggattcgaacatcggccgccaccatgaacgccagcgagttcaggaggaggggcaaggagatggtggactacgtggccaactacatggagggcatcgagggcaggcaggtgtaccccgacgtggagcccggctacctgaggcccctgatccccgccgccgccccccaggagcccgacaccttcgaggacatcatcaacgacgtggagaagatcatcatgcccggcgtgacccactggcacagcccctacttcttcgcctacttccccaccgccagcagctaccccgccatgctggccgacatgctgtgcggcgccatcggctgcatcggcttcagctgggccgccagccccgcctgcaccgagctggagaccgtgatgatggactggctgggcaagatgctggagctgcccaaggccttcctgaacgagaaggccggcgagggcggcggcgtgatccagggcagcgccagcgaggccaccctggtggccctgctggccgccaggaccaaggtgatccacaggctgcaggccgccagccccgagctgacccaggccgccatcatggagaagctggtggcctacagcagcgaccaggcccacagcagcgtggagagggccggcctgatcggcggcgtgaagctgaaggccatccccagcgacggcaacttcgccatgagggccagcgccctgcaggaggccctggagagggacaaggccgccggcctgatccccttcttcatggtggccaccctgggcaccaccacctgctgcagcttcgacaacctgctggaggtgggccccatctgcaacaaggaggacatctggctgcacgtggacgccgcctacgccggcagcgccttcatctgccccgagttcaggcacctgctgaacggcgtggagttcgccgacagcttcaacttcaacccccacaagtggctgctggtgaacttcgactgcagcgccatgtgggtgaagaagaggaccgacctgaccggcgccttcaggctggaccccacctacctgaagcacagccaccaggacagcggcctgatcaccgactacaggcactggcagatccccctgggcaggaggttcaggagcctgaagatgtggttcgtgttcaggatgtacggcgtgaagggcctgcaggcctacatcaggaagcacgtgcagctgagccacgagttcgagagcctggtgaggcaggaccccaggttcgagatctgcgtggaggtgatcctgggcctggtgtgcttcaggctgaagggcagcaacaaggtgaacgaggccctgctgcagaggatcaacagcgccaagaagatccacctggtgccctgccacctgagggacaagttcgtgctgaggttcgccatctgcagcaggaccgtggagagcgcccacgtgcagagggcctgggagcacatcaaggagctggccgccgacgtgctgagggccgagagggagtgactcgagaatcaacctctggattacaaaatttgtgaaagattgactggtattcttaactatgttgctccttttacgctatgtggatacgctgctttaatgcctttgtatcatgctattgcttcccgtatggctttcattttctcctccttgtataaatcctggttgctgtctctttatgaggagttgtggcccgttgtcaggcaacgtggcgtggtgtgcactgtgtttgctgacgcaacccccactggttggggcattgccaccacctgtcagctcctttccgggactttcgctttccccctccctattgccacggcggaactcatcgccgcctgccttgcccgctgctggacaggggctcggctgttgggcactgacaattccgtggtgttgtcggggaaatcatcgtcctttccttggctgctcgcctgtgttgccacctggattctgcgcgggacgtccttctgctacgtcccttcggccctcaatccagcggaccttccttcccgcggcctgctgccggctctgcggcctcttccgcgtcttcgccttcgccctcagacgagtcggatctccctttgggccgcctccccgctaagatacattgatgagtttggacaaaccacaactagaatgcagtgaaaaaaatgctttatttgtgaaatttgtgatgctattgctttatttgtaaccattataagctgcaataaacaagttcggaccgagcggcagatctaggaacccctagtgatggagttggccactccctctctgcgcgctcgctcgctcactgaggccgggcgaccaaaggtcgcccgacgcccgggctttgcccgggcggcctcagtgagcgagcgagcgcgcagctgcctgcagg

SEQ ID NO: 23 - DNA, 4614 bp, synthetic construct
  source 1..4614: mol_type = other DNA
cctgcaggcagctgcgcgctcgctcgctcactgaggccgcccgggcaaagcccgggcgtcgggcgacctttggtcgcccggcctcagtgagcgagcgagcgcgcagagagggagtggccaactccatcactaggggttcctatcgatatccgttacataacttacggtaaatggcccgcctggctgaccgcccaacgacccccgcccattgacgtcaataatgacgtatgttcccatagtaacgtcaatagggactttccattgacgtcaatgggtggagtatttacggtaaactgcccacttggcagtacatcaagtgtatcatatgccaagtacgccccctattgacgtcaatgacggtaaatggcccgcctggcattatgcccagtacatgaccttatgggactttcctacttggcagtacatctacgtattagtcatcgctattaccatggtgatgcggttttggcagtacatcaatgggcgtggatagcggtttgactcacggggatttccaagtctccaccccattgacgtcaatgggagtttgttttgcaccaaaatcaacgggactttccaaaatgtcgtaacaactccgccccattgacgcaaatgggcggtaggcgtgtacggtgggaggtctatataagcagagctaagaggtaagggtttaagggatggttggttggtggggtattaatgtttaattacctggagcacctgcctgaaatcactttttttcaggttgggccaccatgaagttatgggatgtcgtggctgtctgcctggtgctgctccacaccgcgtccgccttcccgctgcccgccggtaagaggcctcccgaggcgcccgccgaagaccgctccctcggccgccgccgcgcgcccttcgcgctgagcagtgactcaaatatgccagaggattatcctgatcagttcgatgatgtcatggattttattcaagccaccattaaaagactgaaaaggtcaccagataaacaaatggcagtgcttcctagaagagagcggaatcggcaggctgcagctgccaacccagagaattccagaggaaaaggtcggagaggccagaggggcaaaaaccggggttgtgtcttaactgcaatacatttaaatgtcactgacttgggtctgggctatgaaaccaaggaggaactgatttttaggtactgcagcggctcttgcgatgcagctgagacaacgtacgacaaaatattgaaaaacttatccagaaatagaaggctggtgagtgacaaagtagggcaggcatgttgcagacccatcgcctttgatgatgacctgtcgtttttagatgataacctggtttaccatattctaagaaagcattccgctaaaaggtgtggatgtatctgaaataaagtctgagtgggcggcagcctgtgtgtgcctgggttctctctgtcccggaatgtgcaaacaatggaggtgaagcttcgttacataacttacggtaaatggcccgcctggctgaccgcccaacgacccccgcccattgacgtcaatagtaacgccaatagggactttccattgacgtcaatgggtggagtatttacggtaaactgcccacttggcagtacatcaagtgtatcatatgccaagtacgccccctattgacgtcaatgacggtaaatggcccgcctggcattgtgcccagtacatgaccttatgggactttcctacttggcagtacatctacgtattagtcatcgctattaccatggtcgaggtgagccccacgttctgcttcactctccccatctcccccccctccccacccccaattttgtatttatttattttttaattattttgtgcagcgatgggggcggggggggggggggggcgcgcgccaggcggggcggggcggggcgaggggcggggcggggcgaggcggagaggtgcggcggcagccaatcagagcggcgcgctccgaaagtttccttttatggcgaggcggcggcggcggcggccctataaaaagcgaagcgcgcggcgggcgggagtcgctgcgcgctgccttcgccccgtgccccgctccgccgccgcctcgcgccgcccgccccggctctgactgaccgcgttactcccacaggtgagcgggcgggacggcccttctcctccgggctgtaattagctgagcaagaggtaagggtttaagggatggttggttggtggggtattaatgtttaattacctggagcacctgcctgaaatcactttttttcaggttgggggattcgaacatcggccgccaccatgaacgccagcgagttcaggaggaggggcaaggagatggtggactacgtggccaactacatggagggcatcgagggcaggcaggtgtaccccgacgtggagcccggctacctgaggcccctgatccccgccgccgccccccaggagcccgacaccttcgaggacatcatcaacgacgtggagaagatcatcatgcccggcgtgacccactggcacagcccctacttcttcgcctacttccccaccgccagcagctaccccgccatgctggccgacatgctgtgcggcgccatcggctgcatcggcttcagctgggccgccagccccgcctgcaccgagctggagaccgtgatgatggactggctgggcaagatgctggagctgcccaaggccttcctgaacgagaaggccggcgagggcggcggcgtgatccagggcagcgccagcgaggccaccctggtggccctgctggccgccaggaccaaggtgatccacaggctgcaggccgccagccccgagctgacccaggccgccatcatggagaagctggtggcctacagcagcgaccaggcccacagcagcgtggagagggccggcctgatcggcggcgtgaagctgaaggccatccccagcgacggcaacttcgccatgagggccagcgccctgcaggaggccctggagagggacaaggccgccggcctgatccccttcttcatggtggccaccctgggcaccaccacctgctgcagcttcgacaacctgctggaggtgggccccatctgcaacaaggaggacatctggctgcacgtggacgccgcctacgccggcagcgccttcatctgccccgagttcaggcacctgctgaacggcgtggagttcgccgacagcttcaacttcaacccccacaagtggctgctggtgaacttcgactgcagcgccatgtgggtgaagaagaggaccgacctgaccggcgccttcaggctggaccccacctacctgaagcacagccaccaggacagcggcctgatcaccgactacaggcactggcagatccccctgggcaggaggttcaggagcctgaagatgtggttcgtgttcaggatgtacggcgtgaagggcctgcaggcctacatcaggaagcacgtgcagctgagccacgagttcgagagcctggtgaggcaggaccccaggttcgagatctgcgtggaggtgatcctgggcctggtgtgcttcaggctgaagggcagcaacaaggtgaacgaggccctgctgcagaggatcaacagcgccaagaagatccacctggtgccctgccacctgagggacaagttcgtgctgaggttcgccatctgcagcaggaccgtggagagcgcccacgtgcagagggcctgggagcacatcaaggagctggccgccgacgtgctgagggccgagagggagtgactcgagaatcaacctctggattacaaaatttgtgaaagattgactggtattcttaactatgttgctccttttacgctatgtggatacgctgctttaatgcctttgtatcatgctattgcttcccgtatggctttcattttctcctccttgtataaatcctggttgctgtctctttatgaggagttgtggcccgttgtcaggcaacgtggcgtggtgtgcactgtgtttgctgacgcaacccccactggttggggcattgccaccacctgtcagctcctttccgggactttcgctttccccctccctattgccacggcggaactcatcgccgcctgccttgcccgctgctggacaggggctcggctgttgggcactgacaattccgtggtgttgtcggggaaatcatcgtcctttccttggctgctcgcctgtgttgccacctggattctgcgcgggacgtccttctgctacgtcccttcggccctcaatccagcggaccttccttcccgcggcctgctgccggctctgcggcctcttccgcgtcttcgccttcgccctcagacgagtcggatctccctttgggccgcctccccgctaagatacattgatgagtttggacaaaccacaactagaatgcagtgaaaaaaatgctttatttgtgaaatttgtgatgctattgctttatttgtaaccattataagctgcaataaacaagttcggaccgagcggcagatctaggaacccctagtgatggagttggccactccctctctgcgcgctcgctcgctcactgaggccgggcgaccaaaggtcgcccgacgcccgggctttgcccgggcggcctcagtgagcgagcgagcgcgcagctgcctgcagg

SEQ ID NO: 24 - DNA, 3988 bp, synthetic construct
  source 1..3988: mol_type = other DNA
cctgcaggcagctgcgcgctcgctcgctcactgaggccgcccgggcaaagcccgggcgtcgggcgacctttggtcgcccggcctcagtgagcgagcgagcgcgcagagagggagtggccaactccatcactaggggttcctatcgatatcaagcttcgttacataacttacggtaaatggcccgcctggctgaccgcccaacgacccccgcccattgacgtcaatagtaacgccaatagggactttccattgacgtcaatgggtggagtatttacggtaaactgcccacttggcagtacatcaagtgtatcatatgccaagtacgccccctattgacgtcaatgacggtaaatggcccgcctggcattgtgcccagtacatgaccttatgggactttcctacttggcagtacatctacgtattagtcatcgctattaccatggtcgaggtgagccccacgttctgcttcactctccccatctcccccccctccccacccccaattttgtatttatttattttttaattattttgtgcagcgatgggggcggggggggggggggggcgcgcgccaggcggggcggggcggggcgaggggcggggcggggcgaggcggagaggtgcggcggcagccaatcagagcggcgcgctccgaaagtttccttttatggcgaggcggcggcggcggcggccctataaaaagcgaagcgcgcggcgggcgggagtcgctgcgcgctgccttcgccccgtgccccgctccgccgccgcctcgcgccgcccgccccggctctgactgaccgcgttactcccacaggtgagcgggcgggacggcccttctcctccgggctgtaattagctgagcaagaggtaagggtttaagggatggttggttggtggggtattaatgtttaattacctggagcacctgcctgaaatcactttttttcaggttgggggattcgaacatcggccgccaccatgaatgctagcgagtttcgcagaaggggcaaggagatggtggattacgtggctaattacatggagggcatcgagggccggcaggtgtacccagatgtggagccaggctacctgagaccactgatccctgctgccgccccacaggagccagacaccttcgaggatatcatcaatgacgtggagaagatcatcatgcctggcgtgacccactggcatagcccatacttctttgcctactttccaacagcctcttcctatcccgctatgctggctgatatgctgtgcggcgctatcggctgcatcggcttctcttgggccgctagccctgcttgcacagagctggagaccgtgatgatggattggctgggcaagatgctggagctgcctaaggcctttctgaacgagaaggctggcgagggcggcggcgtgatccagggctctgcctccgaggctacactggtggctctgctggctgcccggacaaaggtaatccacagactgcaggctgcctctccagagctgacccaggccgctatcatggagaagctggtggcttactctagcgaccaggctcattcttccgtggagcgggctggcctgatcggcggcgtgaagctgaaggccatcccttccgacggcaatttcgccatgagagcttctgccctgcaggaggctctggagagagataaggctgccggcctgatccctttctttatggtggccaccctgggcacaaccacctgttgctccttcgacaacctgctggaggtgggccctatctgtaacaaggaggacatctggctgcatgtggatgccgcttatgctggctctgcctttatctgccccgagtttagacatctgctgaacggcgtggagtttgccgacagctttaacttcaaccctcacaagtggctgctggtgaattttgactgctctgccatgtgggtgaagaagaggacagacctgaccggcgcttttaggctggatccaacctacctgaagcacagccatcaggacagcggcctgatcacagactacagacactggcagatcccactgggcagaaggtttcggtctctgaagatgtggttcgtgtttcgcatgtatggcgtgaagggcctgcaggcttatatccggaagcacgtgcagctgtctcatgagttcgagtccctggtgcggcaggacccaagatttgagatctgcgtggaggtaatcctgggcctggtgtgcttcaggctgaagggctctaataaggtgaacgaggctctgctgcagaggatcaacagcgccaagaagatccatctggtgccttgtcatctgagggacaagttcgtgctgagattcgccatctgctctagaacagtggagtctgctcatgtgcagagggcttgggagcatatcaaggagctggccgctgacgtgctgagggctgagagggaggccaccaacttctccctgctgaagcaggccggcgacgtggaggagaaccccggccccatgaagctgtgggatgtggtggccgtgtgcctggtgctgctgcacaccgcttctgccttcccactgcctgccggcaagagacctcccgaggcccctgccgaggacagaagcctgggcaggcggagagccccatttgctctgtctagcgattccaacatgcctgaggattaccccgatcagttcgatgacgtgatggatttcatccaggccaccatcaagagactgaagagatctcctgacaagcagatggctgtgctgcctagaagggagagaaacaggcaggccgctgctgccaatccagagaactccaggggcaagggcagaaggggccagcgcggcaagaatagaggctgcgtgctgacagccatccacctgaacgtgaccgacctgggcctgggctacgagaccaaggaggagctgatcttcaggtactgtagcggctcctgtgatgctgccgagaccacatacgacaagatcctgaagaacctgtccaggaacagaaggctggtgtctgacaaggtgggccaggcttgctgtaggccaatcgctttcgacgacgatctgtcctttctggatgacaacctggtgtaccacatcctgaggaagcattccgctaagagatgtggctgcatctgactcgagaatcaacctctggattacaaaatttgtgaaagattgactggtattcttaactatgttgctccttttacgctatgtggatacgctgctttaatgcctttgtatcatgctattgcttcccgtatggctttcattttctcctccttgtataaatcctggttgctgtctctttatgaggagttgtggcccgttgtcaggcaacgtggcgtggtgtgcactgtgtttgctgacgcaacccccactggttggggcattgccaccacctgtcagctcctttccgggactttcgctttccccctccctattgccacggcggaactcatcgccgcctgccttgcccgctgctggacaggggctcggctgttgggcactgacaattccgtggtgttgtcggggaaatcatcgtcctttccttggctgctcgcctgtgttgccacctggattctgcgcgggacgtccttctgctacgtcccttcggccctcaatccagcggaccttccttcccgcggcctgctgccggctctgcggcctcttccgcgtcttcgccttcgccctcagacgagtcggatctccctttgggccgcctccccgctaagatacattgatgagtttggacaaaccacaactagaatgcagtgaaaaaaatgctttatttgtgaaatttgtgatgctattgctttatttgtaaccattataagctgcaataaacaagttcggaccgagcggcagatctaggaacccctagtgatggagttggccactccctctctgcgcgctcgctcgctcactgaggccgggcgaccaaaggtcgcccgacgcccgggctttgcccgggcggcctcagtgagcgagcgagcgcgcagctgcctgcagg

SEQ ID NO: 25 - DNA, 4503 bp, synthetic construct
  source 1..4503: mol_type = other DNA
cctgcaggcagctgcgcgctcgctcgctcactgaggccgcccgggcaaagcccgggcgtcgggcgacctttggtcgcccggcctcagtgagcgagcgagcgcgcagagagggagtggccaactccatcactaggggttcctatcgatatccgttacataacttacggtaaatggcccgcctggctgaccgcccaacgacccccgcccattgacgtcaataatgacgtatgttcccatagtaacgtcaatagggactttccattgacgtcaatgggtggagtatttacggtaaactgcccacttggcagtacatcaagtgtatcatatgccaagtacgccccctattgacgtcaatgacggtaaatggcccgcctggcattatgcccagtacatgaccttatgggactttcctacttggcagtacatctacgtattagtcatcgctattaccatggtgatgcggttttggcagtacatcaatgggcgtggatagcggtttgactcacggggatttccaagtctccaccccattgacgtcaatgggagtttgttttgcaccaaaatcaacgggactttccaaaatgtcgtaacaactccgccccattgacgcaaatgggcggtaggcgtgtacggtgggaggtctatataagcagagctgtgagtttggggacccttgattgttctttctttttcgctattgtaaaattcatgttatatggagggggcaaagttttcagggtgttgtttagaatgggaagatgtcccttgtatcaccatggaccctcatgataattttgtttctttcactttctactctgttgacaaccattgtctcctcttattttcttttcattttctgtaactttttcgttaaactttagcttgcatttgtaacgaatttttaaattcacttttgtttatttgtcagattgtaagtactttctctaatcacttttttttcaaggcaatcagggtatattatattgtacttcagcacagttttagagaacaattgttataattaaatgataaggtagaatatttctgcatataaattctggctggcgtggaaatattcttattggtagaaacaactacatcctggtcatcatcctgcctttctctttatggttacaatgatatacactgtttgagatgaggataaaatactctgagtccaaaccgggcccctctgctaaccatgttcatgccttcttctttttcctacaggccaccatgaagctgtgggatgtggtggccgtgtgcctggtgctgctgcacaccgcttctgccttcccactgcctgccggcaagagacctcccgaggcccctgccgaggacagaagcctgggcaggcggagagccccatttgctctgtctagcgattccaacatgcctgaggattaccccgatcagttcgatgacgtgatggatttcatccaggccaccatcaagagactgaagagatctcctgacaagcagatggctgtgctgcctagaagggagagaaacaggcaggccgctgctgccaatccagagaactccaggggcaagggcagaaggggccagcgcggcaagaatagaggctgcgtgctgacagccatccacctgaacgtgaccgacctgggcctgggctacgagaccaaggaggagctgatcttcaggtactgtagcggctcctgtgatgctgccgagaccacatacgacaagatcctgaagaacctgtccaggaacagaaggctggtgtctgacaaggtgggccaggcttgctgtaggccaatcgctttcgacgacgatctgtcctttctggatgacaacctggtgtaccacatcctgaggaagcattccgctaagagatgtggctgcatctgaaataaagtctgagtgggcggcagcctgtgtgtgcctgggttctctctgtcccggaatgtgcaaacaatggaggtgaagcttcgttacataacttacggtaaatggcccgcctggctgaccgcccaacgacccccgcccattgacgtcaatagtaacgccaatagggactttccattgacgtcaatgggtggagtatttacggtaaactgcccacttggcagtacatcaagtgtatcatatgccaagtacgccccctattgacgtcaatgacggtaaatggcccgcctggcattgtgcccagtacatgaccttatgggactttcctacttggcagtacatctacgtattagtcatcgctattaccatggtcgaggtgagccccacgttctgcttcactctccccatctcccccccctccccacccccaattttgtatttatttattttttaattattttgtgcagcgatgggggcggggggggggggggggcgcgcgccaggcggggcggggcggggcgaggggcggggcggggcgaggcggagaggtgcggcggcagccaatcagagcggcgcgctccgaaagtttccttttatggcgaggcggcggcggcggcggccctataaaaagcgaagcgcgcggcgggcgggagtcgctgcgcgctgccttcgccccgtgccccgctccgccgccgcctcgcgccgcccgccccggctctgactgaccgcgttactcccacaggtgagcgggcgggacggcccttctcctccgggctgtaattagctgagcaagaggtaagggtttaagggatggttggttggtggggtattaatgtttaattacctggagcacctgcctgaaatcactttttttcaggttgggggattcgaacatcggccgccaccatgaatgctagcgagtttcgcagaaggggcaaggagatggtggattacgtggctaattacatggagggcatcgagggccggcaggtgtacccagatgtggagccaggctacctgagaccactgatccctgctgccgccccacaggagccagacaccttcgaggatatcatcaatgacgtggagaagatcatcatgcctggcgtgacccactggcatagcccatacttctttgcctactttccaacagcctcttcctatcccgctatgctggctgatatgctgtgcggcgctatcggctgcatcggcttctcttgggccgctagccctgcttgcacagagctggagaccgtgatgatggattggctgggcaagatgctggagctgcctaaggcctttctgaacgagaaggctggcgagggcggcggcgtgatccagggctctgcctccgaggctacactggtggctctgctggctgcccggacaaaggtaatccacagactgcaggctgcctctccagagctgacccaggccgctatcatggagaagctggtggcttactctagcgaccaggctcattcttccgtggagcgggctggcctgatcggcggcgtgaagctgaaggccatcccttccgacggcaatttcgccatgagagcttctgccctgcaggaggctctggagagagataaggctgccggcctgatccctttctttatggtggccaccctgggcacaaccacctgttgctccttcgacaacctgctggaggtgggccctatctgtaacaaggaggacatctggctgcatgtggatgccgcttatgctggctctgcctttatctgccccgagtttagacatctgctgaacggcgtggagtttgccgacagctttaacttcaaccctcacaagtggctgctggtgaattttgactgctctgccatgtgggtgaagaagaggacagacctgaccggcgcttttaggctggatccaacctacctgaagcacagccatcaggacagcggcctgatcacagactacagacactggcagatcccactgggcagaaggtttcggtctctgaagatgtggttcgtgtttcgcatgtatggcgtgaagggcctgcaggcttatatccggaagcacgtgcagctgtctcatgagttcgagtccctggtgcggcaggacccaagatttgagatctgcgtggaggtaatcctgggcctggtgtgcttcaggctgaagggctctaataaggtgaacgaggctctgctgcagaggatcaacagcgccaagaagatccatctggtgccttgtcatctgagggacaagttcgtgctgagattcgccatctgctctagaacagtggagtctgctcatgtgcagagggcttgggagcatatcaaggagctggccgctgacgtgctgagggctgagagggagctcgagtaagatacattgatgagtttggacaaaccacaactagaatgcagtgaaaaaaatgctttatttgtgaaatttgtgatgctattgctttatttgtaaccattataagctgcaataaacaagttcggaccgagcggcagatctaggaacccctagtgatggagttggccactccctctctgcgcgctcgctcgctcactgaggccgggcgaccaaaggtcgcccgacgcccgggctttgcccgggcggcctcagtgagcgagcgagcgcgcagctgcctgcagg

SEQ ID NO: 26 - DNA, 141 bp, synthetic construct
  source 1..141: mol_type = other DNA
cctgcaggcagctgcgcgctcgctcgctcactgaggccgcccgggcaaagcccgggcgtcgggcgacctttggtcgcccggcctcagtgagcgagcgagcgcgcagagagggagtggccaactccatcactaggggttcct

SEQ ID NO: 27 - DNA, 286 bp, synthetic construct
  source 1..286: mol_type = other DNA
cgttacataacttacggtaaatggcccgcctggctgaccgcccaacgacccccgcccattgacgtcaatagtaacgccaatagggactttccattgacgtcaatgggtggagtatttacggtaaactgcccacttggcagtacatcaagtgtatcatatgccaagtacgccccctattgacgtcaatgacggtaaatggcccgcctggcattgtgcccagtacatgaccttatgggactttcctacttggcagtacatctacgtattagtcatcgctattaccatg

SEQ ID NO: 28 - DNA, 278 bp, synthetic construct
  source 1..278: mol_type = other DNA
tcgaggtgagccccacgttctgcttcactctccccatctcccccccctccccacccccaattttgtatttatttattttttaattattttgtgcagcgatgggggcggggggggggggggggcgcgcgccaggcggggcggggcggggcgaggggcggggcggggcgaggcggagaggtgcggcggcagccaatcagagcggcgcgctccgaaagtttccttttatggcgaggcggcggcggcggcggccctataaaaagcgaagcgcgcggcgggcg

SEQ ID NO: 29 - DNA, 228 bp, synthetic construct
  source 1..228: mol_type = other DNA
ggagtcgctgcgcgctgccttcgccccgtgccccgctccgccgccgcctcgcgccgcccgccccggctctgactgaccgcgttactcccacaggtgagcgggcgggacggcccttctcctccgggctgtaattagctgagcaagaggtaagggtttaagggatggttggttggtggggtattaatgtttaattacctggagcacctgcctgaaatcactttttttcag

SEQ ID NO: 30 - DNA, 477 bp, synthetic construct
  source 1..477: mol_type = other DNA
gggtggcatccctgtgacccctccccagtgcctctcctggccctggaagttgccactccagtgcccaccagccttgtcctaataaaattaagttgcatcattttgtctgactaggtgtccttctataatattatggggtggaggggggtggtatggagcaaggggcaagttgggaagacaacctgtagggcctgcggggtctattgggaaccaagctggagtgcagtggcacaatcttggctcactgcaatctccgcctcctgggttcaagcgattctcctgcctcagcctcccgagttgttgggattccaggcatgcatgaccaggctcagctaatttttgtttttttggtagagacggggtttcaccatattggccaggctggtctccaactcctaatctcaggtgatctacccaccttggcctcccaaattgctgggattacaggcgtgaaccactgctcccttccctgtcctt

SEQ ID NO: 31 - DNA, 141 bp, synthetic construct
  source 1..141: mol_type = other DNA
aggaacccctagtgatggagttggccactccctctctgcgcgctcgctcgctcactgaggccgggcgaccaaaggtcgcccgacgcccgggctttgcccgggcggcctcagtgagcgagcgagcgcgcagctgcctgcagg

SEQ ID NO: 32 - DNA, 122 bp, synthetic construct
  source 1..122: mol_type = other DNA
taagatacattgatgagtttggacaaaccacaactagaatgcagtgaaaaaaatgctttatttgtgaaatttgtgatgctattgctttatttgtaaccattataagctgcaataaacaagtt

SEQ ID NO: 33 - DNA, 726 bp, synthetic construct
  source 1..726: mol_type = other DNA
ataacaggcctattgattggaaagtttgtcaacgaattgtgggtcttttggggtttgctgccccttttacgcaatgtggatatcctgctttaatgcctttatatgcatgtatacaagcaaaacaggcttttactttctcgccaacttacaaggcctttctcagtaaacagtatatgaccctttaccccgttgctcggcaacggcctggtctgtgccaagtgtttgctgacgcaacccccactggttggggcttggccataggccatcagcgcatgcgtggaacctttgtgtctcctctgccgatccatactgcggaactcctagccgcttgttttgctcgcagcaggtctggagcaaacctcatcgggaccgacaattctgtcgtactctcccgcaagtatacatcgtttccatggctgctaggctgtgctgccaactggatcctgcgcgggacgtcctttgtttacgtcccgtcggcgctgaatcccgcggacgacccctcccggggccgcttggggctctaccgcccgcttctccgtctgccgtaccgtccgaccacggggcgcacctctctttacgcggactccccgtctgtgccttctcatctgccggaccgtgtgcacttcgcttcacctctgcacgtcgcatggaggccaccgtgaacgcccaccggaacctgcccaaggtcttgcataagaggactcttggactttcagcaatgtcatc

SEQ ID NO: 34 - DNA, 589 bp, synthetic construct
  source 1..589: mol_type = other DNA
aatcaacctctggattacaaaatttgtgaaagattgactggtattcttaactatgttgctccttttacgctatgtggatacgctgctttaatgcctttgtatcatgctattgcttcccgtatggctttcattttctcctccttgtataaatcctggttgctgtctctttatgaggagttgtggcccgttgtcaggcaacgtggcgtggtgtgcactgtgtttgctgacgcaacccccactggttggggcattgccaccacctgtcagctcctttccgggactttcgctttccccctccctattgccacggcggaactcatcgccgcctgccttgcccgctgctggacaggggctcggctgttgggcactgacaattccgtggtgttgtcggggaaatcatcgtcctttccttggctgctcgcctgtgttgccacctggattctgcgcgggacgtccttctgctacgtcccttcggccctcaatccagcggaccttccttcccgcggcctgctgccggctctgcggcctcttccgcgtcttcgccttcgccctcagacgagtcggatctccctttgggccgcctccccgc

SEQ ID NO: 35 - DNA, 203 bp, synthetic construct
  source 1..203: mol_type = other DNA
gtgatgcggttttggcagtacatcaatgggcgtggatagcggtttgactcacggggatttccaagtctccaccccattgacgtcaatgggagtttgttttgcaccaaaatcaacgggactttccaaaatgtcgtaacaactccgccccattgacgcaaatgggcggtaggcgtgtacggtgggaggtctatataagcagagct

SEQ ID NO: 36 - DNA, 1268 bp, synthetic construct
  source 1..1268: mol_type = other DNA
aataaagtctgagtgggcggcagcctgtgtgtgcctgggttctctctgtcccggaatgtgcaaacaatggaggtgggcctacatcaggaagcacgtgcagctgagccacgagttcgagagcctggtgaggcaggaccccaggttcgagatctgcgtggaggtgatcctgggcctggtgtgcttcaggctgaagggcagcaacaaggtgaacgaggccctgctgcagaggatcaacagcgccaagaagatccacctggtgccctgccacctgagggacaagttcgtgctgaggttcgccatctgcagcaggaccgtggagagcgcccacgtgcagagggcctgggagcacatcaaggagctggccgccgacgtgctgagggccgagagggagtgactcgagtaagatacattgatgagtttggacaaaccacaactagaatgcagtgaaaaaaatgctttatttgtgaaatttgtgatgctattgctttatttgtaaccattataagctgcaataaacaagttcgttacataacttacggtaaatggcccgcctggctgaccgcccaacgacccccgcccattgacgtcaataatgacgtatgttcccatagtaacgtcaatagggactttccattgacgtcaatgggtggagtatttacggtaaactgcccacttggcagtacatcaagtgtatcatatgccaagtacgccccctattgacgtcaatgacggtaaatggcccgcctggcattatgcccagtacatgaccttatgggactttcctacttggcagtacatctacgtattagtcatcgctattaccatggtgatgcggttttggcagtacatcaatgggcgtggatagcggtttgactcacggggatttccaagtctccaccccattgacgtcaatgggagtttgttttgcaccaaaatcaacgggactttccaaaatgtcgtaacaactccgccccattgacgcaaatgggcggtaggcgtgtacggtgggaggtctatataagcagagctgccaccatgaagttatgggatgtcgtggctgtctgcctggtgctgctccacaccgcgtccgccttcccgctgcccgccggtaagaggcctcccgaggcgcccgccgaagaccgctccctcggccgccgccgcgcgcccttcgcgctgagcagtgactcaaatatgccagaggattatcctgatcagttcgatgatgtcatggattttattcaagccaccattaaaagactgaaaaggtc

SEQ ID NO: 37 - DNA, 304 bp, synthetic construct
  source 1..304: mol_type = other DNA
cgttacataacttacggtaaatggcccgcctggctgaccgcccaacgacccccgcccattgacgtcaataatgacgtatgttcccatagtaacgtcaatagggactttccattgacgtcaatgggtggagtatttacggtaaactgcccacttggcagtacatcaagtgtatcatatgccaagtacgccccctattgacgtcaatgacggtaaatggcccgcctggcattatgcccagtacatgaccttatgggactttcctacttggcagtacatctacgtattagtcatcgctattaccatg

SEQ ID NO: 38 - DNA, 573 bp, synthetic construct
  source 1..573: mol_type = other DNA
gtgagtttggggacccttgattgttctttctttttcgctattgtaaaattcatgttatatggagggggcaaagttttcagggtgttgtttagaatgggaagatgtcccttgtatcaccatggaccctcatgataattttgtttctttcactttctactctgttgacaaccattgtctcctcttattttcttttcattttctgtaactttttcgttaaactttagcttgcatttgtaacgaatttttaaattcacttttgtttatttgtcagattgtaagtactttctctaatcacttttttttcaaggcaatcagggtatattatattgtacttcagcacagttttagagaacaattgttataattaaatgataaggtagaatatttctgcatataaattctggctggcgtggaaatattcttattggtagaaacaactacatcctggtcatcatcctgcctttctctttatggttacaatgatatacactgtttgagatgaggataaaatactctgagtccaaaccgggcccctctgctaaccatgttcatgccttcttctttttcctacag

SEQ ID NO: 39 - DNA, 92 bp, synthetic construct
  source 1..92: mol_type = other DNA
aagaggtaagggtttaagggatggttggttggtggggtattaatgtttaattacctggagcacctgcctgaaatcactttttttcaggttgg

SEQ ID NO: 40 - DNA, 16 bp, synthetic construct
  source 1..16: mol_type = other DNA
atcgatatccgttaca

SEQ ID NO: 41 - DNA, 2208 bp, synthetic construct
  source 1..2208: mol_type = other DNA
atggctgccgatggttatcttccagattggctcgaggacactctctctgaaggaataagacagtggtggaagctcaaacctggcccaccaccaccaaagcccgcagagcggcataaggacgacagcaggggtcttgtgcttcctgggtacaagtacctcggacccttcaacggactcgacaagggagagccggtcaacgaggcagacgccgcggccctcgagcacgacaaagcctacgaccggcagctcgacagcggagacaacccgtacctcaagtacaaccacgccgacgcggagtttcaggagcgccttaaagaagatacgtcttttgggggcaacctcggacgagcagtcttccaggcgaaaaagagggttcttgaacctctgggcctggttgaggaacctgttaagacggctccgggaaaaaagaggccggtagagcactctcctgtggagccagactcctcctcgggaaccggaaaggcgggccagcagcctgcaagaaaaagattgaattttggtcagactggagacgcagactcagtacctgacccccagcctctcggacagccaccagcagccccctctggtctgggaactaatacgatggctacaggcagtggcgcaccaatggcagacaataacgagggcgccgacggagtgggtaattcctcgggaaattggcattgcgattccacatggatgggcgacagagtcatcaccaccagcacccgaacctgggccctgcccacctacaacaaccacctctacaaacaaatttccagccaatcaggagcctcgaacgacaatcactactttggctacagcaccccttgggggtattttgacttcaacagattccactgccacttttcaccacgtgactggcaaagactcatcaacaacaactggggattccgacccaagagactcaacttcaagctctttaacattcaagtcaaagaggtcacgcagaatgacggtacgacgacgattgccaataaccttaccagcacggttcaggtgtttactgactcggagtaccagctcccgtacgtcctcggctcggcgcatcaaggatgcctcccgccgttcccagcagacgtcttcatggtgccacagtatggatacctcaccctgaacaacgggagtcaggcagtaggacgctcttcattttactgcctggagtactttccttctcagatgctgcgtaccggaaacaactttaccttcagctacacttttgaggacgttcctttccacagcagctacgctcacagccagagtctggaccgtctcatgaatcctctcatcgaccagtacctgtattacttgagcagaacaaacactccaagtggaaccaccacgcagtcaaggcttcagttttctcaggccggagcgagtgacattcgggaccagtctaggaactggcttcctggaccctgttaccgccagcagcgagtatcaaagacatctgcggataacaacaacagtgaatactcgtggactggagctaccaagtaccacctcaatggcagagactctctggtgaatccgggcccggccatggcaagccacaaggacgatgaagaaaagttttttcctcagagcggggttctcatctttgggaagcaaggctcagagaaaacaaatgtggacattgaaaaggtcatgattacagacgaagaggaaatcaggacaaccaatcccgtggctacggagcagtatggttctgtatctaccaacctccagagaggcaacagacaagcagctaccgcagatgtcaacacacaaggcgttcttccaggcatggtctggcaggacagagatgtgtaccttcaggggcccatctgggcaaagattccacacacggacggacattttcacccctctcccctcatgggtggattcggacttaaacaccctcctccacagattctcatcaagaacaccccggtacctgcgaatccttcgaccaccttcagtgcggcaaagtttgcttccttcatcacacagtactccacgggacaggtcagcgtggagatcgagtgggagctgcagaaggaaaacagcaaacgctggaatcccgaaattcagtacacttccaactacaacaagtctgttaatgtggactttactgtggacactaatggcgtgtattcagagcctcgccccattggcaccagatacctgactcgtaatctgtaa

SEQ ID NO: 42 - DNA, 2211 bp, synthetic construct
  source 1..2211: mol_type = other DNA
atggctgccgatggttatcttccagattggctcgaggacaaccttagtgaaggaattcgcgagtggtgggctttgaaacctggagcccctcaacccaaggcaaatcaacaacatcaagacaacgctcgaggtcttgtgcttccgggttacaaataccttggacccggcaacggactcgacaagggggagccggtcaacgcagcagacgcggcggccctcgagcacgacaaggcctacgaccagcagctcaaggccggagacaacccgtacctcaagtacaaccacgccgacgccgagttccaggagcggctcaaagaagatacgtcttttgggggcaacctcgggcgagcagtcttccaggccaaaaagaggcttcttgaacctcttggtctggttgaggaagcggctaagacggctcctggaaagaagaggcctgtagagcagtctcctcaggaaccggactcctccgcgggtattggcaaatcgggtgcacagcccgctaaaaagagactcaatttcggtcagactggcgacacagagtcagtcccagaccctcaaccaatcggagaacctcccgcagccccctcaggtgtgggatctcttacaatggcttcaggtggtggcgcaccagtggcagacaataacgaaggtgccgatggagtgggtagttcctcgggaaattggcattgcgattcccaatggctgggggacagagtcatcaccaccagcacccgaacctgggccctgcccacctacaacaatcacctctacaagcaaatctccaacagcacatctggaggatcttcaaatgacaacgcctacttcggctacagcaccccctgggggtattttgacttcaacagattccactgccacttctcaccacgtgactggcagcgactcatcaacaacaactggggattccggcctaagcgactcaacttcaagctcttcaacattcaggtcaaagaggttacggacaacaatggagtcaagaccatcgccaataaccttaccagcacggtccaggtcttcacggactcagactatcagctcccgtacgtgctcgggtcggctcacgagggctgcctcccgccgttcccagcggacgttttcatgattcctcagtacgggtatctgacgcttaatgatggaagccaggccgtgggtcgttcgtccttttactgcctggaatatttcccgtcgcaaatgctaagaacgggtaacaacttccagttcagctacgagtttgagaacgtacctttccatagcagctacgctcacagccaaagcctggaccgactaatgaatccactcatcgaccaatacttgtactatctctcaaagactattaacggttctggacagaatcaacaaacgctaaaattcagtgtggccggacccagcaacatggctgtccagggaagaaactacatacctggacccagctaccgacaacaacgtgtctcaaccactgtgactcaaaacaacaacagcgaatttgcttggcctggagcttcttcttgggctctcaatggacgtaatagcttgatgaatcctggacctgctatggccagccacaaagaaggagaggaccgtttctttcctttgtctggatctttaatttttggcaaacaaggaactggaagagacaacgtggatgcggacaaagtcatgataaccaacgaagaagaaattaaaactactaacccggtagcaacggagtcctatggacaagtggccacaaaccaccagagtgcccaagcacaggcgcagaccggctgggttcaaaaccaaggaatacttccgggtatggtttggcaggacagagatgtgtacctgcaaggacccatttgggccaaaattcctcacacggacggcaactttcacccttctccgctgatgggagggtttggaatgaagcacccgcctcctcagatcctcatcaaaaacacacctgtacctgcggatcctccaacggccttcaacaaggacaagctgaactctttcatcacccagtattctactggccaagtcagcgtggagatcgagtgggagctgcagaaggaaaacagcaagcgctggaacccggagatccagtacacttccaactattacaagtctaataatgttgaatttgctgttaatactgaaggtgtatatagtgaaccccgccccattggcaccagatacctgactcgtaatctgtaa

SEQ ID NO: 43 - protein, 18 aa, synthetic construct
EGRGSLLTCGDVEENPGP

SEQ ID NO: 44 - protein, 19 aa, synthetic construct
ATNFSLLKQAGDVEENPGP

SEQ ID NO: 45 - protein, 20 aa, synthetic construct
QCTNYALLKLAGDVESNPGP

SEQ ID NO: 46 - protein, 22 aa, synthetic construct
VKQTLNFDLLKLAGDVESNPGP

SEQ ID NO: 47 - DNA, 54 bp, synthetic construct
  source 1..54: mol_type = other DNA
gagggcagaggcagtctgctgacatgcggtgacgtggaagagaatcccggccct

SEQ ID NO: 48 - DNA, 57 bp, synthetic construct
  source 1..57: mol_type = other DNA
gccaccaacttctccctgctgaagcaggccggcgacgtggaggagaaccccggcccc

SEQ ID NO: 49 - DNA, 60 bp, synthetic construct
  source 1..60: mol_type = other DNA
cagtgcaccaactacgccctgctgaagctggccggcgatgtggagagcaaccccgggccc

SEQ ID NO: 50 - DNA, 66 bp, synthetic construct
  source 1..66: mol_type = other DNA
gtgaaacagactttgaattttgaccttctcaagttggcgggagacgtggagtccaaccctggacct

SEQ ID NO: 51 - protein, 1356 aa, Homo sapiens
MQSKVLLAVALWLCVETRAASVGLPSVSLDLPRLSIQKDILTIKANTTLQITCRGQRDLDWLWPNNQSGSEQRVEVTECSDGLFCKTLTIPKVIGNDTGAYKCFYRETDLASVIYVYVQDYRSPFIASVSDQHGVVYITENKNKTVVIPCLGSISNLNVSLCARYPEKRFVPDGNRISWDSKKGFTIPSYMISYAGMVFCEAKINDESYQSIMYIVVVVGYRIYDVVLSPSHGIELSVGEKLVLNCTARTELNVGIDFNWEYPSSKHQHKKLVNRDLKTQSGSEMKKFLSTLTIDGVTRSDQGLYTCAASSGLMTKKNSTFVRVHEKPFVAFGSGMESLVEATVGERVRIPAKYLGYPPPEIKWYKNGIPLESNHTIKAGHVLTIMEVSERDTGNYTVILTNPISKEKQSHVVSLVVYVPPQIGEKSLISPVDSYQYGTTQTLTCTVYAIPPPHHIHWYWQLEEECANEPSQAVSVTNPYPCEEWRSVEDFQGGNKIEVNKNQFALIEGKNKTVSTLVIQAANVSALYKCEAVNKVGRGERVISFHVTRGPEITLQPDMQPTEQESVSLWCTADRSTFENLTWYKLGPQPLPIHVGELPTPVCKNLDTLWKLNATMFSNSTNDILIMELKNASLQDQGDYVCLAQDRKTKKRHCVVRQLTVLERVAPTITGNLENQTTSIGESIEVSCTASGNPPPQIMWFKDNETLVEDSGIVLKDGNRNLTIRRVRKEDEGLYTCQACSVLGCAKVEAFFIIEGAQEKTNLEIIILVGTAVIAMFFWLLLVIILRTVKRANGGELKTGYLSIVMDPDELPLDEHCERLPYDASKWEFPRDRLKLGKPLGRGAFGQVIEADAFGIDKTATCRTVAVKMLKEGATHSEHRALMSELKILIHIGHHLNVVNLLGACTKPGGPLMVIVEFCKFGNLSTYLRSKRNEFVPYKTKGARFRQGKDYVGAIPVDLKRRLDSITSSQSSASSGFVEEKSLSDVEEEEAPEDLYKDFLTLEHLICYSFQVAKGMEFLASRKCIHRDLAARNILLSEKNVVKICDFGLARDIYKDPDYVRKGDARLPLKWMAPETIFDRVYTIQSDVWSFGVLLWEIFSLGASPYPGVKIDEEFCRRLKEGTRMRAPDYTTPEMYQTMLDCWHGEPSQRPTFSELVEHLGNLLQANAQQDGKDYIVLPISETLSMEEDSGLSLPTSPVSCMEEEEVCDPKFHYDNTAGISQYLQNSKRKSRPVSVKTFEDIPLEEPEVKVIPDDNQTDSGMVLASEELKTLEDRTKLSPSFGGMVPSKSRESVASEGSNQTSGYQSGYHSDDTDTTVYSSEEAELLKLIEIGVQTGSTAQILQPDSGTTLSSPPV

SEQ ID NO: 52 - protein, 1338 aa, synthetic construct
MVSYWDTGVLLCALLSCLLLTGSSSGSKLKDPELSLKGTQHIMQAGQTLHLQCRGEAAHKWSLPEMVSKESERLSITKSACGRNGKQFCSTLTLNTAQANHTGFYSCKYLAVPTSKKKETESAIYIFISDTGRPFVEMYSEIPEIIHMTEGRELVIPCRVTSPNITVTLKKFPLDTLIPDGKRIIWDSRKGFIISNATYKEIGLLTCEATVNGHLYKTNYLTHRQTNTIIDVQISTPRPVKLLRGHTLVLNCTATTPLNTRVQMTWSYPDEKNKRASVRRRIDQSNSHANIFYSVLTIDKMQNKDKGLYTCRVRSGPSFKSVNTSVHIYDKAFITVKHRKQQVLETVAGKRSYRLSMKVKAFPSPEVVWLKDGLPATEKSARYLTRGYSLIIKDVTEEDAGNYTILLSIKQSNVFKNLTATLIVNVKPQIYEKAVSSFPDPALYPLGSRQILTCTAYGIPQPTIKWFWHPCNHNHSEARCDFCSNNEESFILDADSNMGNRIESITQRMAIIEGKNKMASTLVVADSRISGIYICIASNKVGTVGRNISFYITDVPNGFHVNLEKMPTEGEDLKLSCTVNKFLYRDVTWILLRTVNNRTMHYSISKQKMAITKEHSITLNLTIMNVSLQDSGTYACRARNVYTGEEILQKKEITIRDQEAPYLLRNLSDHTVAISSSTTLDCHANGVPEPQITWFKNNHKIQQEPGIILGPGSSTLFIERVTEEDEGVYHCKATNQKGSVESSAYLTVQGTSDKSNLELITLTCTCVAATLFWLLLTLFIRKMKRSSSEIKTDYLSIIMDPDEVPLDEQCERLPYDASKWEFARERLKLGKSLGRGAFGKVVQASAFGIKKSPTCRTVAVKMLKEGATASEYKALMTELKILTHIGHHLNVVNLLGACTKQGGPLMVIVEYCKYGNLSNYLKSKRDLFFLNKDAALHMEPKKEKMEPGLEQGKKPRLDSVTSSESFASSGFQEDKSLSDVEEEEDSDGFYKEPITMEDLISYSFQVARGMEFLSSRKCIHRDLAARNILLSENNVVKICDFGLARDIYKNPDYVRKGDTRLPLKWMAPESIFDKIYSTKSDVWSYGVLLWEIFSLGGSPYPGVQMDEDFCSRLREGMRMRAPEYSTPEIYQIMLDCWHRDPKERPRFAELVEKLGDLLQANVQQDGKDYIPINAILTGNSGFTYSTPAFSEDFFKESISAPKFNSGSSDDVRYVNAFKFMSLERIKTFEELLPNATSMFDDYQGDSSTLLASPMLKRFTWTDSKPKASLKIDLRVTSKSKESGLSDVSRPSFCHSSCGHVSEGKRRFTYDHAELERKIACCSPPPDYNSVVLYSTPPI

SEQ ID NO: 53 - protein, 642 aa, synthetic construct
SDTGRPFVEMYSEIPEIIHMTEGRELVIPCRVTSPNITVTLKKFPLDTLIPDGKRIIWDSRKGFIISNATYKEIGLLTCEATVNGHLYKTNYLTHRQTNTIIDVVLSPSHGIELSVGEKLVLNCTARTELNVGIDFNWEYPSSKHQHKKLVNRDLKTQSGSEMKKFLSTLTIDGVTRSDQGLYTCAASSGLMTKKNSTFVRVHEKGGGGSSPFIASVSDQHGVVYITENKNKTVVIPCLGSISNLNVSLCARYPEKRFVPDGNRISWDSKKGFTIPSYMISYAGMVFCEAKINDESYQSIMYIVVVVGYRIYDVVLSPSHGIELSVGEKLVLNCTARTELNVGIDFNWEYPSSKHQHKKLVNRDLKTQSGSEMKKFLSTLTIDGVTRSDQGLYTCAASSGLMTKKNSTFVRVHEKDKTHTCPPCPAPEAAGGPSVFLFPPKPKDTLMISRTPEVTCVVVDVSHEDPEVKFNWYVDGVEVHNAKTKPREEQYNSTYRVVSVLTVLHQDWLNGKEYKCKVSNKALPAPIEKTISKAKGQPREPQVYTLPPSREEMTKNQVSLTCLVKGFYPSDIAVEWESNGQPENNYKTTPPVLDSDGSFFLYSKLTVDKSRWQQGNVFSCSVMHEALHNHYTQKSLSLSPGK

SEQ ID NO: 54 - protein, 642 aa, synthetic construct
SPFIASVSDQHGVVYITENKNKTVVIPCLGSISNLNVSLCARYPEKRFVPDGNRISWDSKKGFTIPSYMISYAGMVFCEAKINDESYQSIMYIVVVVGYRIYDVVLSPSHGIELSVGEKLVLNCTARTELNVGIDFNWEYPSSKHQHKKLVNRDLKTQSGSEMKKFLSTLTIDGVTRSDQGLYTCAASSGLMTKKNSTFVRVHEKGGGGSSDTGRPFVEMYSEIPEIIHMTEGRELVIPCRVTSPNITVTLKKFPLDTLIPDGKRIIWDSRKGFIISNATYKEIGLLTCEATVNGHLYKTNYLTHRQTNTIIDVVLSPSHGIELSVGEKLVLNCTARTELNVGIDFNWEYPSSKHQHKKLVNRDLKTQSGSEMKKFLSTLTIDGVTRSDQGLYTCAASSGLMTKKNSTFVRVHEKDKTHTCPPCPAPEAAGGPSVFLFPPKPKDTLMISRTPEVTCVVVDVSHEDPEVKFNWYVDGVEVHNAKTKPREEQYNSTYRVVSVLTVLHQDWLNGKEYKCKVSNKALPAPIEKTISKAKGQPREPQVYTLPPSREEMTKNQVSLTCLVKGFYPSDIAVEWESNGQPENNYKTTPPVLDSDGSFFLYSKLTVDKSRWQQGNVFSCSVMHEALHNHYTQKSLSLSPGK

SEQ ID NO: 55 - protein, 432 aa, synthetic construct
SPFIASVSDQHGVVYITENKNKTVVIPCLGSISNLNVSLCARYPEKRFVPDGNRISWDSKKGFTIPSYMISYAGMVFCEAKINDESYQSIMYIVVVVGYRIYDVVLSPSHGIELSVGEKLVLNCTARTELNVGIDFNWEYPSSKHQHKKLVNRDLKTQSGSEMKKFLSTLTIDGVTRSDQGLYTCAASSGLMTKKNSTFVRVHEKDKTHTCPPCPAPEAAGGPSVFLFPPKPKDTLMISRTPEVTCVVVDVSHEDPEVKFNWYVDGVEVHNAKTKPREEQYNSTYRVVSVLTVLHQDWLNGKEYKCKVSNKALPAPIEKTISKAKGQPREPQVYTLPPSREEMTKNQVSLTCLVKGFYPSDIAVEWESNGQPENNYKTTPPVLDSDGSFFLYSKLTVDKSRWQQGNVFSCSVMHEALHNHYTQKSLSLSPGK

SEQ ID NO: 56 - protein, 432 aa, synthetic construct
SPFIASVSDQHGVVYITENKNKTVVIPCLGSISNLNVSLVARYPEKRFVPDGNRISWDSKKGFTIPSYMISYAGMVFCEAKINDESYQSIMYIVVVVGYRIYDVVLSPSHGIELSVGEKLVLNCTARTELNVGIDFNWEYPSSKHQHKKLVNRDLKTQSGSEMKKFLSTLTIDGVTRSDQGLYTCAASSGLMTKKNSTFVRVHEKDKTHTCPPCPAPEAAGGPSVFLFPPKPKDTLMISRTPEVTCVVVDVSHEDPEVKFNWYVDGVEVHNAKTKPREEQYNSTYRVVSVLTVLHQDWLNGKEYKCKVSNKALPAPIEKTISKAKGQPREPQVYTLPPSREEMTKNQVSLTCLVKGFYPSDIAVEWESNGQPENNYKTTPPVLDSDGSFFLYSKLTVDKSRWQQGNVFSCSVMHEALHNHYTQKSLSLSPGK

SEQ ID NO: 57 - protein, 642 aa, synthetic construct
SDTGRPFVEMYSEIPEIIHMTEGRELVIPCRVTSPNITVTLKKFPLDTLIPDGKRIIWDSRKGFIISNATYKEIGLLTCEATVNGHLYKTNYLTHRQTNTIIDVVLSPSHGIELSVGEKLVLNCTARTELNVGIDFNWEYPSSKHQHKKLVNRDLKTQSGSEMKKFLSTLTIDGVTRSDQGLYTCAASSGLMTKKNSTFVRVHEKGGGGSSPFIASVSDQHGYVYITENKNKTVVIPCLGSISNLNVSLCARYPEKRFVPDGNRISWDSKKGFTIPSYMISYAGMVFCEAKINDESYQSIMYIVVVVGYRIYDVVLSPSHGIELSVGEKLVLNCTARTELNVGIDFNWEYPSSKHQHKKLVNRDLKTQSGSEMKKFLSTLTIDGVTRSDQGLYTCAASSGLMTKKNSTFVRVHEKDKTHTCPPCPAPEAAGGPSVFLFPPKPKDTLMISRTPEVTCVVVDVSHEDPEVKFNWYVDGVEVHNAKTKPREEQYNSTYRVVSVLTVLHQDWLNGKEYKCKVSNKALPAPIEKTISKAKGQPREPQVYTLPPSREEMTKNQVSLTCLVKGFYPSDIAVEWESNGQPENNYKTTPPVLDSDGSFFLYSKLTVDKSRWQQGNVFSCSVMHEALHNHYTQKSLSLSPGK

SEQ ID NO: 58 - protein, 642 aa, synthetic construct
SDTGRPFVEMYSEIPEIIHMTEGRELVIPCRVTSPNITVTLKKFPLDTLIPDGKRIIWDSRKGFIISNATYKEIGLLTCEATVNGHLYKTNYLTHRQTNTIIDVVLSPSHGIELSVGEKLVLNCTARTELNVGIDFNWEYPSSKHQHKKLVNRDLKTQSGSEMKKFLSTLTIDGVTRSDQGLYTCAASSGLMTKKNSTFVRVHEKGGGGSSPFIASVSDQHGVVYITENKNKTVVIPCLGSISNLNVSLVARYPEKRFVPDGNRISWDSKKGFTIPSYMISYAGMVFCEAKINDESYQSIMYIVVVVGYRIYDVVLSPSHGIELSVGEKLVLNCTARTELNVGIDFNWEYPSSKHQHKKLVNRDLKTQSGSEMKKFLSTLTIDGVTRSDQGLYTCAASSGLMTKKNSTFVRVHEKDKTHTCPPCPAPEAAGGPSVFLFPPKPKDTLMISRTPEVTCVVVDVSHEDPEVKFNWYVDGVEVHNAKTKPREEQYNSTYRVVSVLTVLHQDWLNGKEYKCKVSNKALPAPIEKTISKAKGQPREPQVYTLPPSREEMTKNQVSLTCLVKGFYPSDIAVEWESNGQPENNYKTTPPVLDSDGSFFLYSKLTVDKSRWQQGNVFSCSVMHEALHNHYTQKSLSLSPGK

SEQ ID NO: 59 - protein, 642 aa, synthetic construct
SDTGRPFVEMYSEIPEIIHMTEGRELVIPCRVTSPNITVTLKKFPLDTLIPDGKRIIWDSRKGFIISNATYKEIGLLTCEATVNGHLYKTNYLTHRQTNTIIDVVLSPSHGIELSVGEKLVLNCTARTELNVGIDFNWEYPSSKHQHKKLVNRDLKTQSGSEMKKFLSTLTIDGVTRSDQGLYTCAASSGLMTKKNSTFVRVHEKGGGGSSPFIASVSDQHGVVYITENKNKTVVIPCLGSISNLNVSLCARYPEKRFVPDGNRISWDSKKGFTIPSYMISYAGYVFCEAKINDESYQSIMYIVVVVGYRIYDVVLSPSHGIELSVGEKLVLNCTARTELNVGIDFNWEYPSSKHQHKKLVNRDLKTQSGSEMKKFLSTLTIDGVTRSDQGLYTCAASSGLMTKKNSTFVRVHEKDKTHTCPPCPAPEAAGGPSVFLFPPKPKDTLMISRTPEVTCVVVDVSHEDPEVKFNWYVDGVEVHNAKTKPREEQYNSTYRVVSVLTVLHQDWLNGKEYKCKVSNKALPAPIEKTISKAKGQPREPQVYTLPPSREEMTKNQVSLTCLVKGFYPSDIAVEWESNGQPENNYKTTPPVLDSDGSFFLYSKLTVDKSRWQQGNVFSCSVMHEALHNHYTQKSLSLSPGK

SEQ ID NO: 60 - protein, 642 aa, synthetic construct
SDTGRPFVEMYSEIPEIIHMTEGRELVIPCRVTSPNITVTLKKFPLDTLIPDGKRIIWDSRKGFIISNATYKEIGLLTCEATVNGHLYKTNYLTHRQTNTIIDVVLSPSHGIELSVGEKLVLNCTARTELNVGIDFNWEYPSSKHQHKKLVNRDLKTQSGSEMKKFLSTLTIDGVTRSDQGLYTCAASSGLMTKKNSTFVRVHEKGGGGSSPFIASVSDQHGVVYITENKNKTVVIPCLGSISNLNVSLCARYPEKRFVPDGNRISWDSKKGFTIPSYMISYAGMVQCEAKINDESYQSIMYIVVVVGYRIYDVVLSPSHGIELSVGEKLVLNCTARTELNVGIDFNWEYPSSKHQHKKLVNRDLKTQSGSEMKKFLSTLTIDGVTRSDQGLYTCAASSGLMTKKNSTFVRVHEKDKTHTCPPCPAPEAAGGPSVFLFPPKPKDTLMISRTPEVTCVVVDVSHEDPEVKFNWYVDGVEVHNAKTKPREEQYNSTYRVVSVLTVLHQDWLNGKEYKCKVSNKALPAPIEKTISKAKGQPREPQVYTLPPSREEMTKNQVSLTCLVKGFYPSDIAVEWESNGQPENNYKTTPPVLDSDGSFFLYSKLTVDKSRWQQGNVFSCSVMHEALHNHYTQKSLSLSPGK

SEQ ID NO: 61 - protein, 642 aa, synthetic construct
SDTGRPFVEMYSEIPEIIHMTEGRELVIPCRVTSPNITVTLKKFPLDTLIPDGKRIIWDSRKGFIISNATYKEIGLLTCEATVNGHLYKTNYLTHRQTNTIIDVVLSPSHGIELSVGEKLVLNCTARTELNVGIDFNWEYPSSKHQHKKLVNRDLKTQSGSEMKKFLSTLTIDGVTRSDQGLYTCAASSGLMTKKNSTFVRVHEKGGGGSSPFIASVSDQHGVVYITENKNKTVVIPCLGSISNLNVSLCARYPEKRFVPDGNRISWDSKKGFTIPSYMISYAGMVFCEAKINDESYQSINYIVVVVGYRIYDVVLSPSHGIELSVGEKLVLNCTARTELNVGIDFNWEYPSSKHQHKKLVNRDLKTQSGSEMKKFLSTLTIDGVTRSDQGLYTCAASSGLMTKKNSTFVRVHEKDKTHTCPPCPAPEAAGGPSVFLFPPKPKDTLMISRTPEVTCVVVDVSHEDPEVKFNWYVDGVEVHNAKTKPREEQYNSTYRVVSVLTVLHQDWLNGKEYKCKVSNKALPAPIEKTISKAKGQPREPQVYTLPPSREEMTKNQVSLTCLVKGFYPSDIAVEWESNGQPENNYKTTPPVLDSDGSFFLYSKLTVDKSRWQQGNVFSCSVMHEALHNHYTQKSLSLSPGK

SEQ ID NO: 62 - protein, 642 aa, synthetic construct
SDTGRPFVEMYSEIPEIIHMTEGRELVIPCRVTSPNITVTLKKFPLDTLIPDGKRIIWDSRKGFIISNATYKEIGLLTCEATVNGHLYKTNYLTHRQTNTIIDVVLSPSHGIELSVGEKLVLNCTARTELNVGIDFNWEYPSSKHQHKKLVNRDLKTQSGSEMKKFLSTLTIDGVTRSDQGLYTCAASSGLMTKKNSTFVRVHEKGGGGSSPFIASVSDQHGVVYITENKNKTVVIPCLGSISNLNVSLCARYPEKRFVPDGNRISWDSKKGFTIPSYMISYAGMVFCEAKINDESYQSIMYFVVVVGYRIYDVVLSPSHGIELSVGEKLVLNCTARTELNVGIDFNWEYPSSKHQHKKLVNRDLKTQSGSEMKKFLSTLTIDGVTRSDQGLYTCAASSGLMTKKNSTFVRVHEKDKTHTCPPCPAPEAAGGPSVFLFPPKPKDTLMISRTPEVTCVVVDVSHEDPEVKFNWYVDGVEVHNAKTKPREEQYNSTYRVVSVLTVLHQDWLNGKEYKCKVSNKALPAPIEKTISKAKGQPREPQVYTLPPSREEMTKNQVSLTCLVKGFYPSDIAVEWESNGQPENNYKTTPPVLDSDGSFFLYSKLTVDKSRWQQGNVFSCSVMHEALHNHYTQKSLSLSPGK

SEQ ID NO: 63 - protein, 642 aa, synthetic construct
SDTGRPFVEMYSEIPEIIHMTEGRELVIPCRVTSPNITVTLKKFPLDTLIPDGKRIIWDSRKGFIISNATYKEIGLLTCEATVNGHLYKTNYLTHRQTNTIIDVVLSPSHGIELSVGEKLVLNCTARTELNVGIDFNWEYPSSKHQHKKLVNRDLKTQSGSEMKKFLSTLTIDGVTRSDQGLYTCAASSGLMTKKNSTFVRVHEKGGGGSSPFIASVSDQHGVVYITENKNKTVVIPCLGSISNLNVSLCARYPEKRFVPDGNRISWDSKKGFTIPSYMISYAGMVFCEAKINDESYQSIMYHVVVVGYRIYDVVLSPSHGIELSVGEKLVLNCTARTELNVGIDFNWEYPSSKHQHKKLVNRDLKTQSGSEMKKFLSTLTIDGVTRSDQGLYTCAASSGLMTKKNSTFVRVHEKDKTHTCPPCPAPEAAGGPSVFLFPPKPKDTLMISRTPEVTCVVVDVSHEDPEVKFNWYVDGVEVHNAKTKPREEQYNSTYRVVSVLTVLHQDWLNGKEYKCKVSNKALPAPIEKTISKAKGQPREPQVYTLPPSREEMTKNQVSLTCLVKGFYPSDIAVEWESNGQPENNYKTTPPVLDSDGSFFLYSKLTVDKSRWQQGNVFSCSVMHEALHNHYTQKSLSLSPGK

SEQ ID NO: 64 - protein, 642 aa, synthetic construct
SDTGRPFVEMYSEIPEIIHMTEGRELVIPCRVTSPNITVTLKKFPLDTLIPDGKRIIWDSRKGFIISNATYKEIGLLTCEATVNGHLYKTNYLTHRQTNTIIDVVLSPSHGIELSVGEKLVLNCTARTELNVGIDFNWEYPSSKHQHKKLVNRDLKTQSGSEMKKFLSTLTIDGVTRSDQGLYTCAASSGLMTKKNSTFVRVHEKGGGGSSPFIASVSDQHGVVYITENKNKTVVIPCLGSISNLNVSLCARYPEKRFVPDGNRISWDSKKGFTIPSYMISYAGMVFCEAKINDESYQSIMYIVVVIGYRIYDVVLSPSHGIELSVGEKLVLNCTARTELNVGIDFNWEYPSSKHQHKKLVNRDLKTQSGSEMKKFLSTLTIDGVTRSDQGLYTCAASSGLMTKKNSTFVRVHEKDKTHTCPPCPAPEAAGGPSVFLFPPKPKDTLMISRTPEVTCVVVDVSHEDPEVKFNWYVDGVEVHNAKTKPREEQYNSTYRVVSVLTVLHQDWLNGKEYKCKVSNKALPAPIEKTISKAKGQPREPQVYTLPPSREEMTKNQVSLTCLVKGFYPSDIAVEWESNGQPENNYKTTPPVLDSDGSFFLYSKLTVDKSRWQQGNVFSCSVMHEALHNHYTQKSLSLSPGK

SEQ ID NO: 65 - protein, 642 aa, synthetic construct
SDTGRPFVEMYSEIPEIIHMTEGRELVIPCRVTSPNITVTLKKFPLDTLIPDGKRIIWDSRKGFIISNATYKEIGLLTCEATVNGHLYKTNYLTHRQTNTIIDVVLSPSHGIELSVGEKLVLNCTARTELNVGIDFNWEYPSSKHQHKKLVNRDLKTQSGSEMKKFLSTLTIDGVTRSDQGLYTCAASSGLMTKKNSTFVRVHEKGGGGSSPFIASVSDQHGVVYITENKNKTVVIPCLGSISNLNVSLCARYPEKRFVPDGNRISWDSKKGFTIPSYMISYAGMVFCEAKINDESYQSIMYIVVVVGNRIYDVVLSPSHGIELSVGEKLVLNCTARTELNVGIDFNWEYPSSKHQHKKLVNRDLKTQSGSEMKKFLSTLTIDGVTRSDQGLYTCAASSGLMTKKNSTFVRVHEKDKTHTCPPCPAPEAAGGPSVFLFPPKPKDTLMISRTPEVTCVVVDVSHEDPEVKFNWYVDGVEVHNAKTKPREEQYNSTYRVVSVLTVLHQDWLNGKEYKCKVSNKALPAPIEKTISKAKGQPREPQVYTLPPSREEMTKNQVSLTCLVKGFYPSDIAVEWESNGQPENNYKTTPPVLDSDGSFFLYSKLTVDKSRWQQGNVFSCSVMHEALHNHYTQKSLSLSPGK

SEQ ID NO: 66 - protein, 642 aa, synthetic construct
SDTGRPFVEMYSEIPEIIHMTEGRELVIPCRVTSPNITVTLKKFPLDTLIPDGKRIIWDSRKGFIISNATYKEIGLLTCEATVNGHLYKTNYLTHRQTNTIIDVVLSPSHGIELSVGEKLVLNCTARTELNVGIDFNWEYPSSKHQHKKLVNRDLKTQSGSEMKKFLSTLTIDGVTRSDQGLYTCAASSGLMTKKNSTFVRVHEKGGGGSSPFIASVSDQHGVVYITENKNKTVVIPCLGSISNLNVSLCARYPEKRFVPDGNRISWDSKKGFTIPSYMISYAGMVFCEAKINDESYQSIMYIVVVVGYRIYDVVLSPSHGIELSVGEKLVLNCTARTELNVGIQFNWEYPSSKHQHKKLVNRDLKTQSGSEMKKFLSTLTIDGVTRSDQGLYTCAASSGLMTKKNSTFVRVHEKDKTHTCPPCPAPEAAGGPSVFLFPPKPKDTLMISRTPEVTCVVVDVSHEDPEVKFNWYVDGVEVHNAKTKPREEQYNSTYRVVSVLTVLHQDWLNGKEYKCKVSNKALPAPIEKTISKAKGQPREPQVYTLPPSREEMTKNQVSLTCLVKGFYPSDIAVEWESNGQPENNYKTTPPVLDSDGSFFLYSKLTVDKSRWQQGNVFSCSVMHEALHNHYTQKSLSLSPGK

SEQ ID NO: 67 - protein, 642 aa, synthetic construct
SDTGRPFVEMYSEIPEIIHMTEGRELVIPCRVTSPNITVTLKKFPLDTLIPDGKRIIWDSRKGFIISNATYKEIGLLTCEATVNGHLYKTNYLTHRQTNTIIDVVLSPSHGIELSVGEKLVLNCTARTELNVGIDFNWEYPSSKHQHKKLVNRDLKTQSGSEMKKFLSTLTIDGVTRSDQGLYTCAASSGLMTKKNSTFVRVHEKGGGGSSPFIASVSDQHGVVYITENKNKTVVIPCLGSISNLNVSLCARYPEKRFVPDGNRISWDSKKGFTIPSYMISYAGMVFCEAKINDESYQSIMYIVVVVGYRIYDVVLSPSHGIELSVGEKLVLNCTARTELNVGITFNWEYPSSKHQHKKLVNRDLKTQSGSEMKKFLSTLTIDGVTRSDQGLYTCAASSGLMTKKNSTFVRVHEKDKTHTCPPCPAPEAAGGPSVFLFPPKPKDTLMISRTPEVTCVVVDVSHEDPEVKFNWYVDGVEVHNAKTKPREEQYNSTYRVVSVLTVLHQDWLNGKEYKCKVSNKALPAPIEKTISKAKGQPREPQVYTLPPSREEMTKNQVSLTCLVKGFYPSDIAVEWESNGQPENNYKTTPPVLDSDGSFFLYSKLTVDKSRWQQGNVFSCSVMHEALHNHYTQKSLSLSPGK

SEQ ID NO: 68 - protein, 642 aa, synthetic construct
SDTGRPFVEMYSEIPEIIHMTEGRELVIPCRVTSPNITVTLKKFPLDTLIPDGKRIIWDSRKGFIISNATYKEIGLLTCEATVNGHLYKTNYLTHRQTNTIIDVVLSPSHGIELSVGEKLVLNCTARTELNVGIDFNWEYPSSKHQHKKLVNRDLKTQSGSEMKKFLSTLTIDGVTRSDQGLYTCAASSGLMTKKNSTFVRVHEKGGGGSSPFIASVSDQHGVVYITENKNKTVVIPCLGSISNLNVSLCARYPEKRFVPDGNRISWDSKKGFTIPSYMISYAGMVFCEAKINDESYQSIMYIVVVVGYRIYDVVLSPSHGIELSVGEKLVLNCTARTELNVGIDFNWEYPSSKHQHKKLVFRDLKTQSGSEMKKFLSTLTIDGVTRSDQGLYTCAASSGLMTKKNSTFVRVHEKDKTHTCPPCPAPEAAGGPSVFLFPPKPKDTLMISRTPEVTCVVVDVSHEDPEVKFNWYVDGVEVHNAKTKPREEQYNSTYRVVSVLTVLHQDWLNGKEYKCKVSNKALPAPIEKTISKAKGQPREPQVYTLPPSREEMTKNQVSLTCLVKGFYPSDIAVEWESNGQPENNYKTTPPVLDSDGSFFLYSKLTVDKSRWQQGNVFSCSVMHEALHNHYTQKSLSLSPGK

SEQ ID NO: 69 - protein, 642 aa, synthetic construct
SDTGRPFVEMYSEIPEIIHMTEGRELVIPCRVTSPNITVTLKKFPLDTLIPDGKRIIWDSRKGFIISNATYKEIGLLTCEATVNGHLYKTNYLTHRQTNTIIDVVLSPSHGIELSVGEKLVLNCTARTELNVGIDFNWEYPSSKHQHKKLVNRDLKTQSGSEMKKFLSTLTIDGVTRSDQGLYTCAASSGLMTKKNSTFVRVHEKGGGGSSPFIASVSDQHGVVYITENKNKTVVIPCLGSISNLNVSLCARYPEKRFVPDGNRISWDSKKGFTIPSYMISYAGMVFCEAKINDESYQSIMYIVVVVGYRIYDVVLSPSHGIELSVGEKLVLNCTARTELNVGIDFNWEYPSSKHQHKKLVIRDLKTQSGSEMKKFLSTLTIDGVTRSDQGLYTCAASSGLMTKKNSTFVRVHEKDKTHTCPPCPAPEAAGGPSVFLFPPKPKDTLMISRTPEVTCVVVDVSHEDPEVKFNWYVDGVEVHNAKTKPREEQYNSTYRVVSVLTVLHQDWLNGKEYKCKVSNKALPAPIEKTISKAKGQPREPQVYTLPPSREEMTKNQVSLTCLVKGFYPSDIAVEWESNGQPENNYKTTPPVLDSDGSFFLYSKLTVDKSRWQQGNVFSCSVMHEALHNHYTQKSLSLSPGK

SEQ ID NO: 70 - protein, 642 aa, synthetic construct
SDTGRPFVEMYSEIPEIIHMTEGRELVIPCRVTSPNITVTLKKFPLDTLIPDGKRIIWDSRKGFIISNATYKEIGLLTCEATVNGHLYKTNYLTHRQTNTIIDVVLSPSHGIELSVGEKLVLNCTARTELNVGIDFNWEYPSSKHQHKKLVNRDLKTQSGSEMKKFLSTLTIDGVTRSDQGLYTCAASSGLMTKKNSTFVRVHEKGGGGSSPFIASVSDQHGVVYITENKNKTVVIPCLGSISNLNVSLCARYPEKRFVPDGNRISWDSKKGFTIPSYMISYAGMVFCEAKINDESYQSIMYIVVVVGYRIYDVVLSPSHGIELSVGEKLVLNCTARTELNVGIDFNWEYPSSKHQHKKLVNLDLKTQSGSEMKKFLSTLTIDGVTRSDQGLYTCAASSGLMTKKNSTFVRVHEKDKTHTCPPCPAPEAAGGPSVFLFPPKPKDTLMISRTPEVTCVVVDVSHEDPEVKFNWYVDGVEVHNAKTKPREEQYNSTYRVVSVLTVLHQDWLNGKEYKCKVSNKALPAPIEKTISKAKGQPREPQVYTLPPSREEMTKNQVSLTCLVKGFYPSDIAVEWESNGQPENNYKTTPPVLDSDGSFFLYSKLTVDKSRWQQGNVFSCSVMHEALHNHYTQKSLSLSPGK

SEQ ID NO: 71 - protein, 642 aa, synthetic construct
SDTGRPFVEMYSEIPEIIHMTEGRELVIPCRVTSPNITVTLKKFPLDTLIPDGKRIIWDSRKGFIISNATYKEIGLLTCEATVNGHLYKTNYLTHRQTNTIIDVVLSPSHGIELSVGEKLVLNCTARTELNVGIDFNWEYPSSKHQHKKLVNRDLKTQSGSEMKKFLSTLTIDGVTRSDQGLYTCAASSGLMTKKNSTFVRVHEKGGGGSSPFIASVSDQHGVVYITENKNKTVVIPCLGSISNLNVSLCARYPEKRFVPDGNRISWDSKKGFTIPSYMISYAGMVFCEAKINDESYQSIMYIVVVVGYRIYDVVLSPSHGIELSVGEKLVLNCTARTELNVGIDFNWEYPSSKHQHKKLVNEDLKTQSGSEMKKFLSTLTIDGVTRSDQGLYTCAASSGLMTKKNSTFVRVHEKDKTHTCPPCPAPEAAGGPSVFLFPPKPKDTLMISRTPEVTCVVVDVSHEDPEVKFNWYVDGVEVHNAKTKPREEQYNSTYRVVSVLTVLHQDWLNGKEYKCKVSNKALPAPIEKTISKAKGQPREPQVYTLPPSREEMTKNQVSLTCLVKGFYPSDIAVEWESNGQPENNYKTTPPVLDSDGSFFLYSKLTVDKSRWQQGNVFSCSVMHEALHNHYTQKSLSLSPGK

SEQ ID NO: 72 - protein, 642 aa, synthetic construct
SDTGRPFVEMYSEIPEIIHMTEGRELVIPCRVTSPNITVTLKKFPLDTLIPDGKRIIWDSRKGFIISNATYKEIGLLTCEATVNGHLYKTNYLTHRQTNTIIDVVLSPSHGIELSVGEKLVLNCTARTELNVGIDFNWEYPSSKHQHKKLVNRDLKTQSGSEMKKFLSTLTIDGVTRSDQGLYTCAASSGLMTKKNSTFVRVHEKGGGGSSPFIASVSDQHGVVYITENKNKTVVIPCLGSISNLNVSLCARYPEKRFVPDGNRISWDSKKGFTIPSYMISYAGMVFCEAKINDESYQSIMYIVVVVGYRIYDVVLSPSHGIELSVGEKLVLNCTARTELNVGIDFNWEYPSSKHQHKKLVNRQLKTQSGSEMKKFLSTLTIDGVTRSDQGLYTCAASSGLMTKKNSTFVRVHEKDKTHTCPPCPAPEAAGGPSVFLFPPKPKDTLMISRTPEVTCVVVDVSHEDPEVKFNWYVDGVEVHNAKTKPREEQYNSTYRVVSVLTVLHQDWLNGKEYKCKVSNKALPAPIEKTISKAKGQPREPQVYTLPPSREEMTKNQVSLTCLVKGFYPSDIAVEWESNGQPENNYKTTPPVLDSDGSFFLYSKLTVDKSRWQQGNVFSCSVMHEALHNHYTQKSLSLSPGK

SEQ ID NO: 73 - protein, 642 aa, synthetic construct
SDTGRPFVEMYSEIPEIIHMTEGRELVIPCRVTSPNITVTLKKFPLDTLIPDGKRIIWDSRKGFIISNATYKEIGLLTCEATVNGHLYKTNYLTHRQTNTIIDVVLSPSHGIELSVGEKLVLNCTARTELNVGIDFNWEYPSSKHQHKKLVNRDLKTQSGSEMKKFLSTLTIDGVTRSDQGLYTCAASSGLMTKKNSTFVRVHEKGGGGSSPFIASVSDQHGVVYITENKNKTVVIPCLGSISNLNVSLCARYPEKRFVPDGNRISWDSKKGFTIPSYMISYAGMVFCEAKINDESYQSIMYIVVVVGYRIYDVVLSPSHGIELSVGEKLVLNCTARTELNVGIDFNWEYPSSKHQHKKLVNRDRKTQSGSEMKKFLSTLTIDGVTRSDQGLYTCAASSGLMTKKNSTFVRVHEKDKTHTCPPCPAPEAAGGPSVFLFPPKPKDTLMISRTPEVTCVVVDVSHEDPEVKFNWYVDGVEVHNAKTKPREEQYNSTYRVVSVLTVLHQDWLNGKEYKCKVSNKALPAPIEKTISKAKGQPREPQVYTLPPSREEMTKNQVSLTCLVKGFYPSDIAVEWESNGQPENNYKTTPPVLDSDGSFFLYSKLTVDKSRWQQGNVFSCSVMHEALHNHYTQKSLSLSPGK

SEQ ID NO: 74 - protein, 642 aa, synthetic construct
SDTGRPFVEMYSEIPEIIHMTEGRELVIPCRVTSPNITVTLKKFPLDTLIPDGKRIIWDSRKGFIISNATYKEIGLLTCEATVNGHLYKTNYLTHRQTNTIIDVVLSPSHGIELSVGEKLVLNCTARTELNVGIDFNWEYPSSKHQHKKLVNRDLKTQSGSEMKKFLSTLTIDGVTRSDQGLYTCAASSGLMTKKNSTFVRVHEKGGGGSSPFIASVSDQHGVVYITENKNKTVVIPCLGSISNLNVSLCARYPEKRFVPDGNRISWDSKKGFTIPSYMISYAGMVFCEAKINDESYQSIMYIVVVVGYRIYDVVLSPSHGIELSVGEKLVLNCTARTELNVGIDFNWEYPSSKHQHKKLVNRDLDTQSGSEMKKFLSTLTIDGVTRSDQGLYTCAASSGLMTKKNSTFVRVHEKDKTHTCPPCPAPEAAGGPSVFLFPPKPKDTLMISRTPEVTCVVVDVSHEDPEVKFNWYVDGVEVHNAKTKPREEQYNSTYRVVSVLTVLHQDWLNGKEYKCKVSNKALPAPIEKTISKAKGQPREPQVYTLPPSREEMTKNQVSLTCLVKGFYPSDIAVEWESNGQPENNYKTTPPVLDSDGSFFLYSKLTVDKSRWQQGNVFSCSVMHEALHNHYTQKSLSLSPGK

SEQ ID NO: 75 - protein, 642 aa, synthetic construct
SDTGRPFVEMYSEIPEIIHMTEGRELVIPCRVTSPNITVTLKKFPLDTLIPDGKRIIWDSRKGFIISNATYKEIGLLTCEATVNGHLYKTNYLTHRQTNTIIDVVLSPSHGIELSVGEKLVLNCTARTELNVGIDFNWEYPSSKHQHKKLVNRDLKTQSGSEMKKFLSTLTIDGVTRSDQGLYTCAASSGLMTKKNSTFVRVHEKGGGGSSPFIASVSDQHGVVYITENKNKTVVIPCLGSISNLNVSLCARYPEKRFVPDGNRISWDSKKGFTIPSYMISYAGMVFCEAKINDESYQSIMYIVVVVGYRIYDVVLSPSHGIELSVGEKLVLNCTARTELNVGIDFNWEYPSSKHQHKKLVNRDLSTQSGSEMKKFLSTLTIDGVTRSDQGLYTCAASSGLMTKKNSTFVRVHEKDKTHTCPPCPAPEAAGGPSVFLFPPKPKDTLMISRTPEVTCVVVDVSHEDPEVKFNWYVDGVEVHNAKTKPREEQYNSTYRVVSVLTVLHQDWLNGKEYKCKVSNKALPAPIEKTISKAKGQPREPQVYTLPPSREEMTKNQVSLTCLVKGFYPSDIAVEWESNGQPENNYKTTPPVLDSDGSFFLYSKLTVDKSRWQQGNVFSCSVMHEALHNHYTQKSLSLSPGK

SEQ ID NO: 76 - protein, 642 aa, synthetic construct
SDTGRPFVEMYSEIPEIIHMTEGRELVIPCRVTSPNITVTLKKFPLDTLIPDGKRIIWDSRKGFIISNATYKEIGLLTCEATVNGHLYKTNYLTHRQTNTIIDVVLSPSHGIELSVGEKLVLNCTARTELNVGIDFNWEYPSSKHQHKKLVNRDLKTQSGSEMKKFLSTLTIDGVTRSDQGLYTCAASSGLMTKKNSTFVRVHEKGGGGSSPFIASVSDQHGVVYITENKNKTVVIPCLGSISNLNVSLCARYPEKRFVPDGNRISWDSKKGFTIPSYMISYAGMVFCEAKINDESYQSIMYIVVVVGYRIYDVVLSPSHGIELSVGEKLVLNCTARTELNVGIDFNWEYPSSKHQHKKLVNRDLETQSGSEMKKFLSTLTIDGVTRSDQGLYTCAASSGLMTKKNSTFVRVHEKDKTHTCPPCPAPEAAGGPSVFLFPPKPKDTLMISRTPEVTCVVVDVSHEDPEVKFNWYVDGVEVHNAKTKPREEQYNSTYRVVSVLTVLHQDWLNGKEYKCKVSNKALPAPIEKTISKAKGQPREPQVYTLPPSREEMTKNQVSLTCLVKGFYPSDIAVEWESNGQPENNYKTTPPVLDSDGSFFLYSKLTVDKSRWQQGNVFSCSVMHEALHNHYTQKSLSLSPGK

SEQ ID NO: 77 - protein, 642 aa, synthetic construct
SDTGRPFVEMYSEIPEIIHMTEGRELVIPCRVTSPNITVTLKKFPLDTLIPDGKRIIWDSRKGFIISNATYKEIGLLTCEATVNGHLYKTNYLTHRQTNTIIDVVLSPSHGIELSVGEKLVLNCTARTELNVGIDFNWEYPSSKHQHKKLVNRDLKTQSGSEMKKFLSTLTIDGVTRSDQGLYTCAASSGLMTKKNSTFVRVHEKGGGGSSPFIASVSDQHGVVYITENKNKTVVIPCLGSISNLNVSLCARYPEKRFVPDGNRISWDSKKGFTIPSYMISYAGMVFCEAKINDESYQSIMYIVVVVGYRIYDVVLSPSHGIELSVGEKLVLNCTARTELNVGIDFNWEYPSSKHQHKKLVNRDLKTESGSEMKKFLSTLTIDGVTRSDQGLYTCAASSGLMTKKNSTFVRVHEKDKTHTCPPCPAPEAAGGPSVFLFPPKPKDTLMISRTPEVTCVVVDVSHEDPEVKFNWYVDGVEVHNAKTKPREEQYNSTYRVVSVLTVLHQDWLNGKEYKCKVSNKALPAPIEKTISKAKGQPREPQVYTLPPSREEMTKNQVSLTCLVKGFYPSDIAVEWESNGQPENNYKTTPPVLDSDGSFFLYSKLTVDKSRWQQGNVFSCSVMHEALHNHYTQKSLSLSPGK

SEQ ID NO: 78 - protein, 642 aa, synthetic construct
SDTGRPFVEMYSEIPEIIHMTEGRELVIPCRVTSPNITVTLKKFPLDTLIPDGKRIIWDSRKGFIISNATYKEIGLLTCEATVNGHLYKTNYLTHRQTNTIIDVVLSPSHGIELSVGEKLVLNCTARTELNVGIDFNWEYPSSKHQHKKLVNRDLKTQSGSEMKKFLSTLTIDGVTRSDQGLYTCAASSGLMTKKNSTFVRVHEKGGGGSSPFIASVSDQHGVVYITENKNKTVVIPCLGSISNLNVSLCARYPEKRFVPDGNRISWDSKKGFTIPSYMISYAGMVFCEAKINDESYQSIMYIVVVVGYRIYDVVLSPSHGIELSVGEKLVLNCTARTELNVGIDFNWEYPSSKHQHKKLVNRDLKTQSGTEMKKFLSTLTIDGVTRSDQGLYTCAASSGLMTKKNSTFVRVHEKDKTHTCPPCPAPEAAGGPSVFLFPPKPKDTLMISRTPEVTCVVVDVSHEDPEVKFNWYVDGVEVHNAKTKPREEQYNSTYRVVSVLTVLHQDWLNGKEYKCKVSNKALPAPIEKTISKAKGQPREPQVYTLPPSREEMTKNQVSLTCLVKGFYPSDIAVEWESNGQPENNYKTTPPVLDSDGSFFLYSKLTVDKSRWQQGNVFSCSVMHEALHNHYTQKSLSLSPGK

SEQ ID NO: 79 - protein, 642 aa, synthetic construct
SDTGRPFVEMYSEIPEIIHMTEGRELVIPCRVTSPNITVTLKKFPLDTLIPDGKRIIWDSRKGFIISNATYKEIGLLTCEATVNGHLYKTNYLTHRQTNTIIDVVLSPSHGIELSVGEKLVLNCTARTELNVGIDFNWEYPSSKHQHKKLVNRDLKTQSGSEMKKFLSTLTIDGVTRSDQGLYTCAASSGLMTKKNSTFVRVHEKGGGGSSPFIASVSDQHGVVYITENKNKTVVIPCLGSISNLNVSLCARYPEKRFVPDGNRISWDSKKGFTIPSYMISYAGMVFCEAKINDESYQSIMYIVVVVGYRIYDVVLSPSHGIELSVGEKLVLNCTARTELNVGIDFNWEYPSSKHQHKKLVNRDLKTQSGSHMKKFLSTLTIDGVTRSDQGLYTCAASSGLMTKKNSTFVRVHEKDKTHTCPPCPAPEAAGGPSVFLFPPKPKDTLMISRTPEVTCVVVDVSHEDPEVKFNWYVDGVEVHNAKTKPREEQYNSTYRVVSVLTVLHQDWLNGKEYKCKVSNKALPAPIEKTISKAKGQPREPQVYTLPPSREEMTKNQVSLTCLVKGFYPSDIAVEWESNGQPENNYKTTPPVLDSDGSFFLYSKLTVDKSRWQQGNVFSCSVMHEALHNHYTQKSLSLSPGK

SEQ ID NO: 80 - protein, 642 aa, synthetic construct
SDTGRPFVEMYSEIPEIIHMTEGRELVIPCRVTSPNITVTLKKFPLDTLIPDGKRIIWDSRKGFIISNATYKEIGLLTCEATVNGHLYKTNYLTHRQTNTIIDVVLSPSHGIELSVGEKLVLNCTARTELNVGIDFNWEYPSSKHQHKKLVNRDLKTQSGSEMKKFLSTLTIDGVTRSDQGLYTCAASSGLMTKKNSTFVRVHEKGGGGSSPFIASVSDQHGVVYITENKNKTVVIPCLGSISNLNVSLCARYPEKRFVPDGNRISWDSKKGFTIPSYMISYAGMVFCEAKINDESYQSIMYIVVVVGYRIYDVVLSPSHGIELSVGEKLVLNCTARTELNVGIDFNWEYPSSKHQHKKLVNRDLKTQSGSEMKKYLSTLTIDGVTRSDQGLYTCAASSGLMTKKNSTFVRVHEKDKTHTCPPCPAPEAAGGPSVFLFPPKPKDTLMISRTPEVTCVVVDVSHEDPEVKFNWYVDGVEVHNAKTKPREEQYNSTYRVVSVLTVLHQDWLNGKEYKCKVSNKALPAPIEKTISKAKGQPREPQVYTLPPSREEMTKNQVSLTCLVKGFYPSDIAVEWESNGQPENNYKTTPPVLDSDGSFFLYSKLTVDKSRWQQGNVFSCSVMHEALHNHYTQKSLSLSPGK

SEQ ID NO: 81 - protein, 642 aa, synthetic construct
SDTGRPFVEMYSEIPEIIHMTEGRELVIPCRVTSPNITVTLKKFPLDTLIPDGKRIIWDSRKGFIISNATYKEIGLLTCEATVNGHLYKTNYLTHRQTNTIIDVVLSPSHGIELSVGEKLVLNCTARTELNVGIDFNWEYPSSKHQHKKLVNRDLKTQSGSEMKKFLSTLTIDGVTRSDQGLYTCAASSGLMTKKNSTFVRVHEKGGGGSSPFIASVSDQHGVVYITENKNKTVVIPCLGSISNLNVSLCARYPEKRFVPDGNRISWDSKKGFTIPSYMISYAGMVFCEAKINDESYQSIMYIVVVVGYRIYDVVLSPSHGIELSVGEKLVLNCTARTELNVGIDFNWEYPSSKHQHKKLVNRDLKTQSGSEMKKFYSTLTIDGVTRSDQGLYTCAASSGLMTKKNSTFVRVHEKDKTHTCPPCPAPEAAGGPSVFLFPPKPKDTLMISRTPEVTCVVVDVSHEDPEVKFNWYVDGVEVHNAKTKPREEQYNSTYRVVSVLTVLHQDWLNGKEYKCKVSNKALPAPIEKTISKAKGQPREPQVYTLPPSREEMTKNQVSLTCLVKGFYPSDIAVEWESNGQPENNYKTTPPVLDSDGSFFLYSKLTVDKSRWQQGNVFSCSVMHEALHNHYTQKSLSLSPGK

SEQ ID NO: 82 - protein, 642 aa, synthetic construct
SDTGRPFVEMYSEIPEIIHMTEGRELVIPCRVTSPNITVTLKKFPLDTLIPDGKRIIWDSRKGFIISNATYKEIGLLTCEATVNGHLYKTNYLTHRQTNTIIDVVLSPSHGIELSVGEKLVLNCTARTELNVGIDFNWEYPSSKHQHKKLVNRDLKTQSGSEMKKFLSTLTIDGVTRSDQGLYTCAASSGLMTKKNSTFVRVHEKGGGGSSPFIASVSDQHGVVYITENKNKTVVIPCLGSISNLNVSLCARYPEKRFVPDGNRISWDSKKGFTIPSYMISYAGMVFCEAKINDESYQSIMYIVVVVGYRIYDVVLSPSHGIELSVGEKLVLNCTARTELNVGIDFNWEYPSSKHQHKKLVNRDLKTQSGSEMKKFLSTLTIDGVTRSDQGLYTCAASSGYMTKKNSTFVRVHEKDKTHTCPPCPAPEAAGGPSVFLFPPKPKDTLMISRTPEVTCVVVDVSHEDPEVKFNWYVDGVEVHNAKTKPREEQYNSTYRVVSVLTVLHQDWLNGKEYKCKVSNKALPAPIEKTISKAKGQPREPQVYTLPPSREEMTKNQVSLTCLVKGFYPSDIAVEWESNGQPENNYKTTPPVLDSDGSFFLYSKLTVDKSRWQQGNVFSCSVMHEALHNHYTQKSLSLSPGK

SEQ ID NO: 83 - protein, 642 aa, synthetic construct
SDTGRPFVEMYSEIPEIIHMTEGRELVIPCRVTSPNITVTLKKFPLDTLIPDGKRIIWDSRKGFIISNATYKEIGLLTCEATVNGHLYKTNYLTHRQTNTIIDVVLSPSHGIELSVGEKLVLNCTARTELNVGIDFNWEYPSSKHQHKKLVNRDLKTQSGSEMKKFLSTLTIDGVTRSDQGLYTCAASSGLMTKKNSTFVRVHEKGGGGSSPFIASVSDQHGVVYITENKNKTVVIPCLGSISNLNVSLCARYPEKRFVPDGNRISWDSKKGFTIPSYMISYAGMVFCEAKINDESYQSIMYIVVVVGYRIYDVVLSPSHGIELSVGEKLVLNCTARTELNVGIDFNWEYPSSKHQHKKLVNRDLKTQSGSEMKKFLSTLTIDGVTRSDQGLYTCAASSGLSTKKNSTFVRVHEKDKTHTCPPCPAPEAAGGPSVFLFPPKPKDTLMISRTPEVTCVVVDVSHEDPEVKFNWYVDGVEVHNAKTKPREEQYNSTYRVVSVLTVLHQDWLNGKEYKCKVSNKALPAPIEKTISKAKGQPREPQVYTLPPSREEMTKNQVSLTCLVKGFYPSDIAVEWESNGQPENNYKTTPPVLDSDGSFFLYSKLTVDKSRWQQGNVFSCSVMHEALHNHYTQKSLSLSPGK

SEQ ID NO: 84 - protein, 642 aa, synthetic construct
SDTGRPFVEMYSEIPEIIHMTEGRELVIPCRVTSPNITVTLKKFPLDTLIPDGKRIIWDSRKGFIISNATYKEIGLLTCEATVNGHLYKTNYLTHRQTNTIIDVVLSPSHGIELSVGEKLVLNCTARTELNVGIDFNWEYPSSKHQHKKLVNRDLKTQSGSEMKKFLSTLTIDGVTRSDQGLYTCAASSGLMTKKNSTFVRVHEKGGGGSSPFIASVSDQHGVVYITENKNKTVVIPCLGSISNLNVSLCARYPEKRFVPDGNRISWDSKKGFTIPSYMISYAGMVFCEAKINDESYQSIMYIVVVVGYRIYDVVLSPSHGIELSVGEKLVLNCTARTELNVGIDFNWEYPSSKHQHKKLVNRDLKTQSGSEMKKFLSTLTIDGVTRSDQGLYTCAASSGLQTKKNSTFVRVHEKDKTHTCPPCPAPEAAGGPSVFLFPPKPKDTLMISRTPEVTCVVVDVSHEDPEVKFNWYVDGVEVHNAKTKPREEQYNSTYRVVSVLTVLHQDWLNGKEYKCKVSNKALPAPIEKTISKAKGQPREPQVYTLPPSREEMTKNQVSLTCLVKGFYPSDIAVEWESNGQPENNYKTTPPVLDSDGSFFLYSKLTVDKSRWQQGNVFSCSVMHEALHNHYTQKSLSLSPGK

SEQ ID NO: 85 - protein, 642 aa, synthetic construct
SDTGRPFVEMYSEIPEIIHMTEGRELVIPCRVTSPNITVTLKKFPLDTLIPDGKRIIWDSRKGFIISNATYKEIGLLTCEATVNGHLYKTNYLTHRQTNTIIDVVLSPSHGIELSVGEKLVLNCTARTELNVGIDFNWEYPSSKHQHKKLVNRDLKTQSGSEMKKFLSTLTIDGVTRSDQGLYTCAASSGLMTKKNSTFVRVHEKGGGGSSPFIASVSDQHGVVYITENKNKTVVIPCLGSISNLNVSLCARYPEKRFVPDGNRISWDSKKGFTIPSYMISYAGMVFCEAKINDESYQSIMYIVVVVGNRIYDVVLSPSHGIELSVGEKLVLNCTARTELNVGIDFNWEYPSSKHQHKKLVNRDLKTQSGSEMKKFLSTLTIDGVTRSDQGLYTCAASSGLQTKKNSTFVRVHEKDKTHTCPPCPAPEAAGGPSVFLFPPKPKDTLMISRTPEVTCVVVDVSHEDPEVKFNWYVDGVEVHNAKTKPREEQYNSTYRVVSVLTVLHQDWLNGKEYKCKVSNKALPAPIEKTISKAKGQPREPQVYTLPPSREEMTKNQVSLTCLVKGFYPSDIAVEWESNGQPENNYKTTPPVLDSDGSFFLYSKLTVDKSRWQQGNVFSCSVMHEALHNHYTQKSLSLSPGK

SEQ ID NO: 86 - protein, 642 aa, synthetic construct
SDTGRPFVEMYSEIPEIIHMTEGRELVIPCRVTSPNITVTLKKFPLDTLIPDGKRIIWDSRKGFIISNATYKEIGLLTCEATVNGHLYKTNYLTHRQTNTIIDVVLSPSHGIELSVGEKLVLNCTARTELNVGIDFNWEYPSSKHQHKKLVNRDLKTQSGSEMKKFLSTLTIDGVTRSDQGLYTCAASSGLMTKKNSTFVRVHEKGGGGSSPFIASVSDQHGVVYITENKNKTVVIPCLGSISNLNVSLCARYPEKRFVPDGNRISWDSKKGFTIPSYMISYAGMVFCEAKINDESYQSIMYIVVVVGYRIYDVVLSPSHGIELSVGEKLVLNCTARTELNVGIDFNWEYPSSKHQHKKLVNRDRKTQSGSEMKKFYSTLTIDGVTRSDQGLYTCAASSGLMTKKNSTFVRVHEKDKTHTCPPCPAPEAAGGPSVFLFPPKPKDTLMISRTPEVTCVVVDVSHEDPEVKFNWYVDGVEVHNAKTKPREEQYNSTYRVVSVLTVLHQDWLNGKEYKCKVSNKALPAPIEKTISKAKGQPREPQVYTLPPSREEMTKNQVSLTCLVKGFYPSDIAVEWESNGQPENNYKTTPPVLDSDGSFFLYSKLTVDKSRWQQGNVFSCSVMHEALHNHYTQKSLSLSPGK

SEQ ID NO: 87 - protein, 642 aa, synthetic construct
SDTGRPFVEMYSEIPEIIHMTEGRELVIPCRVTSPNITVTLKKFPLDTLIPDGKRIIWDSRKGFIISNATYKEIGLLTCEATVNGHLYKTNYLTHRQTNTIIDVVLSPSHGIELSVGEKLVLNCTARTELNVGIDFNWEYPSSKHQHKKLVNRDLKTQSGSEMKKFLSTLTIDGVTRSDQGLYTCAASSGLMTKKNSTFVRVHEKGGGGSSPFIASVSDQHGVVYITENKNKTVVIPCLGSISNLNVSLCARYPEKRFVPDGNRISWDSKKGFTIPSYMISYAGMVFCEAKINDESYQSIMYIVVVVGSKIYDVVLSPSHGIELSVGEKLVLNCTARTELNVGIDFNWEYPSSKHQHKKLVNRDLKTQSGSEMKKFLSTLTIDGVTRSDQGLYTCAASSGLMTKKNSTFVRVHEKDKTHTCPPCPAPEAAGGPSVFLFPPKPKDTLMISRTPEVTCVVVDVSHEDPEVKFNWYVDGVEVHNAKTKPREEQYNSTYRVVSVLTVLHQDWLNGKEYKCKVSNKALPAPIEKTISKAKGQPREPQVYTLPPSREEMTKNQVSLTCLVKGFYPSDIAVEWESNGQPENNYKTTPPVLDSDGSFFLYSKLTVDKSRWQQGNVFSCSVMHEALHNHYTQKSLSLSPGK

SEQ ID NO: 88 - protein, 642 aa, synthetic construct
SDTGRPFVEMYSEIPEIIHMTEGRELVIPCRVTSPNITVTLKKFPLDTLIPDGKRIIWDSRKGFIISNATYKEIGLLTCEATVNGHLYKTNYLTHRQTNTIIDVVLSPSHGIELSVGEKLVLNCTARTELNVGIDFNWEYPSSKHQHKKLVNRDLKTQSGSEMKKFLSTLTIDGVTRSDQGLYTCAASSGLMTKKNSTFVRVHEKGGGGSSPFIASVSDQHGVVYITENKNKTVVIPCLGSISNLNVSLCARYPEKRFVPDGNRISWDSKKGFTIPSYMISYAGMVFCEAKINDESYQSIMYIVVVVGYRIYDVVLSPSHGIELSVGEKLVLNCTARTELNVGIDFNWEYPSSKHQHKKLVNRDLKTQSGSEMKKFLSTLTIDGVTRSDQGLYTCAASSGRMTKKNSTFVRVHEKDKTHTCPPCPAPEAAGGPSVFLFPPKPKDTLMISRTPEVTCVVVDVSHEDPEVKFNWYVDGVEVHNAKTKPREEQYNSTYRVVSVLTVLHQDWLNGKEYKCKVSNKALPAPIEKTISKAKGQPREPQVYTLPPSREEMTKNQVSLTCLVKGFYPSDIAVEWESNGQPENNYKTTPPVLDSDGSFFLYSKLTVDKSRWQQGNVFSCSVMHEALHNHYTQKSLSLSPGK

SEQ ID NO: 89 - protein, 642 aa, synthetic construct
SDTGRPFVEMYSEIPEIIHMTEGRELVIPCRVTSPNITVTLKKFPLDTLIPDGKRIIWDSRKGFIISNATYKEIGLLTCEATVNGHLYKTNYLTHRQTNTIIDVVLSPSHGIELSVGEKLVLNCTARTELNVGIDFNWEYPSSKHQHKKLVNRDLKTQSGSEMKKFLSTLTIDGVTRSDQGLYTCAASSGLMTKKNSTFVRVHEKGGGGSSPFIASVSDQHGVVYITENKNKTVVIPCLGSISNLNVSLCARYPEKRFVPDGNRISWDSKKGFTIPSYMISYAGMVFCEAKINDESYQSIMYIVVVVGYRIYDVVLSPSHGIELSVGEKLVLQCTARTELNVGIDFNWEYPSSKHQHKKLVNRDLKTQSGSEMKKFLSTLTIDGVTRSDQGLYTCAASSGLMTKKNSTFVRVHEKDKTHTCPPCPAPEAAGGPSVFLFPPKPKDTLMISRTPEVTCVVVDVSHEDPEVKFNWYVDGVEVHNAKTKPREEQYNSTYRVVSVLTVLHQDWLNGKEYKCKVSNKALPAPIEKTISKAKGQPREPQVYTLPPSREEMTKNQVSLTCLVKGFYPSDIAVEWESNGQPENNYKTTPPVLDSDGSFFLYSKLTVDKSRWQQGNVFSCSVMHEALHNHYTQKSLSLSPGK

SEQ ID NO: 90 - protein, 642 aa, synthetic construct
SDTGRPFVEMYSEIPEIIHMTEGRELVIPCRVTSPNITVTLKKFPLDTLIPDGKRIIWDSRKGFIISNATYKEIGLLTCEATVNGHLYKTNYLTHRQTNTIIDVVLSPSHGIELSVGEKLVLNCTARTELNVGIDFNWEYPSSKHQHKKLVNRDLKTQSGSEMKKFLSTLTIDGVTRSDQGLYTCAASSGLMTKKNSTFVRVHEKGGGGSSPFIASVSDQHGVVYITENKNKTVVIPCLGSISNLNVSLVARYPEKRFVPDGNRISWDSKKGFTIPSYMISYAGMVFCEAKINDESYQSIMYIVVVVGYRIYDVVLSPSHGIELSVGEKLVLNCTARTELNVGIDFNWEYPSSKHQHKKLVFRDLKTQSGSEMKKFLSTLTIDGVTRSDQGLYTCAASSGLMTKKNSTFVRVHEKDKTHTCPPCPAPEAAGGPSVFLFPPKPKDTLMISRTPEVTCVVVDVSHEDPEVKFNWYVDGVEVHNAKTKPREEQYNSTYRVVSVLTVLHQDWLNGKEYKCKVSNKALPAPIEKTISKAKGQPREPQVYTLPPSREEMTKNQVSLTCLVKGFYPSDIAVEWESNGQPENNYKTTPPVLDSDGSFFLYSKLTVDKSRWQQGNVFSCSVMHEALHNHYTQKSLSLSPGK

SEQ ID NO: 91 - protein, 642 aa, synthetic construct
SDTGRPFVEMYSEIPEIIHMTEGRELVIPCRVTSPNITVTLKKFPLDTLIPDGKRIIWDSRKGFIISNATYKEIGLLTCEATVNGHLYKTNYLTHRQTNTIIDVVLSPSHGIELSVGEKLVLNCTARTELNVGIDFNWEYPSSKHQHKKLVNRDLKTQSGSEMKKFLSTLTIDGVTRSDQGLYTCAASSGLMTKKNSTFVRVHEKGGGGSSPFIASVSDQHGVVYITENKNKTVVIPCLGSISNLNVSLVARYPEKRFVPDGNRISWDSKKGFTIPSYMISYAGMVFCEAKINDESYQSIMYIVVVVGYRIYDVVLSPSHGIELSVGEKLVLNCTARTELNVGIDFNWEYPSSKHQHKKLVIRDLKTQSGSEMKKFLSTLTIDGVTRSDQGLYTCAASSGLMTKKNSTFVRVHEKDKTHTCPPCPAPEAAGGPSVFLFPPKPKDTLMISRTPEVTCVVVDVSHEDPEVKFNWYVDGVEVHNAKTKPREEQYNSTYRVVSVLTVLHQDWLNGKEYKCKVSNKALPAPIEKTISKAKGQPREPQVYTLPPSREEMTKNQVSLTCLVKGFYPSDIAVEWESNGQPENNYKTTPPVLDSDGSFFLYSKLTVDKSRWQQGNVFSCSVMHEALHNHYTQKSLSLSPGK

SEQ ID NO: 92 - protein, 642 aa, synthetic construct
SDTGRPFVEMYSEIPEIIHMTEGRELVIPCRVTSPNITVTLKKFPLDTLIPDGKRIIWDSRKGFIISNATYKEIGLLTCEATVNGHLYKTNYLTHRQTNTIIDVVLSPSHGIELSVGEKLVLNCTARTELNVGIDFNWEYPSSKHQHKKLVNRDLKTQSGSEMKKFLSTLTIDGVTRSDQGLYTCAASSGLMTKKNSTFVRVHEKGGGGSSPFIASVSDQHGVVYITENKNKTVVIPCLGSISNLNVSLVARYPEKRFVPDGNRISWDSKKGFTIPSYMISYAGMVFCEAKINDESYQSIMYIVVVVGYRIYDVVLSPSHGIELSVGEKLVLNCTARTELNVGIDFNWEYPSSKHQHKKLVNLDLKTQSGSEMKKFLSTLTIDGVTRSDQGLYTCAASSGLMTKKNSTFVRVHEKDKTHTCPPCPAPEAAGGPSVFLFPPKPKDTLMISRTPEVTCVVVDVSHEDPEVKFNWYVDGVEVHNAKTKPREEQYNSTYRVVSVLTVLHQDWLNGKEYKCKVSNKALPAPIEKTISKAKGQPREPQVYTLPPSREEMTKNQVSLTCLVKGFYPSDIAVEWESNGQPENNYKTTPPVLDSDGSFFLYSKLTVDKSRWQQGNVFSCSVMHEALHNHYTQKSLSLSPGK

SEQ ID NO: 93 - protein, 642 aa, synthetic construct
SDTGRPFVEMYSEIPEIIHMTEGRELVIPCRVTSPNITVTLKKFPLDTLIPDGKRIIWDSRKGFIISNATYKEIGLLTCEATVNGHLYKTNYLTHRQTNTIIDVVLSPSHGIELSVGEKLVLNCTARTELNVGIDFNWEYPSSKHQHKKLVNRDLKTQSGSEMKKFLSTLTIDGVTRSDQGLYTCAASSGLMTKKNSTFVRVHEKGGGGSSPFIASVSDQHGVVYITENKNKTVVIPCLGSISNLNVSLVARYPEKRFVPDGNRISWDSKKGFTIPSYMISYAGMVFCEAKINDESYQSIMYIVVVVGYRIYDVVLSPSHGIELSVGEKLVLNCTARTELNVGIDFNWEYPSSKHQHKKLVNRQLKTQSGSEMKKFLSTLTIDGVTRSDQGLYTCAASSGLMTKKNSTFVRVHEKDKTHTCPPCPAPEAAGGPSVFLFPPKPKDTLMISRTPEVTCVVVDVSHEDPEVKFNWYVDGVEVHNAKTKPREEQYNSTYRVVSVLTVLHQDWLNGKEYKCKVSNKALPAPIEKTISKAKGQPREPQVYTLPPSREEMTKNQVSLTCLVKGFYPSDIAVEWESNGQPENNYKTTPPVLDSDGSFFLYSKLTVDKSRWQQGNVFSCSVMHEALHNHYTQKSLSLSPGK

SEQ ID NO: 94 - protein, 642 aa, synthetic construct
SDTGRPFVEMYSEIPEIIHMTEGRELVIPCRVTSPNITVTLKKFPLDTLIPDGKRIIWDSRKGFIISNATYKEIGLLTCEATVNGHLYKTNYLTHRQTNTIIDVVLSPSHGIELSVGEKLVLNCTARTELNVGIDFNWEYPSSKHQHKKLVNRDLKTQSGSEMKKFLSTLTIDGVTRSDQGLYTCAASSGLMTKKNSTFVRVHEKGGGGSSPFIASVSDQHGVVYITENKNKTVVIPCLGSISNLNVSLVARYPEKRFVPDGNRISWDSKKGFTIPSYMISYAGMVFCEAKINDESYQSIMYIVVVVGYRIYDVVLSPSHGIELSVGEKLVLNCTARTELNVGIDFNWEYPSSKHQHKKLVNRDLKTQSGTEMKKFLSTLTIDGVTRSDQGLYTCAASSGLMTKKNSTFVRVHEKDKTHTCPPCPAPEAAGGPSVFLFPPKPKDTLMISRTPEVTCVVVDVSHEDPEVKFNWYVDGVEVHNAKTKPREEQYNSTYRVVSVLTVLHQDWLNGKEYKCKVSNKALPAPIEKTISKAKGQPREPQVYTLPPSREEMTKNQVSLTCLVKGFYPSDIAVEWESNGQPENNYKTTPPVLDSDGSFFLYSKLTVDKSRWQQGNVFSCSVMHEALHNHYTQKSLSLSPGK

SEQ ID NO: 95 - protein, 642 aa, synthetic construct
SDTGRPFVEMYSEIPEIIHMTEGRELVIPCRVTSPNITVTLKKFPLDTLIPDGKRIIWDSRKGFIISNATYKEIGLLTCEATVNGHLYKTNYLTHRQTNTIIDVVLSPSHGIELSVGEKLVLNCTARTELNVGIDFNWEYPSSKHQHKKLVNRDLKTQSGSEMKKFLSTLTIDGVTRSDQGLYTCAASSGLMTKKNSTFVRVHEKGGGGSSPFIASVSDQHGVVYITENKNKTVVIPCLGSISNLNVSLVARYPEKRFVPDGNRISWDSKKGFTIPSYMISYAGMVFCEAKINDESYQSIMYIVVVVGYRIYDVVLSPSHGIELSVGEKLVLNCTARTELNVGIDFNWEYPSSKHQHKKLVNRDLKTQSGSEMKKFYSTLTIDGVTRSDQGLYTCAASSGLMTKKNSTFVRVHEKDKTHTCPPCPAPEAAGGPSVFLFPPKPKDTLMISRTPEVTCVVVDVSHEDPEVKFNWYVDGVEVHNAKTKPREEQYNSTYRVVSVLTVLHQDWLNGKEYKCKVSNKALPAPIEKTISKAKGQPREPQVYTLPPSREEMTKNQVSLTCLVKGFYPSDIAVEWESNGQPENNYKTTPPVLDSDGSFFLYSKLTVDKSRWQQGNVFSCSVMHEALHNHYTQKSLSLSPGK

SEQ ID NO: 96 - protein, 642 aa, synthetic construct
SDTGRPFVEMYSEIPEIIHMTEGRELVIPCRVTSPNITVTLKKFPLDTLIPDGKRIIWDSRKGFIISNATYKEIGLLTCEATVNGHLYKTNYLTHRQTNTIIDVVLSPSHGIELSVGEKLVLNCTARTELNVGIDFNWEYPSSKHQHKKLVNRDLKTQSGSEMKKFLSTLTIDGVTRSDQGLYTCAASSGLMTKKNSTFVRVHEKGGGGSSPFIASVSDQHGVVYITENKNKTVVIPCLGSISNLNVSLVARYPEKRFVPDGNRISWDSKKGFTIPSYMISYAGMVFCEAKINDESYQSIMYIVVVVGYRIYDVVLSPSHGIELSVGEKLVLNCTARTELNVGIDFNWEYPSSKHQHKKLVNRDLKTQSGSEMKKFLSTLTIDGVTRSDQGLYTCAASSGYMTKKNSTFVRVHEKDKTHTCPPCPAPEAAGGPSVFLFPPKPKDTLMISRTPEVTCVVVDVSHEDPEVKFNWYVDGVEVHNAKTKPREEQYNSTYRVVSVLTVLHQDWLNGKEYKCKVSNKALPAPIEKTISKAKGQPREPQVYTLPPSREEMTKNQVSLTCLVKGFYPSDIAVEWESNGQPENNYKTTPPVLDSDGSFFLYSKLTVDKSRWQQGNVFSCSVMHEALHNHYTQKSLSLSPGK

SEQ ID NO: 97 - protein, 642 aa, synthetic construct
SDTGRPFVEMYSEIPEIIHMTEGRELVIPCRVTSPNITVTLKKFPLDTLIPDGKRIIWDSRKGFIISNATYKEIGLLTCEATVNGHLYKTNYLTHRQTNTIIDVVLSPSHGIELSVGEKLVLNCTARTELNVGIDFNWEYPSSKHQHKKLVNRDLKTQSGSEMKKFLSTLTIDGVTRSDQGLYTCAASSGLMTKKNSTFVRVHEKGGGGSSPFIASVSDQHGVVYITENKNKTVVIPCLGSISNLNVSLVARYPEKRFVPDGNRISWDSKKGFTIPSYMISYAGMVFCEAKINDESYQSIMYIVVVVGYRIYDVVLSPSHGIELSVGEKLVLNCTARTELNVGIDFNWEYPSSKHQHKKLVNRDRKTQSGSEMKKFYSTLTIDGVTRSDQGLYTCAASSGLMTKKNSTFVRVHEKDKTHTCPPCPAPEAAGGPSVFLFPPKPKDTLMISRTPEVTCVVVDVSHEDPEVKFNWYVDGVEVHNAKTKPREEQYNSTYRVVSVLTVLHQDWLNGKEYKCKVSNKALPAPIEKTISKAKGQPREPQVYTLPPSREEMTKNQVSLTCLVKGFYPSDIAVEWESNGQPENNYKTTPPVLDSDGSFFLYSKLTVDKSRWQQGNVFSCSVMHEALHNHYTQKSLSLSPGK

SEQ ID NO: 98 - protein, 642 aa, synthetic construct
SDTGRPFVEMYSEIPEIIHMTEGRELVIPCRVTSPNITVTLKKFPLDTLIPDGKRIIWDSRKGFIISNATYKEIGLLTCEATVNGHLYKTNYLTHRQTNTIIDVVLSPSHGIELSVGEKLVLNCTARTELNVGIDFNWEYPSSKHQHKKLVNRDLKTQSGSEMKKFLSTLTIDGVTRSDQGLYTCAASSGLMTKKNSTFVRVHEKGGGGSSPFIASVSDQHGVVYITENKNKTVVIPCLGSISNLNVSLVARYPEKRFVPDGNRISWDSKKGFTIPSYMISYAGMVFCEAKINDESYQSIMYIVVVVGSKIYDVVLSPSHGIELSVGEKLVLNCTARTELNVGIDFNWEYPSSKHQHKKLVNRDLKTQSGSEMKKFLSTLTIDGVTRSDQGLYTCAASSGLMTKKNSTFVRVHEKDKTHTCPPCPAPEAAGGPSVFLFPPKPKDTLMISRTPEVTCVVVDVSHEDPEVKFNWYVDGVEVHNAKTKPREEQYNSTYRVVSVLTVLHQDWLNGKEYKCKVSNKALPAPIEKTISKAKGQPREPQVYTLPPSREEMTKNQVSLTCLVKGFYPSDIAVEWESNGQPENNYKTTPPVLDSDGSFFLYSKLTVDKSRWQQGNVFSCSVMHEALHNHYTQKSLSLSPGK

SEQ ID NO: 99 - protein, 642 aa, synthetic construct
SDTGRPFVEMYSEIPEIIHMTEGRELVIPCRVTSPNITVTLKKFPLDTLIPDGKRIIWDSRKGFIISNATYKEIGLLTCEATVNGHLYKTNYLTHRQTNTIIDVVLSPSHGIELSVGEKLVLNCTARTELNVGIDFNWEYPSSKHQHKKLVNRDLKTQSGSEMKKFLSTLTIDGVTRSDQGLYTCAASSGLMTKKNSTFVRVHEKGGGGSSPFIASVSDQHGVVYITENKNKTVVIPCLGSISNLNVSLVARYPEKRFVPDGNRISWDSKKGFTIPSYMISYAGMVFCEAKINDESYQSIMYIVVVVGYRIYDVVLSPSHGIELSVGEKLVLNCTARTELNVGIDFNWEYPSSKHQHKKLVNRDLKTQSGSEMKKFLSTLTIDGVTRSDQGLYTCAASSGRMTKKNSTFVRVHEKDKTHTCPPCPAPEAAGGPSVFLFPPKPKDTLMISRTPEVTCVVVDVSHEDPEVKFNWYVDGVEVHNAKTKPREEQYNSTYRVVSVLTVLHQDWLNGKEYKCKVSNKALPAPIEKTISKAKGQPREPQVYTLPPSREEMTKNQVSLTCLVKGFYPSDIAVEWESNGQPENNYKTTPPVLDSDGSFFLYSKLTVDKSRWQQGNVFSCSVMHEALHNHYTQKSLSLSPGK

SEQ ID NO: 100 - protein, 677 aa, synthetic construct
SPFIASVSDQHGVVYITENKNKTVVIPCLGSISNLNVSLVARYPEKRFVPDGNRISWDSKKGFTIPSYMISYAGMVFCEAKINDESYQSIMYIVVVVGYRIYDVVLSPSHGIELSVGEKLVLNCTARTELNVGIDFNWEYPSSKHQHKKLVNRDLKTQSGSEMKKFLSTLTIDGVTRSDQGLYTCAASSGLMTKKNSTFVRVHEKDKTHTCPPCPAPEAAGGPSVFLFPPKPKDTLMISRTPEVTCVVVDVSHEDPEVKFNWYVDGVEVHNAKTKPREEQYNSTYRVVSVLTVLHQDWLNGKEYKCKVSNKALPAPIEKTISKAKGQPREPQVYTLPPSREEMTKNQVSLTCLVKGFYPSDIAVEWESNGQPENNYKTTPPVLDSDGSFFLYSKLTVDKSRWQQGNVFSCSVMHEALHNHYTQKSLSLSPGGGGGSGGGGSGGGGSGGGGSEVQLVESGGGLVQPGGSLRLSCAASGYTFTNYGMNWVRQAPGKGLEWVGWINTYTGEPTYAADFKRRFTFSLDTSKSTAYLQMNSLRAEDTAVYYCAKYPHYYGSSHWYFDVWGQGTLVTVSSASTKGPSVFPLAPSSKSTSGGTAALGCLVKDYFPEPVTVSWNSGALTSGVHTFPAVLQSSGLYSLSSVVTVPSSSLGTQTYICNVNHKPSNTKVDKKVEPKSC

SEQ ID NO: 101 - protein, 214 aa, synthetic construct
DIQMTQSPSSLSASVGDRVTITCSASQDISNYLNWYQQKPGKAPKVLIYFTSSLHSGVPSRFSGSGSGTDFTLTISSLQPEDFATYYCQQYSTVPWTFGQGTKVEIKRTVAAPSVFIFPPSDEQLKSGTASVVCLLNNFYPREAKVQWKVDNALQSGNSQESVTEQDSKDSTYSLSSTLTLSKADYEKHKVYACEVTHQGLSSPVTKSFNRGEC

SEQ ID NO: 102 - protein, 642 aa, synthetic construct
SDTGRPFVEMYSEIPEIIHMTEGRELVIPCRVTSPNITVTLKKFPLDTLIPDGKRIIWDSRKGFIISNATYKEIGLLTCEATVNGHLYKTNYLTHRQTNTIIDVVLSPSHGIELSVGEKLVLNCTARTELNVGIDFNWEYPSSKHQHKKLVNRDLKTQSGSEMKKFLSTLTIDGVTRSDQGLYTCAASSGLMTKKNSTFVRVHEKGGGGSSPFIASVSDQHGVVYITENKNKTVVIPCLGSISNLNVSLIARYPEKRFVPDGNRISWDSKKGFTIPSYMISYAGMVFCEAKINDESYQSIMYIVVVVGYRIYDVVLSPSHGIELSVGEKLVLNCTARTELNVGIDFNWEYPSSKHQHKKLVNRDLKTQSGSEMKKFLSTLTIDGVTRSDQGLYTCAASSGLMTKKNSTFVRVHEKDKTHTCPPCPAPEAAGGPSVFLFPPKPKDTLMISRTPEVTCVVVDVSHEDPEVKFNWYVDGVEVHNAKTKPREEQYNSTYRVVSVLTVLHQDWLNGKEYKCKVSNKALPAPIEKTISKAKGQPREPQVYTLPPSREEMTKNQVSLTCLVKGFYPSDIAVEWESNGQPENNYKTTPPVLDSDGSFFLYSKLTVDKSRWQQGNVFSCSVMHEALHNHYTQKSLSLSPGK

SEQ ID NO: 103 - protein, 642 aa, synthetic construct
SDTGRPFVEMYSEIPEIIHMTEGRELVIPCRVTSPNITVTLKKFPLDTLIPDGKRIIWDSRKGFIISNATYKEIGLLTCEATVNGHLYKTNYLTHRQTNTIIDVVLSPSHGIELSVGEKLVLNCTARTELNVGIDFNWEYPSSKHQHKKLVNRDLKTQSGSEMKKFLSTLTIDGVTRSDQGLYTCAASSGLMTKKNSTFVRVHEKGGGGSSPFIASVSDQHGVVYITENKNKTVVIPCLGSISNLNVSLLARYPEKRFVPDGNRISWDSKKGFTIPSYMISYAGMVFCEAKINDESYQSIMYIVVVVGYRIYDVVLSPSHGIELSVGEKLVLNCTARTELNVGIDFNWEYPSSKHQHKKLVNRDLKTQSGSEMKKFLSTLTIDGVTRSDQGLYTCAASSGLMTKKNSTFVRVHEKDKTHTCPPCPAPEAAGGPSVFLFPPKPKDTLMISRTPEVTCVVVDVSHEDPEVKFNWYVDGVEVHNAKTKPREEQYNSTYRVVSVLTVLHQDWLNGKEYKCKVSNKALPAPIEKTISKAKGQPREPQVYTLPPSREEMTKNQVSLTCLVKGFYPSDIAVEWESNGQPENNYKTTPPVLDSDGSFFLYSKLTVDKSRWQQGNVFSCSVMHEALHNHYTQKSLSLSPGK

SEQ ID NO: 104 - protein, 637 aa, synthetic construct
SDTGRPFVEMYSEIPEIIHMTEGRELVIPCRVTSPNITVTLKKFPLDTLIPDGKRIIWDSRKGFIISNATYKEIGLLTCEATVNGHLYKTNYLTHRQTNTIIDVVLSPSHGIELSVGEKLVLNCTARTELNVGIDFNWEYPSSKHQHKKLVNRDLKTQSGSEMKKFLSTLTIDGVTRSDQGLYTCAASSGLMTKKNSTFVRVHEKSPFIASVSDQHGVVYITENKNKTVVIPCLGSISNLNVSLVARYPEKRFVPDGNRISWDSKKGFTIPSYMISYAGMVFCEAKINDESYQSIMYIVVVVGYRIYDVVLSPSHGIELSVGEKLVLNCTARTELNVGIDFNWEYPSSKHQHKKLVFRDLKTQSGTEMKKFLSTLTIDGVTRSDQGLYTCAASSGLMTKKNSTFVRVHEKDKTHTCPPCPAPEAAGGPSVFLFPPKPKDTLMISRTPEVTCVVVDVSHEDPEVKFNWYVDGVEVHNAKTKPREEQYNSTYRVVSVLTVLHQDWLNGKEYKCKVSNKALPAPIEKTISKAKGQPREPQVYTLPPSREEMTKNQVSLTCLVKGFYPSDIAVEWESNGQPENNYKTTPPVLDSDGSFFLYSKLTVDKSRWQQGNVFSCSVMHEALHNHYTQKSLSLSPGK

SEQ ID NO: 105 - protein, 637 aa, synthetic construct
SDTGRPFVEMYSEIPEIIHMTEGRELVIPCRVTSPNITVTLKKFPLDTLIPDGKRIIWDSRKGFIISNATYKEIGLLTCEATVNGHLYKTNYLTHRQTNTIIDVVLSPSHGIELSVGEKLVLNCTARTELNVGIDFNWEYPSSKHQHKKLVNRDLKTQSGSEMKKFLSTLTIDGVTRSDQGLYTCAASSGLMTKKNSTFVRVHEKSPFIASVSDQHGVVYITENKNKTVVIPCLGSISNLNVSLVARYPEKRFVPDGNRISWDSKKGFTIPSYMISYAGMVFCEAKINDESYQSIMYIVVVVGSKIYDVVLSPSHGIELSVGEKLVLNCTARTELNVGIDFNWEYPSSKHQHKKLVFRDLKTQSGSEMKKFLSTLTIDGVTRSDQGLYTCAASSGLMTKKNSTFVRVHEKDKTHTCPPCPAPEAAGGPSVFLFPPKPKDTLMISRTPEVTCVVVDVSHEDPEVKFNWYVDGVEVHNAKTKPREEQYNSTYRVVSVLTVLHQDWLNGKEYKCKVSNKALPAPIEKTISKAKGQPREPQVYTLPPSREEMTKNQVSLTCLVKGFYPSDIAVEWESNGQPENNYKTTPPVLDSDGSFFLYSKLTVDKSRWQQGNVFSCSVMHEALHNHYTQKSLSLSPGK

SEQ ID NO: 106 - protein, 637 aa, synthetic construct
SDTGRPFVEMYSEIPEIIHMTEGRELVIPCRVTSPNITVTLKKFPLDTLIPDGKRIIWDSRKGFIISNATYKEIGLLTCEATVNGHLYKTNYLTHRQTNTIIDVVLSPSHGIELSVGEKLVLNCTARTELNVGIDFNWEYPSSKHQHKKLVNRDLKTQSGSEMKKFLSTLTIDGVTRSDQGLYTCAASSGLMTKKNSTFVRVHEKSPFIASVSDQHGVVYITENKNKTVVIPCLGSISNLNVSLVARYPEKRFVPDGNRISWDSKKGFTIPSYMISYAGMVFCEAKINDESYQSIMYIVVVVGSKIYDVVLSPSHGIELSVGEKLVLNCTARTELNVGIDFNWEYPSSKHQHKKLVNRDLKTQSGTEMKKFLSTLTIDGVTRSDQGLYTCAASSGLMTKKNSTFVRVHEKDKTHTCPPCPAPEAAGGPSVFLFPPKPKDTLMISRTPEVTCVVVDVSHEDPEVKFNWYVDGVEVHNAKTKPREEQYNSTYRVVSVLTVLHQDWLNGKEYKCKVSNKALPAPIEKTISKAKGQPREPQVYTLPPSREEMTKNQVSLTCLVKGFYPSDIAVEWESNGQPENNYKTTPPVLDSDGSFFLYSKLTVDKSRWQQGNVFSCSVMHEALHNHYTQKSLSLSPGK

SEQ ID NO: 107 - protein, 637 aa, synthetic construct
SDTGRPFVEMYSEIPEIIHMTEGRELVIPCRVTSPNITVTLKKFPLDTLIPDGKRIIWDSRKGFIISNATYKEIGLLTCEATVNGHLYKTNYLTHRQTNTIIDVVLSPSHGIELSVGEKLVLNCTARTELNVGIDFNWEYPSSKHQHKKLVNRDLKTQSGSEMKKFLSTLTIDGVTRSDQGLYTCAASSGLMTKKNSTFVRVHEKSPFIASVSDQHGVVYITENKNKTVVIPCLGSISNLNVSLVARYPEKRFVPDGNRISWDSKKGFTIPSYMISYAGMVFCEAKINDESYQSIMYIVVVVGSKIYDVVLSPSHGIELSVGEKLVLNCTARTELNVGIDFNWEYPSSKHQHKKLVFRDLKTQSGTEMKKFLSTLTIDGVTRSDQGLYTCAASSGLMTKKNSTFVRVHEKDKTHTCPPCPAPEAAGGPSVFLFPPKPKDTLMISRTPEVTCVVVDVSHEDPEVKFNWYVDGVEVHNAKTKPREEQYNSTYRVVSVLTVLHQDWLNGKEYKCKVSNKALPAPIEKTISKAKGQPREPQVYTLPPSREEMTKNQVSLTCLVKGFYPSDIAVEWESNGQPENNYKTTPPVLDSDGSFFLYSKLTVDKSRWQQGNVFSCSVMHEALHNHYTQKSLSLSPGK

SEQ ID NO: 108 - protein, 642 aa, synthetic construct
SDTGRPFVEMYSEIPEIIHMTEGRELVIPCRVTSPNITVTLKKFPLDTLIPDGKRIIWDSRKGFIISNATYKEIGLLTCEATVNGHLYKTNYLTHRQTNTIIDVVLSPSHGIELSVGEKLVLNCTARTELNVGIDFNWEYPSSKHQHKKLVNRDLKTQSGSEMKKFLSTLTIDGVTRSDQGLYTCAASSGLMTKKNSTFVRVHEKGGGGSSPFIASVSDQHGVVYITENKNKTVVIPCLGSISNLNVSLVARYPEKRFVPDGNRISWDSKKGFTIPSYMISYAGMVFCEAKINDESYQSIMYIVVVVGYRIYDVVLSPSHGIELSVGEKLVLNCTARTELNVGIDFNWEYPSSKHQHKKLVFRDLKTQSGTEMKKFLSTLTIDGVTRSDQGLYTCAASSGLMTKKNSTFVRVHEKDKTHTCPPCPAPEAAGGPSVFLFPPKPKDTLMISRTPEVTCVVVDVSHEDPEVKFNWYVDGVEVHNAKTKPREEQYNSTYRVVSVLTVLHQDWLNGKEYKCKVSNKALPAPIEKTISKAKGQPREPQVYTLPPSREEMTKNQVSLTCLVKGFYPSDIAVEWESNGQPENNYKTTPPVLDSDGSFFLYSKLTVDKSRWQQGNVFSCSVMHEALHNHYTQKSLSLSPGK

SEQ ID NO: 109 - protein, 642 aa, synthetic construct
SDTGRPFVEMYSEIPEIIHMTEGRELVIPCRVTSPNITVTLKKFPLDTLIPDGKRIIWDSRKGFIISNATYKEIGLLTCEATVNGHLYKTNYLTHRQTNTIIDVVLSPSHGIELSVGEKLVLNCTARTELNVGIDFNWEYPSSKHQHKKLVNRDLKTQSGSEMKKFLSTLTIDGVTRSDQGLYTCAASSGLMTKKNSTFVRVHEKGGGGSSPFIASVSDQHGVVYITENKNKTVVIPCLGSISNLNVSLVARYPEKRFVPDGNRISWDSKKGFTIPSYMISYAGMVFCEAKINDESYQSIMYIVVVVGSKIYDVVLSPSHGIELSVGEKLVLNCTARTELNVGIDFNWEYPSSKHQHKKLVFRDLKTQSGSEMKKFLSTLTIDGVTRSDQGLYTCAASSGLMTKKNSTFVRVHEKDKTHTCPPCPAPEAAGGPSVFLFPPKPKDTLMISRTPEVTCVVVDVSHEDPEVKFNWYVDGVEVHNAKTKPREEQYNSTYRVVSVLTVLHQDWLNGKEYKCKVSNKALPAPIEKTISKAKGQPREPQVYTLPPSREEMTKNQVSLTCLVKGFYPSDIAVEWESNGQPENNYKTTPPVLDSDGSFFLYSKLTVDKSRWQQGNVFSCSVMHEALHNHYTQKSLSLSPGK

SEQ ID NO: 110 - protein, 642 aa, synthetic construct
SDTGRPFVEMYSEIPEIIHMTEGRELVIPCRVTSPNITVTLKKFPLDTLIPDGKRIIWDSRKGFIISNATYKEIGLLTCEATVNGHLYKTNYLTHRQTNTIIDVVLSPSHGIELSVGEKLVLNCTARTELNVGIDFNWEYPSSKHQHKKLVNRDLKTQSGSEMKKFLSTLTIDGVTRSDQGLYTCAASSGLMTKKNSTFVRVHEKGGGGSSPFIASVSDQHGVVYITENKNKTVVIPCLGSISNLNVSLVARYPEKRFVPDGNRISWDSKKGFTIPSYMISYAGMVFCEAKINDESYQSIMYIVVVVGSKIYDVVLSPSHGIELSVGEKLVLNCTARTELNVGIDFNWEYPSSKHQHKKLVNRDLKTQSGTEMKKFLSTLTIDGVTRSDQGLYTCAASSGLMTKKNSTFVRVHEKDKTHTCPPCPAPEAAGGPSVFLFPPKPKDTLMISRTPEVTCVVVDVSHEDPEVKFNWYVDGVEVHNAKTKPREEQYNSTYRVVSVLTVLHQDWLNGKEYKCKVSNKALPAPIEKTISKAKGQPREPQVYTLPPSREEMTKNQVSLTCLVKGFYPSDIAVEWESNGQPENNYKTTPPVLDSDGSFFLYSKLTVDKSRWQQGNVFSCSVMHEALHNHYTQKSLSLSPGK

SEQ ID NO: 111 - protein, 642 aa, synthetic construct
SDTGRPFVEMYSEIPEIIHMTEGRELVIPCRVTSPNITVTLKKFPLDTLIPDGKRIIWDSRKGFIISNATYKEIGLLTCEATVNGHLYKTNYLTHRQTNTIIDVVLSPSHGIELSVGEKLVLNCTARTELNVGIDFNWEYPSSKHQHKKLVNRDLKTQSGSEMKKFLSTLTIDGVTRSDQGLYTCAASSGLMTKKNSTFVRVHEKGGGGSSPFIASVSDQHGVVYITENKNKTVVIPCLGSISNLNVSLVARYPEKRFVPDGNRISWDSKKGFTIPSYMISYAGMVFCEAKINDESYQSIMYIVVVVGSKIYDVVLSPSHGIELSVGEKLVLNCTARTELNVGIDFNWEYPSSKHQHKKLVFRDLKTQSGTEMKKFLSTLTIDGVTRSDQGLYTCAASSGLMTKKNSTFVRVHEKDKTHTCPPCPAPEAAGGPSVFLFPPKPKDTLMISRTPEVTCVVVDVSHEDPEVKFNWYVDGVEVHNAKTKPREEQYNSTYRVVSVLTVLHQDWLNGKEYKCKVSNKALPAPIEKTISKAKGQPREPQVYTLPPSREEMTKNQVSLTCLVKGFYPSDIAVEWESNGQPENNYKTTPPVLDSDGSFFLYSKLTVDKSRWQQGNVFSCSVMHEALHNHYTQKSLSLSPGK

SEQ ID NO: 112 - protein, 432 aa, synthetic construct
SPFIASVSDQHGVVYITENKNKTVVIPCLGSISNLNVSLVARYPEKRFVPDGNRISWDSKKGFTIPSYMISYAGMVFCEAKINDESYQSIMYIVVVVGYRIYDVVLSPSHGIELSVGEKLVLNCTARTELNVGIDFNWEYPSSKHQHKKLVFRDLKTQSGTEMKKFLSTLTIDGVTRSDQGLYTCAASSGLMTKKNSTFVRVHEKDKTHTCPPCPAPEAAGGPSVFLFPPKPKDTLMISRTPEVTCVVVDVSHEDPEVKFNWYVDGVEVHNAKTKPREEQYNSTYRVVSVLTVLHQDWLNGKEYKCKVSNKALPAPIEKTISKAKGQPREPQVYTLPPSREEMTKNQVSLTCLVKGFYPSDIAVEWESNGQPENNYKTTPPVLDSDGSFFLYSKLTVDKSRWQQGNVFSCSVMHEALHNHYTQKSLSLSPGK

SEQ ID NO: 113 - protein, 432 aa, synthetic construct
SPFIASVSDQHGVVYITENKNKTVVIPCLGSISNLNVSLVARYPEKRFVPDGNRISWDSKKGFTIPSYMISYAGMVFCEAKINDESYQSIMYIVVVVGSKIYDVVLSPSHGIELSVGEKLVLNCTARTELNVGIDFNWEYPSSKHQHKKLVFRDLKTQSGSEMKKFLSTLTIDGVTRSDQGLYTCAASSGLMTKKNSTFVRVHEKDKTHTCPPCPAPEAAGGPSVFLFPPKPKDTLMISRTPEVTCVVVDVSHEDPEVKFNWYVDGVEVHNAKTKPREEQYNSTYRVVSVLTVLHQDWLNGKEYKCKVSNKALPAPIEKTISKAKGQPREPQVYTLPPSREEMTKNQVSLTCLVKGFYPSDIAVEWESNGQPENNYKTTPPVLDSDGSFFLYSKLTVDKSRWQQGNVFSCSVMHEALHNHYTQKSLSLSPGK

SEQ ID NO: 114 - protein, 432 aa, synthetic construct
SPFIASVSDQHGVVYITENKNKTVVIPCLGSISNLNVSLVARYPEKRFVPDGNRISWDSKKGFTIPSYMISYAGMVFCEAKINDESYQSIMYIVVVVGSKIYDVVLSPSHGIELSVGEKLVLNCTARTELNVGIDFNWEYPSSKHQHKKLVNRDLKTQSGTEMKKFLSTLTIDGVTRSDQGLYTCAASSGLMTKKNSTFVRVHEKDKTHTCPPCPAPEAAGGPSVFLFPPKPKDTLMISRTPEVTCVVVDVSHEDPEVKFNWYVDGVEVHNAKTKPREEQYNSTYRVVSVLTVLHQDWLNGKEYKCKVSNKALPAPIEKTISKAKGQPREPQVYTLPPSREEMTKNQVSLTCLVKGFYPSDIAVEWESNGQPENNYKTTPPVLDSDGSFFLYSKLTVDKSRWQQGNVFSCSVMHEALHNHYTQKSLSLSPGK

SEQ ID NO: 115 - protein, 432 aa, synthetic construct
SPFIASVSDQHGVVYITENKNKTVVIPCLGSISNLNVSLVARYPEKRFVPDGNRISWDSKKGFTIPSYMISYAGMVFCEAKINDESYQSIMYIVVVVGSKIYDVVLSPSHGIELSVGEKLVLNCTARTELNVGIDFNWEYPSSKHQHKKLVFRDLKTQSGTEMKKFLSTLTIDGVTRSDQGLYTCAASSGLMTKKNSTFVRVHEKDKTHTCPPCPAPEAAGGPSVFLFPPKPKDTLMISRTPEVTCVVVDVSHEDPEVKFNWYVDGVEVHNAKTKPREEQYNSTYRVVSVLTVLHQDWLNGKEYKCKVSNKALPAPIEKTISKAKGQPREPQVYTLPPSREEMTKNQVSLTCLVKGFYPSDIAVEWESNGQPENNYKTTPPVLDSDGSFFLYSKLTVDKSRWQQGNVFSCSVMHEALHNHYTQKSLSLSPGK

SEQ ID NO: 116 - protein, 637 aa, synthetic construct
SDTGRPFVEMYSEIPEIIHMTEGRELVIPCRVTSPNITVTLKKFPLDTLIPDGKRIIWDSRKGFIISNATYKEIGLLTCEATVNGHLYKTNYLTHRQTNTIIDVVLSPSHGIELSVGEKLVLNCTARTELNVGIDFNWEYPSSKHQHKKLVNRDLKTQSGSEMKKFLSTLTIDGVTRSDQGLYTCAASSGLMTKKNSTFVRVHEKSPFIASVSDQHGVVYITENKNKTVVIPCLGSISNLNVSLVARYPEKRFVPDGNRISWDSKKGFTIPSYMISYAGMVFCEAKINDESYQSIMYIVVVVGSKIYDVVLSPSHGIELSVGEKLVLNCTARTELNVGIDFNWEYPSSKHQHKKLVNRDLKTQSGSEMKKFLSTLTIDGVTRSDQGLYTCAASSGLMTKKNSTFVRVHEKDKTHTCPPCPAPEAAGGPSVFLFPPKPKDTLMISRTPEVTCVVVDVSHEDPEVKFNWYVDGVEVHNAKTKPREEQYNSTYRVVSVLTVLHQDWLNGKEYKCKVSNKALPAPIEKTISKAKGQPREPQVYTLPPSREEMTKNQVSLTCLVKGFYPSDIAVEWESNGQPENNYKTTPPVLDSDGSFFLYSKLTVDKSRWQQGNVFSCSVMHEALHNHYTQKSLSLSPGK

SEQ ID NO: 117 - protein, 677 aa, synthetic construct
SPFIASVSDQHGVVYITENKNKTVVIPCLGSISNLNVSLVARYPEKRFVPDGNRISWDSKKGFTIPSYMISYAGMVFCEAKINDESYQSIMYIVVVVGSKIYDVVLSPSHGIELSVGEKLVLNCTARTELNVGIDFNWEYPSSKHQHKKLVFRDLKTQSGTEMKKFLSTLTIDGVTRSDQGLYTCAASSGLMTKKNSTFVRVHEKDKTHTCPPCPAPEAAGGPSVFLFPPKPKDTLMISRTPEVTCVVVDVSHEDPEVKFNWYVDGVEVHNAKTKPREEQYNSTYRVVSVLTVLHQDWLNGKEYKCKVSNKALPAPIEKTISKAKGQPREPQVYTLPPSREEMTKNQVSLTCLVKGFYPSDIAVEWESNGQPENNYKTTPPVLDSDGSFFLYSKLTVDKSRWQQGNVFSCSVMHEALHNHYTQKSLSLSPGGGGGSGGGGSGGGGSGGGGSEVQLVESGGGLVQPGGSLRLSCAASGYTFTNYGMNWVRQAPGKGLEWVGWINTYTGEPTYAADFKRRFTFSLDTSKSTAYLQMNSLRAEDTAVYYCAKYPHYYGSSHWYFDVWGQGTLVTVSSASTKGPSVFPLAPSSKSTSGGTAALGCLVKDYFPEPVTVSWNSGALTSGVHTFPAVLQSSGLYSLSSVVTVPSSSLGTQTYICNVNHKPSNTKVDKKVEPKSC

SEQ ID NO: 118 - protein, 214 aa, synthetic construct; identical to SEQ ID NO: 101

SEQ ID NO: 119 - protein, 205 aa, Homo sapiens
SPFIASVSDQHGVVYITENKNKTVVIPCLGSISNLNVSLCARYPEKRFVPDGNRISWDSKKGFTIPSYMISYAGMVFCEAKINDESYQSIMYIVVVVGYRIYDVVLSPSHGIELSVGEKLVLNCTARTELNVGIDFNWEYPSSKHQHKKLVNRDLKTQSGSEMKKFLSTLTIDGVTRSDQGLYTCAASSGLMTKKNSTFVRVHEK

SEQ ID NO: 120 - protein, 431 aa, synthetic construct
SDTGRPFVEMYSEIPEIIHMTEGRELVIPCRVTSPNITVTLKKFPLDTLIPDGKRIIWDSRKGFIISNATYKEIGLLTCEATVNGHLYKTNYLTHRQTNTIIDVVLSPSHGIELSVGEKLVLNCTARTELNVGIDFNWEYPSSKHQHKKLVNRDLKTQSGSEMKKFLSTLTIDGVTRSDQGLYTCAASSGLMTKKNSTFVRVHEKDKTHTCPPCPAPELLGGPSVFLFPPKPKDTLMISRTPEVTCVVVDVSHEDPEVKFNWYVDGVEVHNAKTKPREEQYNSTYRVVSVLTVLHQDWLNGKEYKCKVSNKALPAPIEKTISKAKGQPREPQVYTLPPSRDELTKNQVSLTCLVKGFYPSDIAVEWESNGQPENNYKTTPPVLDSDGSFFLYSKLTVDKSRWQQGNVFSCSVMHEALHNHYTQKSLSLSPG

SEQ ID NO: 121 - protein, 537 aa, synthetic construct
YSMTPPTLNITEESHVIDTGDSLSISCRGQHPLEWAWPGAQEAPATGDKDSEDTGVVRDCEGTDARPYCKVLLLHEVHAQDTGSYVCYYKYIKARIEGTTAASSYVFVRDFEQPFINKPDTLLVNRKDAMWVPCLVSIPGLNVTLRSQSSVLWPDGQEVVWDDRRGMLVSTPLLHDALYLQCETTWGDQDFLSNPFLVHITGNELYDIQLLPRKSLELLVGEKLVLNCTVWAEFNSGVTFDWDYPGKQAERGKWVPERRSQQTHTELSSILTIHNVSQHDLGSYVCKANNGIQRFRESTEVIVHEEPKSCDKTHTCPPCPAPELLGGPSVFLFPPKPKDTLMISRTPEVTCVVVDVSHEDPEVKFNWYVDGVEVHNAKTKPREEQYNSTYRVVSVLTVLHQDWLNGKEYKCKVSNKALPAPIEKTISKAKGQPREPQVYTLPPSRDELTKNQVSLTCLVKGFYPSDIAVEWESNGQPENNYKTTPPVLDSDGSFFLYSKLTVDKSRWQQGNVFSCSVMHEALHNHYTQKSLSLSPGK

SEQ ID NO: 122 - protein, 453 aa, synthetic construct
EVQLVESGGGLVQPGGSLRLSCAASGYTFTNYGMNWVRQAPGKGLEWVGWINTYTGEPTYAADFKRRFTFSLDTSKSTAYLQMNSLRAEDTAVYYCAKYPHYYGSSHWYFDVWGQGTLVTVSSASTKGPSVFPLAPSSKSTSGGTAALGCLVKDYFPEPVTVSWNSGALTSGVHTFPAVLQSSGLYSLSSVVTVPSSSLGTQTYICNVNHKPSNTKVDKKVEPKSCDKTHTCPPCPAPEAAGGPSVFLFPPKPKDTLMISRTPEVTCVVVDVSHEDPEVKFNWYVDGVEVHNAKTKPREEQYNSTYRVVSVLTVLHQDWLNGKEYKCKVSNKALPAPIEKTISKAKGQPREPQVYTLPPSREEMTKNQVSLTCLVKGFYPSDIAVEWESNGQPENNYKTTPPVLDSDGSFFLYSKLTVDKSRWQQGNVFSCSVMHEALHNHYTQKSLSLSPGK

SEQ ID NO: 123 - protein, 214 aa, synthetic construct; identical to SEQ ID NO: 101

SEQ ID NO: 124 - DNA, 304 bp, synthetic construct
  source 1..304: mol_type = other DNA
cgttacataacttacggtaaatggcccgcctggctgaccgcccaacgacccccgcccattgacgtcaataatgacgtatgttcccatagtaacgccaatagggactttccattgacgtcaatgggtggagtatttacggtaaactgcccacttggcagtacatcaagtgtatcatatgccaagtacgccccctattgacgtcaatgacggtaaatggcccgcctggcattatgcccagtacatgaccttatgggactttcctacttggcagtacatctacgtattagtcatcgctattaccatg

SEQ ID NO: 125 - DNA, 309 bp, synthetic construct
  source 1..309: mol_type = other DNA
tgctgatgcggttttggcagtacaccaatgggcgtggatagcggtttgactcacggggatttccaagtctccaccccattgacgtcaatgggagtttgttttggcaccaaaatcaacgggactttccaaaatgtcgtaataaccccgccccgttgacgcaaatgggcggtaggcgtgtacggtgggaggtctatataagcagagctcgtttagtgaaccgtcagatcgcctggagaggccatccacgctgttttgacctccatagtggacaccgggaccgatccagcctccgcgtctcaggggaagctt

SEQ ID NO: 126 - DNA, 43 bp, synthetic construct
  source 1..43: mol_type = other DNA
cttgttctttttgcagaagctcagaataaacgctcaactttgg

SEQ ID NO: 127 - protein, 745 aa, synthetic construct
MAADGYLPDWLEDTLSEGIRQWWKLKPGPPPPKPAERHKDDSRGLVLPGYKYLGPFNGLDKGEPVNEADAAALEHDKAYDRQLDSGDNPYLKYNHADAEFQERLKEDTSFGGNLGRAVFQAKKRVLEPLGLVEEPVKTAPGKKRPVEHSPVEPDSSSGTGKAGQQPARKRLNFGQTGDADSVPDPQPLGQPPAAPSGLGTNTMATGSGAPMADNNEGADGVGNSSGNWHCDSTWMGDRVITTSTRTWALPTYNNHLYKQISSQSGASNDNHYFGYSTPWGYFDFNRFHCHFSPRDWQRLINNNWGFRPKRLNFKLFNIQVKEVTQNDGTTTIANNLTSTVQVFTDSEYQLPYVLGSAHQGCLPPFPADVFMVPQYGYLTLNNGSQAVGRSSFYCLEYFPSQMLRTGNNFTFSYTFEDVPFHSSYAHSQSLDRLMNPLIDQYLYYLSRTNTPSGTTTQSRLQFSQAGASDIRDQSRNWLPGPCYRQQRVSKTSADNNNSEYSWTGATKYHLNGRDSLVNPGPAMASHKDDEEKFFPQSGVLIFGKQGSEKTNVDIEKVMITDEEEIRTTNPVATEQYGSVSTNLQRGNLALGDTTRPARQAATADVNTQGVLPGMVWQDRDVYLQGPIWAKIPHTDGHFHPSPLMGGFGLKHPPPQILIKNTPVPANPSTTFSAAKFASFITQYSTGQVSVEIEWELQKENSKRWNPEIQYTSNYNKSINVDFTVDTNGVYSEPRPIGTRYLTRNL

SEQ ID NO: 128 - DNA, 1977 bp, synthetic construct
  source 1..1977: mol_type = other DNA
atgcctctgctgctgctgttgcctttgttgtgggctggcgccctggcttctgataccggcagacctttcgtggaaatgtacagcgagatccccgagatcatccacatgaccgagggcagagagctggtcatcccctgcagagtgacctctcctaacatcaccgtgactctgaagaagttccctctggacacactgatccccgacggcaagagaatcatctgggactcccggaagggcttcatcatctccaacgccacctacaaagagatcggcctgctgacctgcgaggccaccgttaatggccacctgtacaagaccaactatctgacccacagacagaccaacaccatcatcgacgtggtgctgagcccctctcatggcatcgagctgtccgtgggagaaaagctggtgctgaactgcaccgccagaaccgagctgaacgtgggcatcgacttcaactgggagtacccctccagcaagcaccagcacaagaagctggtcaaccgggacctgaaaacccagtccggctccgagatgaagaaattcctgagcaccctgaccatcgacggcgtgaccagatctgaccagggcctgtatacctgcgccgcttcttctggcctgatgaccaagaaaaactccaccttcgtgcgggtgcacgagaaaggtggcggaggcagctctccttttatcgcctctgtgtctgatcagcacggcgtggtgtacatcaccgagaacaagaacaagaccgtcgtgatcccctgcctgggctccatctctaacctgaacgtgtccctggtggctagataccccgagaagagattcgtgcctgacggcaaccggatctcctgggacagcaagaagggctttacaatcccctcctacatgatctcctacgccggcatggtgttctgcgaggctaagatcaacgacgagtcctaccagtccatcatgtacatcgtggtggtcgtgggctacagaatctacgatgtggtgctgtcccctagccacggaatcgaactgagcgtgggcgagaaactggtcctcaactgtaccgctcggacagaactgaatgtggggattgatttcaattgggaataccctagctccaaacatcagcataagaaactcgtgaaccgcgatctcaagacccagagcggaacagaaatgaagaagtttctgtccacactcaccattgacggggtcaccagaagcgatcagggactctatacctgtgctgcctccagcggactgatgacaaaaaagaacagcacatttgtccgcgtccacgagaaggacaaaactcacacatgcccaccgtgcccggcgcctgaagccgctgggggaccgtcagtcttcctcttccccccaaaacccaaggacaccctcatgatctcccggacccctgaggtcacatgcgtggtggtggacgtgagccacgaagaccctgaggtcaagttcaactggtacgtggacggcgtggaggtgcataatgccaagacaaagccgcgggaggagcagtacaacagcacgtaccgggtggtcagcgtcctcaccgtcctgcaccaggactggctgaatggcaaggagtacaagtgcaaggtctccaacaaagccctcccagcccccatcgagaaaaccatctccaaagccaaagggcagcccagggaaccacaggtgtacaccctgcccccatcccgggaggagatgaccaagaaccaggtcagcctgacctgcctggtcaaaggcttctatcccagcgacatcgccgtggagtgggagagcaatgggcagccggagaacaactacaagaccacgcctcccgtgctggactccgacggctccttcttcctctacagcaagctcaccgtggacaagagcaggtggcagcaggggaacgtcttctcatgctccgtgatgcatgaggctctgcacaaccactacacgcagaagagcctctccctgtctccgggtaaataa

SEQ ID NO: 129 - DNA, 1977 bp, synthetic construct
  source 1..1977: mol_type = other DNA
atgcctctgctgctgctgctgcctctgctgtgggccggcgccctggcctccgacaccggccggccttttgttgaaatgtactccgagatccccgaaatcatccacatgacagaaggcagagagctggtgatcccttgtagagtgaccagcccaaacatcaccgtgactctgaagaagttccccctggatacactgatccctgatggaaagagaatcatttgggatagcagaaagggctttatcatcagcaacgccacatacaaagagatcggcctgctcacctgcgaggccaccgtgaacggccacctgtataagacaaactacctgacacatagacagaccaacaccatcattgacgtggtgctgtccccaagccacggaatcgagctgtctgtgggcgagaagctggtgctgaactgcaccgccagaacagagctgaacgtgggcattgacttcaattgggagtaccctagctccaaacaccaacacaagaagctggtgaatagagatctgaaaacccagtctggcagcgaaatgaagaaatttctgagcacactgaccattgacggcgtgacccgcagcgaccagggcctgtacacctgtgccgcctcttctggccttatgaccaaaaaaaattctaccttcgtgcgggtgcacgagaagggcggaggcggctctagccccttcatcgccagcgtcagcgatcagcacggcgtggtctacatcaccgaaaacaagaacaagaccgtggtcattccttgcctgggcagcatcagtaatctgaacgtgagcctggtggccagataccctgagaagcggttcgtgcccgacggcaacaggatcagctgggacagcaagaagggctttacgatcccctcttatatgatctcctacgccggaatggtgttctgcgaggctaagatcaacgacgagagctaccagagcatcatgtacatcgtggtcgtggtcggctaccggatctacgacgtggtgctgagcccttctcacggcatcgagctgtccgtcggagagaagctggtgttgaattgcaccgccagaaccgagctgaacgtgggcatcgactttaactgggaataccccagctctaaacaccagcacaagaagctggtgaaccgggacctgaagacccaatctggtacagagatgaagaagttcctaagcacactgaccatcgacggcgtcacaagaagcgatcagggactgtacacctgcgccgctagcagcggactgatgaccaagaaaaacagcaccttcgtgcgggtgcacgagaaagacaagacacacacctgccctccatgtcctgcccctgaagctgctggcggaccttctgtgttcctcttcccacctaagcctaaggacaccctgatgatcagccggacacctgaagtgacatgcgtggtggtggatgtgtctcacgaagatcccgaggtgaaattcaactggtacgtggacggcgttgaagtgcataatgccaagaccaagcccagagaggaacagtacaacagcacctacagagtggtgtccgtactgaccgtgctgcaccaggactggctgaacggcaaggaatacaagtgcaaggtgtccaacaaagccctgcctgcccctatcgagaagaccatctctaaggccaagggccagcctagagaaccccaagtgtacacactgcctccttccagagaggaaatgaccaagaaccaggtgtcattgacatgtctggtgaaggggttctacccaagcgacatcgccgtggaatgggagagcaacggacagcccgagaacaactacaagaccacacctccagtgctcgatagcgacggcagcttcttcctgtatagcaagctgaccgtggacaagtccagatggcagcagggcaatgtgttcagctgcagcgtgatgcacgaggctctgcacaaccactacacccagaagagcctgtccctgagccccggcaagtga

SEQ ID NO: 130 - DNA, 1977 bp, synthetic construct
  source 1..1977: mol_type = other DNA
atgcccctgctcctgctcctgcccctgctgtgggccggcgccctggctagcgacaccggcagacccttcgtggagatgtacagcgagatccccgagatcatccacatgaccgagggcagagagctcgtgatcccttgcagagtgacaagccccaacatcaccgtgaccctgaaaaagttccccctggacaccctgatccccgacggcaagagaatcatctgggacagcagaaagggcttcatcatcagcaacgccacctacaaggagatcggcctgctgacctgcgaggccaccgtgaacggccacctgtacaagaccaactacctgacccacagacagaccaacaccatcatcgacgtcgtgctgagccctagccacggcatcgagctgagcgtgggcgaaaaactggtcctcaactgtaccgctcggaccgaactgaacgtggggatcgatttcaactgggagtatcctagctccaagcatcagcataagaagctggtcaacagagatctcaagacacagagcggctccgaaatgaaaaaattcctctccaccctgacaattgacggcgtcacacggagcgaccaaggcctgtatacctgcgctgctagcagcgggctgatgaccaagaagaactccacctttgtcagagtgcacgaaaagggcgggggcggcagcagccccttcatcgctagcgtgagcgatcagcacggcgtggtgtacatcaccgagaacaagaacaagaccgtggtgatcccctgcctgggcagcatcagcaacctgaacgtgagcctggtggctagataccccgagaagagattcgtgcccgacggcaacagaatcagctgggacagcaagaagggcttcaccatccctagctacatgatcagctacgccggcatggtgttctgcgaggccaagatcaacgacgagagctatcagagcatcatgtacatcgtggtcgtggtgggctacagaatctacgacgtggtgctgtcccctagccacggcattgaactgtccgtgggggagaagctggtgctgaactgtaccgcccggacagagctgaacgtgggcatcgactttaactgggagtaccctagcagcaaacatcagcacaagaagctggtgaaccgggacctgaagacacagagcggcacagaaatgaagaaattcctgagcacactgacaattgatggcgtgacaagaagcgaccaaggcctgtacacctgcgccgctagcagcggcctcatgacaaagaagaacagcacatttgtgcgggtgcacgagaaagacaaaacacatacctgtcctccctgtcccgcccctgaagccgctggggggcctagcgtgttcctgttcccccccaagcccaaggacacactgatgatcagcagaacccccgaggtgacctgcgtggtcgtggacgtgagccacgaggaccccgaggtgaagttcaactggtacgtggacggcgtggaggtgcacaacgccaagaccaagcctagagaggagcagtacaacagcacctacagagtggtgagcgtgctgaccgtgctgcaccaagactggctgaacggcaaggagtacaagtgcaaggtgagcaacaaggccctgcccgcccccatcgagaagaccatcagcaaggccaaggggcagcctagagagccccaagtgtacaccctgccccctagcagagaggagatgaccaaaaaccaagtgagcctgacctgcctggtgaagggcttctaccctagcgacatcgccgtggagtgggagagcaacgggcagcccgagaacaactacaagaccaccccccccgtgctggacagcgacggcagcttcttcctgtacagcaagctgaccgtggacaagagcagatggcagcaaggcaacgtgttcagctgcagcgtgatgcacgaggccctgcacaaccactacacacagaagagcctgagcctgagccccggcaagtga

SEQ ID NO: 131 - DNA, 1977 bp, synthetic construct
  source 1..1977: mol_type = other DNA
atgcctctgctgctgctgttgcctttgttgtgggctggcgccctggcttctgataccggcagacctttcgtggaaatgtacagcgagatccccgagatcatccacatgaccgagggcagagagctggtcatcccctgcagagtgacctctcctaacatcaccgtgactctgaagaagttccctctggacacactgatccccgacggcaagagaatcatctgggactcccggaagggcttcatcatctccaacgccacctacaaagagatcggcctgctgacctgcgaggccaccgttaatggccacctgtacaagaccaactatctgacccacagacagaccaacaccatcatcgacgtggtgctgagcccctctcatggcatcgagctgtccgtgggagaaaagctggtgctgaactgcaccgccagaaccgagctgaacgtgggcatcgacttcaactgggagtacccctccagcaagcaccagcacaagaagctggtcaaccgggacctgaaaacccagtccggctccgagatgaagaaattcctgagcaccctgaccatcgacggcgtgaccagatctgaccagggcctgtatacctgcgccgcttcttctggcctgatgaccaagaaaaactccaccttcgtgcgggtgcacgagaaaggtggcggaggcagctctccttttatcgcctctgtgtctgatcagcacggcgtggtgtacatcaccgagaacaagaacaagaccgtcgtgatcccctgcctgggctccatctctaacctgaacgtgtccctggtggctagataccccgagaagagattcgtgcctgacggcaaccggatctcctgggacagcaagaagggctttacaatcccctcctacatgatctcctacgccggcatggtgttctgcgaggctaagatcaacgacgagtcctaccagtccatcatgtacatcgtggtggtcgtgggctccaagatctacgatgtggtgctgtcccctagccacggaatcgaactgagcgtgggcgagaaactggtcctcaactgtaccgctcggacagaactgaatgtggggattgatttcaattgggaataccctagctccaaacatcagcataagaaactcgtgttccgcgatctcaagacccagagcggaacagaaatgaagaagtttctgtccacactcaccattgacggggtcaccagaagcgatcagggactctatacctgtgctgcctccagcggactgatgacaaaaaagaacagcacatttgtccgcgtccacgagaaggacaaaactcacacatgcccaccgtgcccggcgcctgaagccgctgggggaccgtcagtcttcctcttccccccaaaacccaaggacaccctcatgatctcccggacccctgaggtcacatgcgtggtggtggacgtgagccacgaagaccctgaggtcaagttcaactggtacgtggacggcgtggaggtgcataatgccaagacaaagccgcgggaggagcagtacaacagcacgtaccgggtggtcagcgtcctcaccgtcctgcaccaggactggctgaatggcaaggagtacaagtgcaaggtctccaacaaagccctcccagcccccatcgagaaaaccatctccaaagccaaagggcagcccagggaaccacaggtgtacaccctgcccccatcccgggaggagatgaccaagaaccaggtcagcctgacctgcctggtcaaaggcttctatcccagcgacatcgccgtggagtgggagagcaatgggcagccggagaacaactacaagaccacgcctcccgtgctggactccgacggctccttcttcctctacagcaagctcaccgtggacaagagcaggtggcagcaggggaacgtcttctcatgctccgtgatgcatgaggctctgcacaaccactacacgcagaagagcctctccctgtctccgggtaaataa

SEQ ID NO: 132 - DNA, 1977 bp, synthetic construct
  source 1..1977: mol_type = other DNA
atgcctctgctgctgctcctgcctctgctgtgggccggcgccctggccagcgataccggcagaccattcgtggaaatgtacagcgaaatccccgagatcatccacatgaccgagggcagagaactggtgatcccctgcagagtgaccagcccaaacatcaccgtgaccctcaagaagtttcccctggacaccctgatccctgatggaaaaagaatcatctgggacagcagaaagggctttatcatttctaatgccacatacaaagagataggactgttgacctgtgaagctacagttaacggccacctgtacaagaccaactacctgacccaccggcagacaaacaccatcatcgacgtggtgctgagccctagccacggaatcgagctgtccgtgggagaaaagctggtgctgaattgcaccgccagaaccgagctgaacgtaggcatcgacttcaactgggagtatccttcaagcaaacatcagcacaaaaaactggtgaacagagacctgaagacccagagtggcagcgagatgaaaaagttcctgagcacactgacaatcgacggagtgactcggagcgatcagggcctgtatacatgtgctgcttctagcggcctgatgacaaagaagaacagcacattcgtgcgggtgcacgagaaggggggcggcggatcttccccattcatcgccagcgtgtccgaccagcatggcgtggtttacatcacagaaaacaagaacaagaccgtggtgatcccctgcctgggctccatcagcaacctgaatgtgtcgctggtggccagataccccgaaaagcggttcgtccccgacggcaacagaatcagctgggacagcaaaaagggcttcaccatcccaagctatatgatcagctacgccggaatggtgttctgcgaggccaaaatcaacgacgagtcctaccagagcatcatgtacatcgtggtggttgtcggcagcaagatctacgacgtcgtgctgagcccatctcacggcattgagctgtctgtgggcgagaagctggtgctgaattgcaccgcccggacagaactcaatgtgggcatcgatttcaactgggagtaccctagctctaagcaccagcacaagaagctggtctttagagatctgaaaacccaatctggcaccgagatgaaaaagttcctgagcaccctgaccatcgacggcgtgaccagaagcgaccagggcctgtacacctgcgccgcctctagcggcctgatgaccaagaaaaacagcaccttcgtgcgcgttcacgagaaagataagacacacacctgtcctccttgtcctgcccctgaggccgctggcggaccttctgtgttcctgttccctccaaagcccaaggacaccctgatgatcagcagaacacccgaagtgacctgcgtggtggtggacgtctctcacgaggaccccgaggtgaaatttaactggtacgtggacggcgtcgaggtgcataatgccaagacaaagcctcgggaagagcagtacaacagcacatacagagtggtcagcgtgctgacagtgctgcaccaggattggctgaacggcaaggaatacaagtgcaaggtgagcaacaaggccctgcctgctcctatcgagaagaccattagcaaggccaagggccagcctagggagcctcaggtgtacaccttaccacctagcagagaggaaatgacgaagaaccaggtgtccctgacatgcctggtgaagggtttctacccttctgatatcgccgtggaatgggaatccaacggccaacctgagaacaactacaagaccacccctcccgtgctcgatagcgacggctccttcttcctgtacagcaagctgaccgtggataagagccggtggcagcagggcaatgtgtttagctgctctgtgatgcacgaagccctgcacaaccactacacccaaaagagcctgagcctgagccccggcaagtga

SEQ ID NO: 133 - DNA, 1977 bp, synthetic construct
  source 1..1977: mol_type = other DNA
atgcccctgctcctgctcctgcccctgctgtgggccggcgccctggctagcgacaccggcagacccttcgtggagatgtacagcgagatccccgagatcatccacatgaccgagggcagagagctcgtgatcccttgcagagtgacaagccccaacatcaccgtgaccctgaaaaagttccccctggacaccctgatccccgacggcaagagaatcatctgggacagcagaaagggcttcatcatcagcaacgccacctacaaggagatcggcctgctgacctgcgaggccaccgtgaacggccacctgtacaagaccaactacctgacccacagacagaccaacaccatcatcgacgtcgtgctgagccctagccacggcatcgagctgtccgtgggcgaaaagctcgtcctgaactgcaccgctagaaccgaactcaacgtggggattgatttcaactgggagtatcctagctccaagcaccaacacaagaagctggtgaaccgggatctgaagacacagagcgggagcgagatgaagaagttcctgagcaccctgacaatcgacggggtgacaagatccgaccaaggcctgtacacctgcgctgctagcagcggcctgatgacaaagaaaaatagcacatttgtgagagtgcacgagaagggcgggggcggcagcagccccttcatcgctagcgtgagcgatcagcacggcgtggtgtacatcaccgagaacaagaacaagaccgtggtgatcccctgcctgggcagcatcagcaacctgaacgtgagcctggtggctagataccccgagaagagattcgtgcccgacggcaacagaatcagctgggacagcaagaagggcttcaccatccctagctacatgatcagctacgccggcatggtgttctgcgaggccaagatcaacgacgagagctatcagagcatcatgtacatcgtggtcgtggtgggcagcaagatctacgacgtggtgctgagcccctcccacggcattgagctcagcgtgggcgagaagctggtcctcaactgcacagcccggaccgagctgaacgtgggcatcgattttaactgggagtaccctagcagcaagcatcagcataaaaagctggtgttccgggacctgaagacccaaagcggcaccgaaatgaagaagtttctctccaccctgaccatcgacggcgtgacaagaagcgaccaaggcctgtacacatgcgccgctagctccggcctcatgacaaagaagaattccacctttgtcagagtccatgaaaaagataagacacacacctgtcccccttgtcccgcccccgaagccgctgggggccctagcgtgttcctgttcccccccaagcccaaggataccctgatgatcagcagaacccccgaggtgacctgcgtggtcgtggacgtgagccacgaggaccccgaggtgaagttcaactggtacgtggacggcgtggaggtgcacaacgccaagaccaagcctagagaggagcagtacaacagcacctacagagtggtgagcgtgctgaccgtgctgcaccaagactggctgaacggcaaggagtacaagtgcaaggtgagcaacaaggccctgcccgcccccatcgagaagaccatcagcaaggccaaggggcagcctagagagccccaagtgtacaccctgccccctagcagagaggagatgaccaagaaccaagtgagcctgacctgcctggtgaagggcttctaccctagcgacatcgccgtggagtgggagagcaacgggcagcccgagaacaactacaagaccaccccccccgtgctggacagcgacggcagcttcttcctgtacagcaagctgaccgtggacaagagcagatggcagcaaggcaacgtgttcagctgcagcgtgatgcacgaggccctgcacaaccactacacacagaagagcctgagcctgagccccggcaagtga

SEQ ID NO: 134 - protein, 2826 aa, synthetic construct
ATGCCTCTGCTGCTGCTGTTGCCTTTGTTGTGGGCTGGCGCTCTGGCCTCTCCTTTTATCGCCTCTGTGTCTGATCAGCACGGCGTGGTGTACATCACCGAGAACAAGAACAAGACCGTCGTGATCCCCTGCCTGGGCTCCATCTCTAACCTGAACGTGTCCCTGGTGGCTAGATACCCCGAGAAGAGATTCGTGCCTGACGGCAACCGGATCTCCTGGGACAGCAAGAAGGGCTTTACAATCCCCTCCTACATGATCTCCTACGCCGGCATGGTGTTCTGCGAGGCTAAGATCAACGACGAGTCCTACCAGTCCATCATGTACATCGTGGTGGTCGTGGGCTACAGAATCTACGATGTGGTGCTGTCCCCTAGCCACGGAATCGAACTGAGCGTGGGCGAGAAACTGGTCCTCAACTGTACCGCTCGGACAGAACTGAATGTGGGGATTGATTTCAATTGGGAATACCCTAGCTCCAAACATCAGCATAAGAAACTCGTGAACCGCGATCTCAAGACCCAGAGCGGAAGCGAAATGAAGAAGTTTCTGTCCACACTCACCATTGACGGGGTCACCAGAAGCGATCAGGGACTCTATACCTGTGCTGCCTCCAGCGGACTGATGACAAAAAAGAACAGCACATTTGTCCGCGTCCACGAGAAGGACAAAACTCACACATGCCCACCGTGCCCGGCGCCTGAAGCCGCTGGGGGACCGTCAGTCTTCCTCTTCCCCCCAAAACCCAAGGACACCCTCATGATCTCCCGGACCCCTGAGGTCACATGCGTGGTGGTGGACGTGAGCCACGAAGACCCTGAGGTCAAGTTCAACTGGTACGTGGACGGCGTGGAGGTGCATAATGCCAAGACAAAGCCGCGGGAGGAGCAGTACAACAGCACGTACCGGGTGGTCAGCGTCCTCACCGTCCTGCACCAGGACTGGCTGAATGGCAAGGAGTACAAGTGCAAGGTCTCCAACAAAGCCCTCCCAGCCCCCATCGAGAAAACCATCTCCAAAGCCAAAGGGCAGCCCAGGGAACCACAGGTGTACACCCTGCCCCCATCCCGGGAGGAGATGACCAAGAACCAGGTCAGCCTGACCTGCCTGGTCAAAGGCTTCTATCCCAGCGACATCGCCGTGGAGTGGGAGAGCAATGGGCAGCCGGAGAACAACTACAAGACCACGCCTCCCGTGCTGGACTCCGACGGCTCCTTCTTCCTCTACAGCAAGCTCACCGTGGACAAGAGCAGGTGGCAGCAGGGGAACGTCTTCTCATGCTCCGTGATGCATGAGGCTCTGCACAACCACTACACGCAGAAGAGCCTCTCCCTGTCTCCGGGTGGCGGAGGCGGCTCCGGTGGAGGCGGTTCAGGCGGAGGTGGCTCTGGCGGTGGCGGATCGGAGGTGCAGCTGGTGGAGAGCGGGGGGGGACTGGTGCAGCCAGGAGGAAGCCTGAGACTGAGCTGTGCCGCCAGCGGGTACACATTTACCAACTACGGAATGAACTGGGTGAGGCAGGCTCCTGGCAAGGGGCTGGAGTGGGTGGGGTGGATTAACACCTACACCGGAGAGCCCACATACGCTGCTGATTTTAAGCGGAGATTCACCTTCAGCCTGGACACCAGCAAGAGCACCGCTTACCTGCAGATGAACAGCCTGAGAGCCGAGGACACAGCCGTGTACTACTGCGCCAAATACCCCCATTACTACGGCAGCAGCCACTGGTACTTCGACGTGTGGGGCCAGGGAACACTGGTGACCGTGAGCAGCGCTAGCACCAAGGGCCCATCGGTCTTCCCCCTGGCACCCTCCTCCAAGAGCACCTCTGGGGGCACAGCGGCCCTGGGCTGCCTGGTCAAGGACTACTTCCCCGAACCGGTGACGGTGTCGTGGAACTCAGGCGCCCTGACCAGCGGCGTGCACACCTTCCCGGCTGTCCTACAGTCCTCAGGACTCTACTCCCTCAGCAGCGTGGTGACCGTGCCCTCCAGCAGCTTGGGCACCCAGACCTACATCTGCAACGTGAATCACAAGCCCAGCAACACCAAGGTGGACAAGAAAGTTGAGCCCAAATCTTGTGAGGGCAGAGGAAGTCTTCTAACATGCGGTGACGTGGAGGAGAATCCCGGCCCTATGCCTCTGCTGCTGCTGTTGCCTTTGTTGTGGGCTGGCGCTCTGGCCGACATTCAGATGACCCAGAGCCCCAGCAGCCTGAGCGCCAGCGTGGGAGACAGAGTGACCATCACCTGCAGCGCCAGCCAGGACATCAGCAACTACCTGAACTGGTATCAGCAGAAACCCGGCAAAGCCCCCAAAGTGCTGATCTACTTCACAAGTTCACTGCACAGCGGAGTGCCCAGCAGATTTTCAGGAAGCGGCAGCGGCACCGACTTCACCCTGACCATCAGCAGCCTGCAGCCCGAGGATTTCGCCACCTACTACTGCCAGCAGTACTCTACCGTGCCATGGACCTTCGGCCAGGGGACCAAGGTGGAAATCAAGCGTACGGTGGCTGCACCATCTGTCTTCATCTTCCCGCCATCTGATGAGCAGTTGAAATCTGGAACTGCCTCTGTTGTGTGCCTGCTGAATAACTTCTATCCCAGAGAGGCCAAAGTACAGTGGAAGGTGGATAACGCCCTCCAATCGGGTAACTCCCAGGAGAGTGTCACAGAGCAGGACAGCAAGGACAGCACCTACAGCCTCAGCAGCACCCTGACGCTGAGCAAAGCAGACTACGAGAAACACAAAGTCTACGCCTGCGAAGTCACCCATCAGGGCCTGAGTTCGCCCGTCACAAAGAGCTTCAACAGGGGAGAGTGTTAA

SEQ ID NO: 135 - DNA, 2826 bp, synthetic construct
  source 1..2826: mol_type = other DNA
atgcctctgcttctgctgctgcctctgctttgggctggcgccctggccagccccttcatcgcctctgttagtgaccagcatggcgtggtgtatatcacggagaacaagaataagacagtagtgattccttgcctgggcagcatctctaatctgaacgtgtcgctggttgccagataccctgagaagagattcgtgcccgacggcaaccggatcagctgggacagcaagaagggctttaccatcccctcttacatgatcagctatgccggaatggtgttctgcgaagccaagatcaacgacgagtcctatcagtctatcatgtacatcgtggtcgtagtgggctacagaatctacgacgtggtgctgagcccatctcacggcatcgagctgagcgtgggagagaagctggtgctgaactgcacagctagaaccgagctgaacgtgggcatagacttcaactgggagtacccctccagcaagcaccagcacaagaaactggtcaacagagatctgaagacccagagcggctctgagatgaagaagttcctgtccaccctgacaatcgacggcgtgaccagaagcgatcagggactgtacacttgtgctgcgagctctggcctgatgaccaagaaaaacagcaccttcgtgcgggtgcacgagaaggacaagacccacacatgccctccttgtcctgcccctgaggccgctggcggccctagcgtgttcctgttcccccctaaacccaaggacaccctcatgatctcccggacacctgaagtgacttgcgtggtcgtggacgtcagccacgaagatccagaggtgaagttcaactggtatgtggatggcgtggaagtgcataatgcgaagacaaagcctcgggaagagcagtacaactccacgtacagagtggtgagcgtgctgaccgtgctgcatcaagactggctgaacggcaaggaatacaagtgcaaggtgtccaacaaggccctgcccgctcctatcgaaaaaaccatctctaaggccaagggccagcctagagagcctcaggtgtataccctgcctcctagccgggaagaaatgacaaagaaccaggtgtctctgacctgcctggtgaagggcttctaccccagcgacatcgccgtggagtgggagtccaacggccaacctgaaaacaattacaagaccacccctcccgtgctggacagcgacggcagcttcttcctgtattccaagctgaccgtcgacaagagcagatggcagcagggcaacgtgtttagctgtagcgtgatgcacgaggccctgcacaaccactacacacaaaagtctctgtccctgagccctggaggcggcggcggaagcggagggggcggctccggcggcggaggcagcggcggcggcggttccgaagtgcagctggtggaaagcggaggcggtctggttcagccgggcggcagcctgagactgtcttgcgccgccagcggctacacattcaccaactacggcatgaactgggtcagacaggcccctggcaagggcctggaatgggtgggatggatcaacacctacaccggcgaaccaacatacgccgctgattttaagcggaggttcaccttttctctggatacctccaaaagcaccgcctacctgcaaatgaacagcctgcgggccgaggacaccgccgtttactactgcgccaaatatcctcactactacggcagctctcactggtacttcgacgtttggggccagggcacactggtgaccgtgtcctcggccagcacaaagggccctagcgtgttcccactggcaccatctagcaagagcaccagtggaggcaccgccgccctgggatgcctggtgaaagattacttccccgagcctgtcaccgtgtcttggaactccggtgctctgacgagcggagtgcacaccttcccagccgtgcttcagtccagcggtctgtacagcctgtcttctgttgtgaccgtgccttccagctccctgggcacgcagacctacatctgcaacgtgaaccacaagcctagcaataccaaggtggataagaaggtggaacccaaaagctgcgagggaagaggctccctcctgacatgcggcgacgtggaagagaaccccggccctatgcccctgctgctgctgctgcctctgctgtgggccggcgccctggccgatatccagatgacccagtctccttcctccttatccgcctctgtgggcgacagagtgaccatcacctgttctgccagccaggatatcagcaactacctgaactggtaccagcagaagcccggcaaagccccaaaggtgctgatttacttcacaagcagcctgcacagcggagtgcctagccgcttcagcggctctggcagcgggaccgactttacactgaccattagcagcctgcagcctgaggatttcgccacatactactgtcagcaatacagcacagtcccttggacctttggacaaggaacaaaggtggaaatcaagcggaccgtggccgctcccagcgtgttcatcttccctcctagcgacgagcaactgaaatctggcaccgccagcgtcgtgtgcctgctgaacaacttctacccgagagaggctaaggtgcagtggaaggtggacaacgccctgcagagcgggaatagccaggagagcgtgaccgagcaggactccaaagacagcacatactctctgagcagcacccttacactgagcaaggccgactacgagaaacacaaagtgtacgcttgtgaggtgacccaccagggcctgagctctcccgtgaccaaaagctttaatagaggcgagtgctga

SEQ ID NO: 136 - DNA, 2826 bp, synthetic construct
  source 1..2826: mol_type = other DNA
atgcctctgctgctgcttctgcctcttctttgggctggcgctctggctagcccttttatcgcctccgtgtccgatcagcacggcgtggtgtacatcaccgagaacaagaacaagaccgtggtcatcccctgcctgggcagcatcagcaacctgaatgtgtccctggtggccagatatcccgagaagagattcgtgcccgacggcaacagaatcagctgggacagcaagaagggcttcacaatccccagctacatgatcagctacgccggcatggtgttctgcgaggccaagatcaacgacgagagctaccagagcatcatgtacatcgtggtggtcgtgggctacagaatctacgacgtggtgctgagccctagccacggcattgaactgtctgtgggcgagaagctggtgctgaactgtaccgccagaaccgagctgaacgtgggcatcgacttcaactgggagtaccccagcagcaagcaccagcacaagaaactggtcaaccgggacctgaaaacccagagcggcagcgagatgaagaagttcctgagcaccctgaccatcgacggcgtgaccagatctgaccagggcctgtacacatgtgccgccagctctggcctgatgaccaagaaaaacagcaccttcgtgcgggtgcacgagaaggacaagacccacacctgtcctccatgtcctgctccagaagctgctggcggcccttccgtgtttctgttccctccaaagcctaaggacaccctgatgatcagcagaacccctgaagtgacctgcgtggtggtggatgtgtcccacgaggatcccgaagtgaagttcaattggtacgtggacggcgtggaagtgcacaacgccaagaccaagcctagagaggaacagtacaactccacctacagagtggtgtccgtgctgaccgtgctgcaccaggattggctgaacggcaaagagtacaagtgcaaggtgtccaacaaggccctgcctgctcctatcgagaaaaccatcagcaaggccaagggccagcctagggaaccccaggtttacacactgcctccaagccgggaagagatgacaaagaaccaggtgtccctgacctgcctggtcaagggcttctacccttccgatatcgccgtggaatgggagagcaatggccagcctgagaacaactacaagacaacccctcctgtgctggacagcgacggctcattcttcctgtacagcaagctgacagtggacaagagcagatggcagcagggcaacgtgttcagctgcagcgtgatgcacgaggccctgcacaaccactacacccagaagtccctgtctctgtctcctggcggaggcggaggatctggtggcggaggaagcggtggcggcggatcaggcggtggtggttctgaagttcagctggtggaaagcggcggtggccttgttcaacctggcggatctctgagactgagctgtgccgcctctggctacaccttcaccaactacggcatgaattgggtccgacaggcccctggcaaaggcctggaatgggtcggatggatcaacacctacaccggcgagccaacatacgccgccgacttcaagcggagattcaccttcagcctggacaccagcaagagcaccgcctacctgcagatgaactccctgagagccgaggacaccgccgtgtactactgcgccaagtatccccactactacggcagcagccactggtactttgacgtgtggggacagggcaccctggtcacagttagcagcgcctctacaaagggccccagcgttttcccactggctcctagcagcaagtctacctccggtggaacagctgccctgggctgtctcgtgaaggactactttcctgagcctgtgaccgtgtcctggaactctggcgcactgacatctggcgtgcacacctttccagctgtgctgcagtctagcggcctgtactctctgagcagcgtcgtgacagtgcctagcagctctctgggcacccagacctacatctgcaatgtgaaccacaagcctagcaacaccaaggtcgacaagaaggtggaacccaagagctgcgaaggcagaggcagcctgcttacatgtggcgacgtggaagagaaccccggacctatgccacttctcctgctgttgccattgctgtgggcaggcgcactggccgacattcagatgacacagagcccaagcagcctgagcgcctctgtgggagatagagtgaccatcacctgttccgccagccaggacatctccaactacctgaactggtatcagcaaaagcccggcaaggcccctaaggtgctgatctactttaccagcagcctgcacagcggcgtgcccagcagattttctggctctggcagcggcaccgacttcaccctgacaatatctagcctgcagccagaggacttcgccacctactactgccagcagtacagcaccgtgccttggacatttggccagggcaccaaggtggaaatcaagcggacagtcgccgctcctagcgtgttcatctttccacctagcgacgagcagctgaagtctggcacagcctctgtcgtgtgcctgctgaacaacttctaccccagagaagccaaggtgcagtggaaggtggacaatgccctgcagtccggcaacagccaagagagcgtgacagagcaggactccaaggacagcacctacagcctgtctagcacactgaccctgagcaaggccgactatgagaagcacaaagtgtacgcctgcgaagtgacccaccaggggctttctagcccagtgaccaagagcttcaaccggggcgagtgttga

SEQ ID NO: 137 - DNA, 133 bp, synthetic construct
  source 1..133: mol_type = other DNA
gtctagaaaccagcctcaagaacacccgaatggagtctctaagctacataataccaacttacactttacaaaatgttgtcccccaaaatgtagccattcgtatctgctcctaataaaaagaaagtttcttcac

SEQ ID NO: 138 - DNA, 589 bp, synthetic construct; identical to SEQ ID NO: 34
  source 1..589: mol_type = other DNA

SEQ ID NO: 139 - DNA, 140 bp, synthetic construct
  source 1..140: mol_type = other DNA
cctaggtaagatacattgatgagtttggacaaaccacaactagaatgcagtgaaaaaaatgctttatttgtgaaatttgtgatgctattgctttatttgtaaccattataagctgcaataaacaagttatcgatagatct

SEQ ID NO: 140 - DNA, 3988 bp, synthetic construct
  source 1..3988: mol_type = other DNA
cctgcaggcagctgcgcgctcgctcgctcactgaggccgcccgggcaaagcccgggcgtcgggcgacctttggtcgcccggcctcagtgagcgagcgagcgcgcagagagggagtggccaactccatcactaggggttcctatcgatatcaagcttcgttacataacttacggtaaatggcccgcctggctgaccgcccaacgacccccgcccattgacgtcaatagtaacgccaatagggactttccattgacgtcaatgggtggagtatttacggtaaactgcccacttggcagtacatcaagtgtatcatatgccaagtacgccccctattgacgtcaatgacggtaaatggcccgcctggcattgtgcccagtacatgaccttatgggactttcctacttggcagtacatctacgtattagtcatcgctattaccatggtcgaggtgagccccacgttctgcttcactctccccatctcccccccctccccacccccaattttgtatttatttattttttaattattttgtgcagcgatgggggcggggggggggggggggcgcgcgccaggcggggcggggcggggcgaggggcggggcggggcgaggcggagaggtgcggcggcagccaatcagagcggcgcgctccgaaagtttccttttatggcgaggcggcggcggcggcggccctataaaaagcgaagcgcgcggcgggcgggagtcgctgcgcgctgccttcgccccgtgccccgctccgccgccgcctcgcgccgcccgccccggctctgactgaccgcgttactcccacaggtgagcgggcgggacggcccttctcctccgggctgtaattagctgagcaagaggtaagggtttaagggatggttggttggtggggtattaatgtttaattacctggagcacctgcctgaaatcactttttttcaggttgggggattcgaacatcggccgccaccatgaacgccagcgagtttcggcggagaggcaaagaaatggtggactacgtggccaactacatggaaggcatcgagggcagacaggtgtaccccgatgtggaacctggctacctgaggcctctgattcctgccgctgctccccaagagcctgacaccttcgaggacatcatcaacgacgtggaaaagatcatcatgcccggcgtgacccactggcacagcccctactttttcgcctactttcccaccgccagcagctaccctgctatgctggctgatatgctgtgtggcgccatcggctgcatcggcttttcttgggctgcctctcctgcctgcaccgagctggaaaccgtgatgatggattggctgggcaagatgctggaactgcccaaggccttcctgaacgagaaagctggcgaaggcggcggagtgattcagggatctgcctctgaagccacactggtggctctgctggccgccagaacaaaagtgatccacagactgcaggccgcctctccagaactgacacaggccgccatcatggaaaagctggtggcctacagcagcgatcaggcccacagctctgtggaaagagccggactgattggcggcgtgaagctgaaggccattcctagcgacggcaacttcgccatgagagcctctgctctgcaagaggccctggaaagagataaggccgctggactgatccccttcttcatggtggctaccctgggcaccaccacctgttgcagcttcgacaacctgctggaagtgggccccatctgcaacaaagaggacatctggctgcacgtggacgccgcctatgccggctctgcctttatctgccccgagttcagacatctgctgaacggcgtggaattcgccgacagcttcaacttcaaccctcacaagtggctgctggtcaacttcgactgcagcgctatgtgggtcaagaagcggaccgatctgaccggcgccttcagactggatcccacctacctgaagcactcccaccaggatagcggcctgatcaccgactaccggcactggcagattcctctgggcagaagatttcggagcctgaagatgtggttcgtgttccggatgtatggcgtgaagggcctccaggcctacatcagaaaacatgtgcagctgagccacgagttcgagagccttgtcagacaggaccccagattcgagatctgcgtggaagtgatcctgggcctcgtgtgctttagactgaagggcagcaacaaagtgaacgaggccctgctgcagcggatcaacagcgccaaaaagatccacctggtgccttgccacctgagagacaagttcgtgctgagattcgccatctgcagccggacagtggaaagcgcccatgtgcagagagcctgggagcacatcaaagaactggccgccgatgtgctgagggccgagagagaagccaccaacttctccctgctgaagcaggccggcgacgtggaggagaaccccggccccatgaagctgtgggacgtggtggccgtgtgcctggtgctgctgcacaccgccagcgccttccccctgcccgccggcaagcgcccccccgaggcccccgccgaggaccgcagcctgggccgccgccgcgcccccttcgccctgagcagcgacagcaacatgcccgaggactaccccgaccagttcgacgacgtgatggacttcatccaggccaccatcaagcgcctgaagcgcagccccgacaagcagatggccgtgctgccccgccgcgagcgcaaccgccaggccgccgccgccaaccccgagaacagccgcggcaagggccgccgcggccagcgcggcaagaaccgcggctgcgtgctgaccgccatccacctgaacgtgaccgacctgggcctgggctacgagaccaaggaggagctgatcttccgctactgcagcggcagctgcgacgccgccgagaccacctacgacaagatcctgaagaacctgagccgcaaccgccgcctggtgagcgacaaggtgggccaggcctgctgccgccccatcgccttcgacgacgacctgagcttcctggacgacaacctggtgtaccacatcctgcgcaagcacagcgccaagcgctgcggctgcatctaactcgagaatcaacctctggattacaaaatttgtgaaagattgactggtattcttaactatgttgctccttttacgctatgtggatacgctgctttaatgcctttgtatcatgctattgcttcccgtatggctttcattttctcctccttgtataaatcctggttgctgtctctttatgaggagttgtggcccgttgtcaggcaacgtggcgtggtgtgcactgtgtttgctgacgcaacccccactggttggggcattgccaccacctgtcagctcctttccgggactttcgctttccccctccctattgccacggcggaactcatcgccgcctgccttgcccgctgctggacaggggctcggctgttgggcactgacaattccgtggtgttgtcggggaaatcatcgtcctttccttggctgctcgcctgtgttgccacctggattctgcgcgggacgtccttctgctacgtcccttcggccctcaatccagcggaccttccttcccgcggcctgctgccggctctgcggcctcttccgcgtcttcgccttcgccctcagacgagtcggatctccctttgggccgcctccccgctaagatacattgatgagtttggacaaaccacaactagaatgcagtgaaaaaaatgctttatttgtgaaatttgtgatgctattgctttatttgtaaccattataagctgcaataaacaagttcggaccgagcggcagatctaggaacccctagtgatggagttggccactccctctctgcgcgctcgctcgctcactgaggccgggcgaccaaaggtcgcccgacgcccgggctttgcccgggcggcctcagtgagcgagcgagcgcgcagctgcctgcagg

SEQ ID NO: 141 - DNA, 4506 bp, synthetic construct
  source 1..4506: mol_type = other DNA
cctgcaggcagctgcgcgctcgctcgctcactgaggccgcccgggcaaagcccgggcgtcgggcgacctttggtcgcccggcctcagtgagcgagcgagcgcgcagagagggagtggccaactccatcactaggggttcctatcgatatccgttacataacttacggtaaatggcccgcctggctgaccgcccaacgacccccgcccattgacgtcaataatgacgtatgttcccatagtaacgtcaatagggactttccattgacgtcaatgggtggagtatttacggtaaactgcccacttggcagtacatcaagtgtatcatatgccaagtacgccccctattgacgtcaatgacggtaaatggcccgcctggcattatgcccagtacatgaccttatgggactttcctacttggcagtacatctacgtattagtcatcgctattaccatggtgatgcggttttggcagtacatcaatgggcgtggatagcggtttgactcacggggatttccaagtctccaccccattgacgtcaatgggagtttgttttgcaccaaaatcaacgggactttccaaaatgtcgtaacaactccgccccattgacgcaaatgggcggtaggcgtgtacggtgggaggtctatataagcagagctgtgagtttggggacccttgattgttctttctttttcgctattgtaaaattcatgttatatggagggggcaaagttttcagggtgttgtttagaatgggaagatgtcccttgtatcaccatggaccctcatgataattttgtttctttcactttctactctgttgacaaccattgtctcctcttattttcttttcattttctgtaactttttcgttaaactttagcttgcatttgtaacgaatttttaaattcacttttgtttatttgtcagattgtaagtactttctctaatcacttttttttcaaggcaatcagggtatattatattgtacttcagcacagttttagagaacaattgttataattaaatgataaggtagaatatttctgcatataaattctggctggcgtggaaatattcttattggtagaaacaactacatcctggtcatcatcctgcctttctctttatggttacaatgatatacactgtttgagatgaggataaaatactctgagtccaaaccgggcccctctgctaaccatgttcatgccttcttctttttcctacaggccaccatgaagctgtgggacgtggtggccgtgtgcctggtgctgctgcacaccgccagcgccttccccctgcccgccggcaagcgcccccccgaggcccccgccgaggaccgcagcctgggccgccgccgcgcccccttcgccctgagcagcgacagcaacatgcccgaggactaccccgaccagttcgacgacgtgatggacttcatccaggccaccatcaagcgcctgaagcgcagccccgacaagcagatggccgtgctgccccgccgcgagcgcaaccgccaggccgccgccgccaaccccgagaacagccgcggcaagggccgccgcggccagcgcggcaagaaccgcggctgcgtgctgaccgccatccacctgaacgtgaccgacctgggcctgggctacgagaccaaggaggagctgatcttccgctactgcagcggcagctgcgacgccgccgagaccacctacgacaagatcctgaagaacctgagccgcaaccgccgcctggtgagcgacaaggtgggccaggcctgctgccgccccatcgccttcgacgacgacctgagcttcctggacgacaacctggtgtaccacatcctgcgcaagcacagcgccaagcgctgcggctgcatctaaaataaagtctgagtgggcggcagcctgtgtgtgcctgggttctctctgtcccggaatgtgcaaacaatggaggtgaagcttcgttacataacttacggtaaatggcccgcctggctgaccgcccaacgacccccgcccattgacgtcaatagtaacgccaatagggactttccattgacgtcaatgggtggagtatttacggtaaactgcccacttggcagtacatcaagtgtatcatatgccaagtacgccccctattgacgtcaatgacggtaaatggcccgcctggcattgtgcccagtacatgaccttatgggactttcctacttggcagtacatctacgtattagtcatcgctattaccatggtcgaggtgagccccacgttctgcttcactctccccatctcccccccctccccacccccaattttgtatttatttattttttaattattttgtgcagcgatgggggcggggggggggggggggcgcgcgccaggcggggcggggcggggcgaggggcggggcggggcgaggcggagaggtgcggcggcagccaatcagagcggcgcgctccgaaagtttccttttatggcgaggcggcggcggcggcggccctataaaaagcgaagcgcgcggcgggcgggagtcgctgcgcgctgccttcgccccgtgccccgctccgccgccgcctcgcgccgcccgccccggctctgactgaccgcgttactcccacaggtgagcgggcgggacggcccttctcctccgggctgtaattagctgagcaagaggtaagggtttaagggatggttggttggtggggtattaatgtttaattacctggagcacctgcctgaaatcactttttttcaggttgggggattcgaacatcggccgccaccatgaacgccagcgagtttcggcggagaggcaaagaaatggtggactacgtggccaactacatggaaggcatcgagggcagacaggtgtaccccgatgtggaacctggctacctgaggcctctgattcctgccgctgctccccaagagcctgacaccttcgaggacatcatcaacgacgtggaaaagatcatcatgcccggcgtgacccactggcacagcccctactttttcgcctactttcccaccgccagcagctaccctgctatgctggctgatatgctgtgtggcgccatcggctgcatcggcttttcttgggctgcctctcctgcctgcaccgagctggaaaccgtgatgatggattggctgggcaagatgctggaactgcccaaggccttcctgaacgagaaagctggcgaaggcggcggagtgattcagggatctgcctctgaagccacactggtggctctgctggccgccagaacaaaagtgatccacagactgcaggccgcctctccagaactgacacaggccgccatcatggaaaagctggtggcctacagcagcgatcaggcccacagctctgtggaaagagccggactgattggcggcgtgaagctgaaggccattcctagcgacggcaacttcgccatgagagcctctgctctgcaagaggccctggaaagagataaggccgctggactgatccccttcttcatggtggctaccctgggcaccaccacctgttgcagcttcgacaacctgctggaagtgggccccatctgcaacaaagaggacatctggctgcacgtggacgccgcctatgccggctctgcctttatctgccccgagttcagacatctgctgaacggcgtggaattcgccgacagcttcaacttcaaccctcacaagtggctgctggtcaacttcgactgcagcgctatgtgggtcaagaagcggaccgatctgaccggcgccttcagactggatcccacctacctgaagcactcccaccaggatagcggcctgatcaccgactaccggcactggcagattcctctgggcagaagatttcggagcctgaagatgtggttcgtgttccggatgtatggcgtgaagggcctccaggcctacatcagaaaacatgtgcagctgagccacgagttcgagagccttgtcagacaggaccccagattcgagatctgcgtggaagtgatcctgggcctcgtgtgctttagactgaagggcagcaacaaagtgaacgaggccctgctgcagcggatcaacagcgccaaaaagatccacctggtgccttgccacctgagagacaagttcgtgctgagattcgccatctgcagccggacagtggaaagcgcccatgtgcagagagcctgggagcacatcaaagaactggccgccgatgtgctgagggccgagagagaatgactcgagtaagatacattgatgagtttggacaaaccacaactagaatgcagtgaaaaaaatgctttatttgtgaaatttgtgatgctattgctttatttgtaaccattataagctgcaataaacaagttcggaccgagcggcagatctaggaacccctagtgatggagttggccactccctctctgcgcgctcgctcgctcactgaggccgggcgaccaaaggtcgcccgacgcccgggctttgcccgggcggcctcagtgagcgagcgagcgcgcagctgcctgcagg